European Patent Application EP 4 810 525 A1, published September 23, 2026. Title: キメラ抗原受容体. Applicant: 大塚製薬株式会社. The sequence listing filed with the application follows.

SEQUENCE LISTING (162 sequences)

SEQ ID NO: 1 - protein, 5 aa, synthetic construct
NYWMN

SEQ ID NO: 2 - protein, 19 aa, synthetic construct
EIRLKSNNYATHYAESVKG

SEQ ID NO: 3 - protein, 6 aa, synthetic construct
LPSFDY

SEQ ID NO: 4 - protein, 117 aa, synthetic construct
EVKLEESGGGLVQPGGSMKLSCVASGFTFSNYWMNWVRQSPEKGLEWVAEIRLKSNNYATHYAESVKGRFTISRDDSKSSVYLQMNNLRAEDTGIYYCSRLPSFDYWGQGTTLTVSS

SEQ ID NO: 5 - protein, 16 aa, synthetic construct
RSTKSLLHSNGNTYLY

SEQ ID NO: 6 - protein, 7 aa, synthetic construct
RMSNLAS

SEQ ID NO: 7 - protein, 9 aa, synthetic construct
MQHLEYPFT

SEQ ID NO: 8 - protein, 113 aa, synthetic construct
DIVMTQAAPSVPVTPGESVSISCRSTKSLLHSNGNTYLYWFLQRPGQSPQLLIYRMSNLASGVPDRFSGSGSGTAFTLRITRVEAEDVGIYYCMQHLEYPFTFGAGTKLELKR

SEQ ID NO: 9 - DNA, 15 bp, synthetic construct
  source 1..15: mol_type = other DNA
aattactggatgaac

SEQ ID NO: 10 - DNA, 57 bp, synthetic construct
  source 1..57: mol_type = other DNA
gaaattagattgaaatctaataattatgcaacacattatgcggagtctgtgaaaggg

SEQ ID NO: 11 - DNA, 18 bp, synthetic construct
  source 1..18: mol_type = other DNA
ctcccgtcctttgactac

SEQ ID NO: 12 - DNA, 351 bp, synthetic construct
  source 1..351: mol_type = other DNA
gaagtgaagcttgaggagtctggaggaggcttggtgcaacctggaggatccatgaaactctcctgtgttgcctctggattcactttcagtaattactggatgaactgggtccgccagtctccagagaaggggcttgagtgggttgctgaaattagattgaaatctaataattatgcaacacattatgcggagtctgtgaaagggaggttcaccatctcaagagatgattccaaaagtagtgtctacctgcaaatgaacaacttaagagctgaagacactggcatttattactgttccagactcccgtcctttgactactggggccaaggcaccactctcacagtctcctca

SEQ ID NO: 13 - DNA, 48 bp, synthetic construct
  source 1..48: mol_type = other DNA
aggtctactaagagtctcctgcatagtaatggcaacacttacttgtat

SEQ ID NO: 14 - DNA, 21 bp, synthetic construct
  source 1..21: mol_type = other DNA
cggatgtccaaccttgcctca

SEQ ID NO: 15 - DNA, 27 bp, synthetic construct
  source 1..27: mol_type = other DNA
atgcaacatctagaatatcctttcacg

SEQ ID NO: 16 - DNA, 339 bp, synthetic construct
  source 1..339: mol_type = other DNA
gatattgtgatgactcaggctgcaccctctgtacctgtcactcctggagagtcagtatccatctcctgcaggtctactaagagtctcctgcatagtaatggcaacacttacttgtattggttcctgcagaggccaggccagtctcctcagctcctgatatatcggatgtccaaccttgcctcaggagtcccagacaggttcagtggcagtgggtcaggaactgctttcacactgagaatcactagagtggaggctgaggatgtgggtatttattactgtatgcaacatctagaatatcctttcacgttcggtgctgggaccaagctggagctgaaacgg

SEQ ID NO: 17 - protein, 529 aa, Homo sapiens
MSQDTEVDMKEVELNELEPEKQPMNAASGAAMSLAGAEKNGLVKIKVAEDEAEAAAAAKFTGLSKEELLKVAGSPGWVRTRWALLLLFWLGWLGMLAGAVVIIVRAPRCRELPAQKWWHTGALYRIGDLQAFQGHGAGNLAGLKGRLDYLSSLKVKGLVLGPIHKNQKDDVAQTDLLQIDPNFGSKEDFDSLLQSAKKKSIRVILDLTPNYRGENSWFSTQVDTVATKVKDALEFWLQAGVDGFQVRDIENLKDASSFLAEWQNITKGFSEDRLLIAGTNSSDLQQILSLLESNKDLLLTSSYLSDSGSTGEHTKSLVTQYLNATGNRWCSWSLSQARLLTSFLPAQLLRLYQLMLFTLPGTPVFSYGDEIGLDAAALPGQPMEAPVMLWDESSFPDIPGAVSANMTVKGQSEDPGSLLSLFRRLSDQRSKERSLLHGDFHAFSAGPGLFSYIRHWDQNERFLVVLNFGDVGLSAGLQASDLPASASLPAKADLLLSTQPGREEGSPLELERLKLEPHEGLLLRFPYAA

SEQ ID NO: 18 - protein, 65 aa, Homo sapiens
FSYGDEIGLDAAALPGQPMEAPVMLWDESSFPDIPGAVSANMTVKGQSEDPGSLLSLFRRLSDQR

SEQ ID NO: 19 - protein, 45 aa, Homo sapiens
FSYGDEIGLDAAALPGQPMEAPVMLWDESSFPDIPGAVSANMTVK

SEQ ID NO: 20 - protein, 225 aa, Homo sapiens
VILDLTPNYRGENSWFSTQVDTVATKVKDALEFWLQAGVDGFQVRDIENLKDASSFLAEWQNITKGFSEDRLLIAGTNSSDLQQILSLLESNKDLLLTSSYLSDSGSTGEHTKSLVTQYLNATGNRWCSWSLSQARLLTSFLPAQLLRLYQLMLFTLPGTPVFSYGDEIGLDAAALPGQPMEAPVMLWDESSFPDIPGAVSANMTVKGQSEDPGSLLSLFRRLSD

SEQ ID NO: 21 - protein, 18 aa, synthetic construct
GSTSGSGKPGSGEGSTKG

SEQ ID NO: 22 - protein, 5 aa, synthetic construct
GGGGS

SEQ ID NO: 23 - protein, 21 aa, synthetic construct
LLLVTSLLLCELPHPAFLLIP

SEQ ID NO: 24 - protein, 117 aa, synthetic construct
EVKLEESGGGLVQPGGSMKLSCVASGFTFSNYWMNWVRQSPEKGLEWVAEIRLKSNNYATHYAESVKGRFTISRDDSKSSVYLQMNNLRAEDTGRYYCSRLPSFDYWGQGTTLTVSS

SEQ ID NO: 25 - protein, 113 aa, synthetic construct
DIVMTQAAPSVRVTPGESVSISCRSTKSLLHSNGNTYLYWFLQRPGQSPQLLIYRMSNLASGVPDRFSGSGSGTAFTLRITRVEAEDVGRYYCMQHLEYPFTFGAGTKLELKR

SEQ ID NO: 26 - skipped

SEQ ID NO: 27 - protein, 113 aa, synthetic construct
DIVMTQAAPSVQVTPGESVSISCRSTKSLLHSNGNTYLYWFLQRPGQSPQLLIYRMSNLASGVPDRFSGSGSGTAFTLRITRVEAEDVGRYYCMQHLEYPFTFGAGTKLELKR

SEQ ID NO: 28 - protein, 18 aa, synthetic construct
GSTSGSGKPGSGEGSTKG

SEQ ID NO: 29 - protein, 10 aa, synthetic construct
GGGGSGGGGS

SEQ ID NO: 30 - protein, 15 aa, synthetic construct
GGGGSGGGGSGGGGS

SEQ ID NO: 31 - protein, 20 aa, synthetic construct
GGGGSGGGGSGGGGSGGGGS

SEQ ID NO: 32 - protein, 25 aa, synthetic construct
GGGGSGGGGSGGGGSGGGGSGGGGS

SEQ ID NO: 33 - protein, 30 aa, synthetic construct
GGGGSGGGGSGGGGSGGGGSGGGGSGGGGS

SEQ ID NO: 34 - protein, 35 aa, synthetic construct
GGGGSGGGGSGGGGSGGGGSGGGGSGGGGSGGGGS

SEQ ID NO: 35 - protein, 40 aa, synthetic construct
GGGGSGGGGSGGGGSGGGGSGGGGSGGGGSGGGGSGGGGS

SEQ ID NO: 36 - protein, 50 aa, synthetic construct
GGGGSGGGGSGGGGSGGGGSGGGGSGGGGSGGGGSGGGGSGGGGSGGGGS

SEQ ID NO: 37 - protein, 39 aa, synthetic construct
IEVMYPPPYLDNEKSNGTIIHVKGKHLCPSPLFPGPSKP

SEQ ID NO: 38 - protein, 45 aa, synthetic construct
TTTPAPRPPTPAPTIASQPLSLRPEACRPAAGGAVHTRGLDFACD

SEQ ID NO: 39 - protein, 27 aa, synthetic construct
FWVLVVVGGVLACYSLLVTVAFIIFWV

SEQ ID NO: 40 - protein, 24 aa, synthetic construct
IYIWAPLAGTCGVLLLSLVITLYC

SEQ ID NO: 41 - protein, 41 aa, synthetic construct
RSKRSRLLHSDYMNMTPRRPGPTRKHYQPYAPPRDFAAYRS

SEQ ID NO: 42 - protein, 42 aa, synthetic construct
KRGRKKLLYIFKQPFMRPVQTTQEEDGCSCRFPEEEEGGCEL

SEQ ID NO: 43 - skipped

SEQ ID NO: 44 - protein, 112 aa, synthetic construct
RVKFSRSADAPAYQQGQNQLYNELNLGRREEYDVLDKRRGRDPEMGGKPRRKNPQEGLYNELQKDKMAEAYSEIGMKGERRRGKGHDGLYQGLSTATKDTYDALHMQALPPR

SEQ ID NO: 45 - DNA, 1479 bp, synthetic construct
  source 1..1479: mol_type = other DNA
atgcttctcctggtgacaagccttctgctctgtgagttaccacacccagcattcctcctgatcccagaagtgaagcttgaggagtctggaggaggcttggtgcaacctggaggatccatgaaactctcctgtgttgcctctggattcactttcagtaattactggatgaactgggtccgccagtctccagagaaggggcttgagtgggttgctgaaattagattgaaatctaataattatgcaacacattatgcggagtctgtgaaagggaggttcaccatctcaagagatgattccaaaagtagtgtctacctgcaaatgaacaacttaagagctgaagacactggcatttattactgttccagactcccgtcctttgactactggggccaaggcaccactctcacagtctcctcaggctccacctctggatccggcaagcccggatctggcgagggatccaccaagggcgatattgtgatgactcaggctgcaccctctgtacctgtcactcctggagagtcagtatccatctcctgcaggtctactaagagtctcctgcatagtaatggcaacacttacttgtattggttcctgcagaggccaggccagtctcctcagctcctgatatatcggatgtccaaccttgcctcaggagtcccagacaggttcagtggcagtgggtcaggaactgctttcacactgagaatcactagagtggaggctgaggatgtgggtatttattactgtatgcaacatctagaatatcctttcacgttcggtgctgggaccaagctggagctgaaacgggcggccgcaattgaagttatgtatcctcctccttacctagacaatgagaagagcaatggaaccattatccatgtgaaagggaaacacctttgtccaagtcccctatttcccggaccttctaagcccttttgggtgctggtggtggttggtggagtcctggcttgctatagcttgctagtaacagtggcctttattattttctgggtgaggagtaagaggagcaggctcctgcacagtgactacatgaacatgactccccgccgccccgggcccacccgcaagcattaccagccctatgccccaccacgcgacttcgcagcctatcgctccagagtgaagttcagcaggagcgcagacgcccccgcgtaccagcagggccagaaccagctctataacgagctcaatctaggacgaagagaggagtacgatgttttggacaagagacgtggccgggaccctgagatggggggaaagccgagaaggaagaaccctcaggaaggcctgtacaatgaactgcagaaagataagatggcggaggcctacagtgagattgggatgaaaggcgagcgccggaggggcaaggggcacgatggcctttaccagggtctcagtacagccaccaaggacacctacgacgcccttcacatgcaggccctgccccctcgctga

SEQ ID NO: 46 - DNA, 1479 bp, unidentified
  source 1..1479: mol_type = other DNA
atgcttctcctggtgacaagccttctgctctgtgagttaccacacccagcattcctcctgatcccagatattgtgatgactcaggctgcaccctctgtacctgtcactcctggagagtcagtatccatctcctgcaggtctactaagagtctcctgcatagtaatggcaacacttacttgtattggttcctgcagaggccaggccagtctcctcagctcctgatatatcggatgtccaaccttgcctcaggagtcccagacaggttcagtggcagtgggtcaggaactgctttcacactgagaatcactagagtggaggctgaggatgtgggtatttattactgtatgcaacatctagaatatcctttcacgttcggtgctgggaccaagctggagctgaaacggggctccacctctggatccggcaagcccggatctggcgagggatccaccaagggcgaagtgaagcttgaggagtctggaggaggcttggtgcaacctggaggatccatgaaactctcctgtgttgcctctggattcactttcagtaattactggatgaactgggtccgccagtctccagagaaggggcttgagtgggttgctgaaattagattgaaatctaataattatgcaacacattatgcggagtctgtgaaagggaggttcaccatctcaagagatgattccaaaagtagtgtctacctgcaaatgaacaacttaagagctgaagacactggcatttattactgttccagactcccgtcctttgactactggggccaaggcaccactctcacagtctcctcagcggccgcaattgaagttatgtatcctcctccttacctagacaatgagaagagcaatggaaccattatccatgtgaaagggaaacacctttgtccaagtcccctatttcccggaccttctaagcccttttgggtgctggtggtggttggtggagtcctggcttgctatagcttgctagtaacagtggcctttattattttctgggtgaggagtaagaggagcaggctcctgcacagtgactacatgaacatgactccccgccgccccgggcccacccgcaagcattaccagccctatgccccaccacgcgacttcgcagcctatcgctccagagtgaagttcagcaggagcgcagacgcccccgcgtaccagcagggccagaaccagctctataacgagctcaatctaggacgaagagaggagtacgatgttttggacaagagacgtggccgggaccctgagatggggggaaagccgagaaggaagaaccctcaggaaggcctgtacaatgaactgcagaaagataagatggcggaggcctacagtgagattgggatgaaaggcgagcgccggaggggcaaggggcacgatggcctttaccagggtctcagtacagccaccaaggacacctacgacgcccttcacatgcaggccctgccccctcgctga

SEQ ID NO: 47 - DNA, 1479 bp, synthetic construct; identical to SEQ ID NO: 45
  source 1..1479: mol_type = other DNA

SEQ ID NO: 48 - DNA, 1455 bp, synthetic construct
  source 1..1455: mol_type = other DNA
atgcttctcctggtgacaagccttctgctctgtgagttaccacacccagcattcctcctgatcccagaagtgaagcttgaggagtctggaggaggcttggtgcaacctggaggatccatgaaactctcctgtgttgcctctggattcactttcagtaattactggatgaactgggtccgccagtctccagagaaggggcttgagtgggttgctgaaattagattgaaatctaataattatgcaacacattatgcggagtctgtgaaagggaggttcaccatctcaagagatgattccaaaagtagtgtctacctgcaaatgaacaacttaagagctgaagacactggcatttattactgttccagactcccgtcctttgactactggggccaaggcaccactctcacagtctcctcaggaggtggcggttccggaggaggtggatcagatattgtgatgactcaggctgcaccctctgtacctgtcactcctggagagtcagtatccatctcctgcaggtctactaagagtctcctgcatagtaatggcaacacttacttgtattggttcctgcagaggccaggccagtctcctcagctcctgatatatcggatgtccaaccttgcctcaggagtcccagacaggttcagtggcagtgggtcaggaactgctttcacactgagaatcactagagtggaggctgaggatgtgggtatttattactgtatgcaacatctagaatatcctttcacgttcggtgctgggaccaagctggagctgaaacgggcggccgcaattgaagttatgtatcctcctccttacctagacaatgagaagagcaatggaaccattatccatgtgaaagggaaacacctttgtccaagtcccctatttcccggaccttctaagcccttttgggtgctggtggtggttggtggagtcctggcttgctatagcttgctagtaacagtggcctttattattttctgggtgaggagtaagaggagcaggctcctgcacagtgactacatgaacatgactccccgccgccccgggcccacccgcaagcattaccagccctatgccccaccacgcgacttcgcagcctatcgctccagagtgaagttcagcaggagcgcagacgcccccgcgtaccagcagggccagaaccagctctataacgagctcaatctaggacgaagagaggagtacgatgttttggacaagagacgtggccgggaccctgagatggggggaaagccgagaaggaagaaccctcaggaaggcctgtacaatgaactgcagaaagataagatggcggaggcctacagtgagattgggatgaaaggcgagcgccggaggggcaaggggcacgatggcctttaccagggtctcagtacagccaccaaggacacctacgacgcccttcacatgcaggccctgccccctcgctga

SEQ ID NO: 49 - DNA, 1470 bp, synthetic construct
  source 1..1470: mol_type = other DNA
atgcttctcctggtgacaagccttctgctctgtgagttaccacacccagcattcctcctgatcccagaagtgaagcttgaggagtctggaggaggcttggtgcaacctggaggatccatgaaactctcctgtgttgcctctggattcactttcagtaattactggatgaactgggtccgccagtctccagagaaggggcttgagtgggttgctgaaattagattgaaatctaataattatgcaacacattatgcggagtctgtgaaagggaggttcaccatctcaagagatgattccaaaagtagtgtctacctgcaaatgaacaacttaagagctgaagacactggcatttattactgttccagactcccgtcctttgactactggggccaaggcaccactctcacagtctcctcaggaggtggcggttccggaggaggtggatcaggaggcggaggctctgatattgtgatgactcaggctgcaccctctgtacctgtcactcctggagagtcagtatccatctcctgcaggtctactaagagtctcctgcatagtaatggcaacacttacttgtattggttcctgcagaggccaggccagtctcctcagctcctgatatatcggatgtccaaccttgcctcaggagtcccagacaggttcagtggcagtgggtcaggaactgctttcacactgagaatcactagagtggaggctgaggatgtgggtatttattactgtatgcaacatctagaatatcctttcacgttcggtgctgggaccaagctggagctgaaacgggcggccgcaattgaagttatgtatcctcctccttacctagacaatgagaagagcaatggaaccattatccatgtgaaagggaaacacctttgtccaagtcccctatttcccggaccttctaagcccttttgggtgctggtggtggttggtggagtcctggcttgctatagcttgctagtaacagtggcctttattattttctgggtgaggagtaagaggagcaggctcctgcacagtgactacatgaacatgactccccgccgccccgggcccacccgcaagcattaccagccctatgccccaccacgcgacttcgcagcctatcgctccagagtgaagttcagcaggagcgcagacgcccccgcgtaccagcagggccagaaccagctctataacgagctcaatctaggacgaagagaggagtacgatgttttggacaagagacgtggccgggaccctgagatggggggaaagccgagaaggaagaaccctcaggaaggcctgtacaatgaactgcagaaagataagatggcggaggcctacagtgagattgggatgaaaggcgagcgccggaggggcaaggggcacgatggcctttaccagggtctcagtacagccaccaaggacacctacgacgcccttcacatgcaggccctgccccctcgctga

SEQ ID NO: 50 - DNA, 1485 bp, synthetic construct
  source 1..1485: mol_type = other DNA
atgcttctcctggtgacaagccttctgctctgtgagttaccacacccagcattcctcctgatcccagaagtgaagcttgaggagtctggaggaggcttggtgcaacctggaggatccatgaaactctcctgtgttgcctctggattcactttcagtaattactggatgaactgggtccgccagtctccagagaaggggcttgagtgggttgctgaaattagattgaaatctaataattatgcaacacattatgcggagtctgtgaaagggaggttcaccatctcaagagatgattccaaaagtagtgtctacctgcaaatgaacaacttaagagctgaagacactggcatttattactgttccagactcccgtcctttgactactggggccaaggcaccactctcacagtctcctcaggaggtggcggttccggaggaggtggatcaggaggcggaggctctggtggcggtggctcagatattgtgatgactcaggctgcaccctctgtacctgtcactcctggagagtcagtatccatctcctgcaggtctactaagagtctcctgcatagtaatggcaacacttacttgtattggttcctgcagaggccaggccagtctcctcagctcctgatatatcggatgtccaaccttgcctcaggagtcccagacaggttcagtggcagtgggtcaggaactgctttcacactgagaatcactagagtggaggctgaggatgtgggtatttattactgtatgcaacatctagaatatcctttcacgttcggtgctgggaccaagctggagctgaaacgggcggccgcaattgaagttatgtatcctcctccttacctagacaatgagaagagcaatggaaccattatccatgtgaaagggaaacacctttgtccaagtcccctatttcccggaccttctaagcccttttgggtgctggtggtggttggtggagtcctggcttgctatagcttgctagtaacagtggcctttattattttctgggtgaggagtaagaggagcaggctcctgcacagtgactacatgaacatgactccccgccgccccgggcccacccgcaagcattaccagccctatgccccaccacgcgacttcgcagcctatcgctccagagtgaagttcagcaggagcgcagacgcccccgcgtaccagcagggccagaaccagctctataacgagctcaatctaggacgaagagaggagtacgatgttttggacaagagacgtggccgggaccctgagatggggggaaagccgagaaggaagaaccctcaggaaggcctgtacaatgaactgcagaaagataagatggcggaggcctacagtgagattgggatgaaaggcgagcgccggaggggcaaggggcacgatggcctttaccagggtctcagtacagccaccaaggacacctacgacgcccttcacatgcaggccctgccccctcgctga

SEQ ID NO: 51 - DNA, 1500 bp, synthetic construct
  source 1..1500: mol_type = other DNA
atgcttctcctggtgacaagccttctgctctgtgagttaccacacccagcattcctcctgatcccagaagtgaagcttgaggagtctggaggaggcttggtgcaacctggaggatccatgaaactctcctgtgttgcctctggattcactttcagtaattactggatgaactgggtccgccagtctccagagaaggggcttgagtgggttgctgaaattagattgaaatctaataattatgcaacacattatgcggagtctgtgaaagggaggttcaccatctcaagagatgattccaaaagtagtgtctacctgcaaatgaacaacttaagagctgaagacactggcatttattactgttccagactcccgtcctttgactactggggccaaggcaccactctcacagtctcctcaggaggtggcggttccggaggaggtggatcaggaggcggaggctctggtggcggtggctcaggtggaggcggctcagatattgtgatgactcaggctgcaccctctgtacctgtcactcctggagagtcagtatccatctcctgcaggtctactaagagtctcctgcatagtaatggcaacacttacttgtattggttcctgcagaggccaggccagtctcctcagctcctgatatatcggatgtccaaccttgcctcaggagtcccagacaggttcagtggcagtgggtcaggaactgctttcacactgagaatcactagagtggaggctgaggatgtgggtatttattactgtatgcaacatctagaatatcctttcacgttcggtgctgggaccaagctggagctgaaacgggcggccgcaattgaagttatgtatcctcctccttacctagacaatgagaagagcaatggaaccattatccatgtgaaagggaaacacctttgtccaagtcccctatttcccggaccttctaagcccttttgggtgctggtggtggttggtggagtcctggcttgctatagcttgctagtaacagtggcctttattattttctgggtgaggagtaagaggagcaggctcctgcacagtgactacatgaacatgactccccgccgccccgggcccacccgcaagcattaccagccctatgccccaccacgcgacttcgcagcctatcgctccagagtgaagttcagcaggagcgcagacgcccccgcgtaccagcagggccagaaccagctctataacgagctcaatctaggacgaagagaggagtacgatgttttggacaagagacgtggccgggaccctgagatggggggaaagccgagaaggaagaaccctcaggaaggcctgtacaatgaactgcagaaagataagatggcggaggcctacagtgagattgggatgaaaggcgagcgccggaggggcaaggggcacgatggcctttaccagggtctcagtacagccaccaaggacacctacgacgcccttcacatgcaggccctgccccctcgctga

SEQ ID NO: 52 - DNA, 1485 bp, synthetic construct; identical to SEQ ID NO: 50
  source 1..1485: mol_type = other DNA

SEQ ID NO: 53 - DNA, 1500 bp, synthetic construct; identical to SEQ ID NO: 51
  source 1..1500: mol_type = other DNA

SEQ ID NO: 54 - DNA, 1515 bp, synthetic construct
  source 1..1515: mol_type = other DNA
atgcttctcctggtgacaagccttctgctctgtgagttaccacacccagcattcctcctgatcccagaagtgaagcttgaggagtctggaggaggcttggtgcaacctggaggatccatgaaactctcctgtgttgcctctggattcactttcagtaattactggatgaactgggtccgccagtctccagagaaggggcttgagtgggttgctgaaattagattgaaatctaataattatgcaacacattatgcggagtctgtgaaagggaggttcaccatctcaagagatgattccaaaagtagtgtctacctgcaaatgaacaacttaagagctgaagacactggcatttattactgttccagactcccgtcctttgactactggggccaaggcaccactctcacagtctcctcaggaggtggcggttccggaggaggtggatcaggaggtggcggttccggaggaggtggatcaggaggtggcggttccggaggaggtggatcagatattgtgatgactcaggctgcaccctctgtacctgtcactcctggagagtcagtatccatctcctgcaggtctactaagagtctcctgcatagtaatggcaacacttacttgtattggttcctgcagaggccaggccagtctcctcagctcctgatatatcggatgtccaaccttgcctcaggagtcccagacaggttcagtggcagtgggtcaggaactgctttcacactgagaatcactagagtggaggctgaggatgtgggtatttattactgtatgcaacatctagaatatcctttcacgttcggtgctgggaccaagctggagctgaaacgggcagccgcaattgaagttatgtatcctcctccttacctagacaatgagaagagcaatggaaccattatccatgtgaaagggaaacacctttgtccaagtcccctatttcccggaccttctaagcccttttgggtgctggtggtggttggtggagtcctggcttgctatagcttgctagtaacagtggcctttattattttctgggtgaggagtaagaggagcaggctcctgcacagtgactacatgaacatgactccccgccgccccgggcccacccgcaagcattaccagccctatgccccaccacgcgacttcgcagcctatcgctccagagtgaagttcagcaggagcgcagacgcccccgcgtaccagcagggccagaaccagctctataacgagctcaatctaggacgaagagaggagtacgatgttttggacaagagacgtggccgggaccctgagatggggggaaagccgagaaggaagaaccctcaggaaggcctgtacaatgaactgcagaaagataagatggcggaggcctacagtgagattgggatgaaaggcgagcgccggaggggcaaggggcacgatggcctttaccagggtctcagtacagccaccaaggacacctacgacgcccttcacatgcaggccctgccccctcgctga

SEQ ID NO: 55 - DNA, 1530 bp, synthetic construct
  source 1..1530: mol_type = other DNA
atgcttctcctggtgacaagccttctgctctgtgagttaccacacccagcattcctcctgatcccagaagtgaagcttgaggagtctggaggaggcttggtgcaacctggaggatccatgaaactctcctgtgttgcctctggattcactttcagtaattactggatgaactgggtccgccagtctccagagaaggggcttgagtgggttgctgaaattagattgaaatctaataattatgcaacacattatgcggagtctgtgaaagggaggttcaccatctcaagagatgattccaaaagtagtgtctacctgcaaatgaacaacttaagagctgaagacactggcatttattactgttccagactcccgtcctttgactactggggccaaggcaccactctcacagtctcctcaggaggtggcggttccggaggaggtggatcaggaggtggcggttccggaggaggtggatcaggaggtggcggttccggaggaggtggatcaggaggaggtggatcagatattgtgatgactcaggctgcaccctctgtacctgtcactcctggagagtcagtatccatctcctgcaggtctactaagagtctcctgcatagtaatggcaacacttacttgtattggttcctgcagaggccaggccagtctcctcagctcctgatatatcggatgtccaaccttgcctcaggagtcccagacaggttcagtggcagtgggtcaggaactgctttcacactgagaatcactagagtggaggctgaggatgtgggtatttattactgtatgcaacatctagaatatcctttcacgttcggtgctgggaccaagctggagctgaaacgggcagccgcaattgaagttatgtatcctcctccttacctagacaatgagaagagcaatggaaccattatccatgtgaaagggaaacacctttgtccaagtcccctatttcccggaccttctaagcccttttgggtgctggtggtggttggtggagtcctggcttgctatagcttgctagtaacagtggcctttattattttctgggtgaggagtaagaggagcaggctcctgcacagtgactacatgaacatgactccccgccgccccgggcccacccgcaagcattaccagccctatgccccaccacgcgacttcgcagcctatcgctccagagtgaagttcagcaggagcgcagacgcccccgcgtaccagcagggccagaaccagctctataacgagctcaatctaggacgaagagaggagtacgatgttttggacaagagacgtggccgggaccctgagatggggggaaagccgagaaggaagaaccctcaggaaggcctgtacaatgaactgcagaaagataagatggcggaggcctacagtgagattgggatgaaaggcgagcgccggaggggcaaggggcacgatggcctttaccagggtctcagtacagccaccaaggacacctacgacgcccttcacatgcaggccctgccccctcgctga

SEQ ID NO: 56 - DNA, 1545 bp, synthetic construct
  source 1..1545: mol_type = other DNA
atgcttctcctggtgacaagccttctgctctgtgagttaccacacccagcattcctcctgatcccagaagtgaagcttgaggagtctggaggaggcttggtgcaacctggaggatccatgaaactctcctgtgttgcctctggattcactttcagtaattactggatgaactgggtccgccagtctccagagaaggggcttgagtgggttgctgaaattagattgaaatctaataattatgcaacacattatgcggagtctgtgaaagggaggttcaccatctcaagagatgattccaaaagtagtgtctacctgcaaatgaacaacttaagagctgaagacactggcatttattactgttccagactcccgtcctttgactactggggccaaggcaccactctcacagtctcctcaggaggtggcggttccggaggaggtggatcaggaggtggcggttccggaggaggtggatcaggaggtggcggttccggaggaggtggatcaggaggaggtggatcaggaggaggtggatcagatattgtgatgactcaggctgcaccctctgtacctgtcactcctggagagtcagtatccatctcctgcaggtctactaagagtctcctgcatagtaatggcaacacttacttgtattggttcctgcagaggccaggccagtctcctcagctcctgatatatcggatgtccaaccttgcctcaggagtcccagacaggttcagtggcagtgggtcaggaactgctttcacactgagaatcactagagtggaggctgaggatgtgggtatttattactgtatgcaacatctagaatatcctttcacgttcggtgctgggaccaagctggagctgaaacgggcagccgcaattgaagttatgtatcctcctccttacctagacaatgagaagagcaatggaaccattatccatgtgaaagggaaacacctttgtccaagtcccctatttcccggaccttctaagcccttttgggtgctggtggtggttggtggagtcctggcttgctatagcttgctagtaacagtggcctttattattttctgggtgaggagtaagaggagcaggctcctgcacagtgactacatgaacatgactccccgccgccccgggcccacccgcaagcattaccagccctatgccccaccacgcgacttcgcagcctatcgctccagagtgaagttcagcaggagcgcagacgcccccgcgtaccagcagggccagaaccagctctataacgagctcaatctaggacgaagagaggagtacgatgttttggacaagagacgtggccgggaccctgagatggggggaaagccgagaaggaagaaccctcaggaaggcctgtacaatgaactgcagaaagataagatggcggaggcctacagtgagattgggatgaaaggcgagcgccggaggggcaaggggcacgatggcctttaccagggtctcagtacagccaccaaggacacctacgacgcccttcacatgcaggccctgccccctcgctga

SEQ ID NO: 57 - DNA, 1575 bp, synthetic construct
  source 1..1575: mol_type = other DNA
atgcttctcctggtgacaagccttctgctctgtgagttaccacacccagcattcctcctgatcccagaagtgaagcttgaggagtctggaggaggcttggtgcaacctggaggatccatgaaactctcctgtgttgcctctggattcactttcagtaattactggatgaactgggtccgccagtctccagagaaggggcttgagtgggttgctgaaattagattgaaatctaataattatgcaacacattatgcggagtctgtgaaagggaggttcaccatctcaagagatgattccaaaagtagtgtctacctgcaaatgaacaacttaagagctgaagacactggcatttattactgttccagactcccgtcctttgactactggggccaaggcaccactctcacagtctcctcaggaggtggcggttccggaggaggtggatcaggaggtggcggttccggaggaggtggatcaggaggtggcggttccggaggaggtggatcaggaggaggtggatcaggaggaggtggatcaggaggaggtggatcaggaggaggtggatcagatattgtgatgactcaggctgcaccctctgtacctgtcactcctggagagtcagtatccatctcctgcaggtctactaagagtctcctgcatagtaatggcaacacttacttgtattggttcctgcagaggccaggccagtctcctcagctcctgatatatcggatgtccaaccttgcctcaggagtcccagacaggttcagtggcagtgggtcaggaactgctttcacactgagaatcactagagtggaggctgaggatgtgggtatttattactgtatgcaacatctagaatatcctttcacgttcggtgctgggaccaagctggagctgaaacgggcagccgcaattgaagttatgtatcctcctccttacctagacaatgagaagagcaatggaaccattatccatgtgaaagggaaacacctttgtccaagtcccctatttcccggaccttctaagcccttttgggtgctggtggtggttggtggagtcctggcttgctatagcttgctagtaacagtggcctttattattttctgggtgaggagtaagaggagcaggctcctgcacagtgactacatgaacatgactccccgccgccccgggcccacccgcaagcattaccagccctatgccccaccacgcgacttcgcagcctatcgctccagagtgaagttcagcaggagcgcagacgcccccgcgtaccagcagggccagaaccagctctataacgagctcaatctaggacgaagagaggagtacgatgttttggacaagagacgtggccgggaccctgagatggggggaaagccgagaaggaagaaccctcaggaaggcctgtacaatgaactgcagaaagataagatggcggaggcctacagtgagattgggatgaaaggcgagcgccggaggggcaaggggcacgatggcctttaccagggtctcagtacagccaccaaggacacctacgacgcccttcacatgcaggccctgccccctcgctga

SEQ ID NO: 58 - DNA, 1479 bp, synthetic construct
  source 1..1479: mol_type = other DNA
atgctgttgctggtcaccagcctcctcttgtgtgagcttcctcatccagcctttcttctgattcccgaagtcaaactcgaggagtctggcggtgggttggtgcagccaggtggctccatgaagctgtcatgtgtcgcaagcggcttcacgttctcaaactactggatgaattgggtgagacaatcacccgagaaggggctggaatgggtggcagaaatccgtctgaaaagcaacaactatgctacccattacgcggagtctgtgaagggtcggttcacaattagccgcgacgacagcaagtccagtgtctatctccagatgaacaacctccgagccgaggatactggaaggtactattgcagcagactgcctagcttcgattactggggccaaggcactactttgacagtgtcctcagggagtaccagcgggtccggtaaaccaggctcaggagaaggttccacgaaaggggacattgtgatgacacaggctgctcctagcgttcgggtgacacctggagagagcgtaagtatcagctgcagaagcaccaagtctctcctgcactctaatggcaatacctacctgtactggttccttcagcggccagggcagtctcctcagcttctgatataccgcatgtctaatctggcgtcaggggtacctgacagattctcagggtctggaagcggaaccgcctttactctgcggattacacgggtggaagctgaggatgttgggcgctattactgcatgcagcacttggagtatccgttcacttttggcgcgggtacaaagctggaactcaaaagagcagccgctatcgaggtgatgtatccacctccctatctggacaacgagaaatccaacggcaccataatccacgtgaaaggcaagcatctgtgtccctctcccctgtttcccgggccgagtaaaccgttttgggttctggtggtagtgggcggtgtcctggcttgctattccctgcttgtcacggtggcctttatcatcttctgggttcgatccaaaaggagcagactgctgcattccgactacatgaatatgactccaagacgccctggaccaacacggaagcactaccaaccgtatgcaccaccccgcgactttgcagcctacaggtctagggtcaagttctcccgcagtgccgatgctcccgcctatcagcaagggcagaatcagctgtacaacgagctcaatctgggacgtcgtgaggaatacgacgttctcgacaagaggcgaggacgggatcccgaaatgggaggcaaacccaggcgcaagaatcctcaagaaggcctgtacaacgaactgcagaaggacaagatggccgaagcttacagtgagattggcatgaagggagagagaaggcgaggcaaaggccacgatggtctttatcagggactgagtaccgccactaaggatacctatgatgccctccacatgcaggcattgccacccaggtga

SEQ ID NO: 59 - DNA, 1479 bp, synthetic construct
  source 1..1479: mol_type = other DNA
atgttgttgctcgtcacctctcttctgctgtgtgagctccctcatccggccttcctgcttatccccgaagttaagctcgaggagtccggaggagggctggtccagcccggaggtagtatgaagctgtcatgcgtagcctccggcttcacattcagcaattactggatgaactgggtcagacagagtcccgagaaaggtctggaatgggtggccgaaatacggctgaagagcaataactatgccacacattacgcagagtcagtcaagggccgtttcaccattagcagagatgactccaagagtagcgtgtatctgcagatgaacaacctcagggctgaggacactggtcgctactactgctctagactgccctcctttgactactggggacaaggcaccactctgactgtctcaagtgggagcacatctggaagtggcaaacctgggtctggggaaggcagcactaaaggtgatatcgtgatgacacaggcagctccctccgtccaagtgacaccaggcgaatctgtcagcatttcttgtcggtccactaagtctctccttcactctaacgggaatacctacctctactggttcctgcaacgaccaggacaatccccacagctgctcatctatcggatgagcaatctcgccagtggggtgcctgatcggtttagcggtagcggctctggtacggcatttaccctgcgcattacacgcgttgaagcagaggatgttgggagatactattgcatgcagcacctggaatatccctttaccttcggcgctggcacgaagctcgagctgaagagggctgccgctattgaggtgatgtaccctcctccctacctggacaacgagaaaagcaatggaaccatcattcacgtaaaaggcaagcatctgtgtccgtcaccactgtttccggggccaagtaaacccttttgggtgttggtggttgttggtggggtactcgcgtgctattccctgcttgtgaccgtggccttcatcatcttctgggtgcgctcaaagcgatccagacttctgcatagcgactacatgaacatgactcccaggcgccctgggccaacacgtaagcactatcagccctatgctcctccacgggattttgccgcatacagatccagagtgaagttctcaaggagcgctgatgctccggcctatcagcagggccagaatcagctgtacaatgagctgaatcttggaaggagagaggaatacgacgtgttggacaaacgccgaggaagggaccctgaaatgggtggcaaaccacggaggaagaaccctcaggaaggactgtataacgagctgcagaaagataagatggcggaggcgtactcagagataggcatgaagggagaacgccgtcgaggcaaaggccacgatggcctgtatcaggggttgagcactgccacgaaagacacctatgacgcactgcacatgcaagccttgccaccccggtga

SEQ ID NO: 60 - DNA, 1461 bp, synthetic construct
  source 1..1461: mol_type = other DNA
atggccttaccagtgaccgccttgctcctgccgctggccttgctgctccacgccgccaggccggacatccagatgacacagactacatcctccctgtctgcctctctgggagacagagtcaccatcagttgcagggcaagtcaggacattagtaaatatttaaattggtatcagcagaaaccagatggaactgttaaactcctgatctaccatacatcaagattacactcaggagtcccatcaaggttcagtggcagtgggtctggaacagattattctctcaccattagcaacctggagcaagaagatattgccacttacttttgccaacagggtaatacgcttccgtacacgttcggaggggggaccaagctggagatcacaggtggcggtggctcgggcggtggtgggtcgggtggcggcggatctgaggtgaaactgcaggagtcaggacctggcctggtggcgccctcacagagcctgtccgtcacatgcactgtctcaggggtctcattacccgactatggtgtaagctggattcgccagcctccacgaaagggtctggagtggctgggagtaatatggggtagtgaaaccacatactataattcagctctcaaatccagactgaccatcatcaaggacaactccaagagccaagttttcttaaaaatgaacagtctgcaaactgatgacacagccatttactactgtgccaaacattattactacggtggtagctatgctatggactactggggccaaggaacctcagtcaccgtctcctcaaccacgacgccagcgccgcgaccaccaacaccggcgcccaccatcgcgtcgcagcccctgtccctgcgcccagaggcgtgccggccagcggcggggggcgcagtgcacacgagggggctggacttcgcctgtgatatctacatctgggcgcccttggccgggacttgtggggtccttctcctgtcactggttatcaccctttactgcaaacggggcagaaagaaactcctgtatatattcaaacaaccatttatgagaccagtacaaactactcaagaggaagatggctgtagctgccgatttccagaagaagaagaaggaggatgtgaactgagagtgaagttcagcaggagcgcagacgcccccgcgtacaagcagggccagaaccagctctataacgagctcaatctaggacgaagagaggagtacgatgttttggacaagagacgtggccgggaccctgagatggggggaaagccgagaaggaagaaccctcaggaaggcctgtacaatgaactgcagaaagataagatggcggaggcctacagtgagattgggatgaaaggcgagcgccggaggggcaaggggcacgatggcctttaccagggtctcagtacagccaccaaggacacctacgacgcccttcacatgcaggccctgccccctcgctaa

SEQ ID NO: 61 - DNA, 1470 bp, synthetic construct
  source 1..1470: mol_type = other DNA
atgcttctcctggtgacaagccttctgctctgtgagttaccacacccagcattcctcctgatcccagaagtgaagcttgaggagtctggaggaggcttggtgcaacctggaggatccatgaaactctcctgtgttgcctctggattcactttcagtaattactggatgaactgggtccgccagtctccagagaaggggcttgagtgggttgctgaaattagattgaaatctaataattatgcaacacattatgcggagtctgtgaaagggaggttcaccatctcaagagatgattccaaaagtagtgtctacctgcaaatgaacaacttaagagctgaagacactggcatttattactgttccagactcccgtcctttgactactggggccaaggcaccactctcacagtctcctcaggctccacctctggatccggcaagcccggatctggcgagggatccaccaagggcgatattgtgatgactcaggctgcaccctctgtacctgtcactcctggagagtcagtatccatctcctgcaggtctactaagagtctcctgcatagtaatggcaacacttacttgtattggttcctgcagaggccaggccagtctcctcagctcctgatatatcggatgtccaaccttgcctcaggagtcccagacaggttcagtggcagtgggtcaggaactgctttcacactgagaatcactagagtggaggctgaggatgtgggtatttattactgtatgcaacatctagaatatcctttcacgttcggtgctgggaccaagctggagctgaaacggattgaagttatgtatcctcctccttacctagacaatgagaagagcaatggaaccattatccatgtgaaagggaaacacctttgtccaagtcccctatttcccggaccttctaagcccttttgggtgctggtggtggttggtggagtcctggcttgctatagcttgctagtaacagtggcctttattattttctgggtgaggagtaagaggagcaggctcctgcacagtgactacatgaacatgactccccgccgccccgggcccacccgcaagcattaccagccctatgccccaccacgcgacttcgcagcctatcgctccagagtgaagttcagcaggagcgcagacgcccccgcgtaccagcagggccagaaccagctctataacgagctcaatctaggacgaagagaggagtacgatgttttggacaagagacgtggccgggaccctgagatggggggaaagccgagaaggaagaaccctcaggaaggcctgtacaatgaactgcagaaagataagatggcggaggcctacagtgagattgggatgaaaggcgagcgccggaggggcaaggggcacgatggcctttaccagggtctcagtacagccaccaaggacacctacgacgcccttcacatgcaggccctgccccctcgctga

SEQ ID NO: 62 - DNA, 1482 bp, synthetic construct
  source 1..1482: mol_type = other DNA
atgcttctcctggtgacaagccttctgctctgtgagttaccacacccagcattcctcctgatcccagaagtgaagcttgaggagtctggaggaggcttggtgcaacctggaggatccatgaaactctcctgtgttgcctctggattcactttcagtaattactggatgaactgggtccgccagtctccagagaaggggcttgagtgggttgctgaaattagattgaaatctaataattatgcaacacattatgcggagtctgtgaaagggaggttcaccatctcaagagatgattccaaaagtagtgtctacctgcaaatgaacaacttaagagctgaagacactggcatttattactgttccagactcccgtcctttgactactggggccaaggcaccactctcacagtctcctcaggctccacctctggatccggcaagcccggatctggcgagggatccaccaagggcgatattgtgatgactcaggctgcaccctctgtacctgtcactcctggagagtcagtatccatctcctgcaggtctactaagagtctcctgcatagtaatggcaacacttacttgtattggttcctgcagaggccaggccagtctcctcagctcctgatatatcggatgtccaaccttgcctcaggagtcccagacaggttcagtggcagtgggtcaggaactgctttcacactgagaatcactagagtggaggctgaggatgtgggtatttattactgtatgcaacatctagaatatcctttcacgttcggtgctgggaccaagctggagctgaaacggaccacgacgccagcgccgcgaccaccaacaccggcgcccaccatcgcgtcgcagcccctgtccctgcgcccagaggcgtgccggccagcggcggggggcgcagtgcacacgagggggctggacttcgcctgtgatatctacatctgggcgcccttggccgggacttgtggggtccttctcctgtcactggttatcaccctttactgcaaacggggcagaaagaaactcctgtatatattcaaacaaccatttatgagaccagtacaaactactcaagaggaagatggctgtagctgccgatttccagaagaagaagaaggaggatgtgaactgagagtgaagttcagcaggagcgcagacgcccccgcgtaccagcagggccagaaccagctctataacgagctcaatctaggacgaagagaggagtacgatgttttggacaagagacgtggccgggaccctgagatggggggaaagccgagaaggaagaaccctcaggaaggcctgtacaatgaactgcagaaagataagatggcggaggcctacagtgagattgggatgaaaggcgagcgccggaggggcaaggggcacgatggcctttaccagggtctcagtacagccaccaaggacacctacgacgcccttcacatgcaggccctgccccctcgctga

SEQ ID NO: 63 - DNA, 1614 bp, synthetic construct
  source 1..1614: mol_type = other DNA
atgcttctcctggtgacaagccttctgctctgtgagttaccacacccagcattcctcctgatcccagaagtgaagcttgaggagtctggaggaggcttggtgcaacctggaggatccatgaaactctcctgtgttgcctctggattcactttcagtaattactggatgaactgggtccgccagtctccagagaaggggcttgagtgggttgctgaaattagattgaaatctaataattatgcaacacattatgcggagtctgtgaaagggaggttcaccatctcaagagatgattccaaaagtagtgtctacctgcaaatgaacaacttaagagctgaagacactggcatttattactgttccagactcccgtcctttgactactggggccaaggcaccactctcacagtctcctcaggctccacctctggatccggcaagcccggatctggcgagggatccaccaagggcgatattgtgatgactcaggctgcaccctctgtacctgtcactcctggagagtcagtatccatctcctgcaggtctactaagagtctcctgcatagtaatggcaacacttacttgtattggttcctgcagaggccaggccagtctcctcagctcctgatatatcggatgtccaaccttgcctcaggagtcccagacaggttcagtggcagtgggtcaggaactgctttcacactgagaatcactagagtggaggctgaggatgtgggtatttattactgtatgcaacatctagaatatcctttcacgttcggtgctgggaccaagctggagctgaaacggaccacgacgccagcgccgcgaccaccaacaccggcgcccaccatcgcgtcgcagcccctgtccctgcgcccagaggcgtgccggccagcggcggggggcgcagtgcacacgagggggctggacttcgcctgtgatttttgggtgctggtggtggttggtggagtcctggcttgctatagcttgctagtaacagtggcctttattattttctgggtgaggagtaagaggagcaggctcctgcacagtgactacatgaacatgactccccgccgccccgggcccacccgcaagcattaccagccctatgccccaccacgcgacttcgcagcctatcgctccaaacggggcagaaagaaactcctgtatatattcaaacaaccatttatgagaccagtacaaactactcaagaggaagatggctgtagctgccgatttccagaagaagaagaaggaggatgtgaactgagagtgaagttcagcaggagcgcagacgcccccgcgtaccagcagggccagaaccagctctataacgagctcaatctaggacgaagagaggagtacgatgttttggacaagagacgtggccgggaccctgagatggggggaaagccgagaaggaagaaccctcaggaaggcctgtacaatgaactgcagaaagataagatggcggaggcctacagtgagattgggatgaaaggcgagcgccggaggggcaaggggcacgatggcctttaccagggtctcagtacagccaccaaggacacctacgacgcccttcacatgcaggccctgccccctcgctga

SEQ ID NO: 64 - DNA, 1476 bp, synthetic construct
  source 1..1476: mol_type = other DNA
atgcttctcctggtgacaagccttctgctctgtgagttaccacacccagcattcctcctgatcccagaagtgaagcttgaggagtctggaggaggcttggtgcaacctggaggatccatgaaactctcctgtgttgcctctggattcactttcagtaattactggatgaactgggtccgccagtctccagagaaggggcttgagtgggttgctgaaattagattgaaatctaataattatgcaacacattatgcggagtctgtgaaagggaggttcaccatctcaagagatgattccaaaagtagtgtctacctgcaaatgaacaacttaagagctgaagacactggcatttattactgttccagactcccgtcctttgactactggggccaaggcaccactctcacagtctcctcaggaggtggcggttccggaggaggtggatcaggaggcggaggctctggtggcggtggctcagatattgtgatgactcaggctgcaccctctgtacctgtcactcctggagagtcagtatccatctcctgcaggtctactaagagtctcctgcatagtaatggcaacacttacttgtattggttcctgcagaggccaggccagtctcctcagctcctgatatatcggatgtccaaccttgcctcaggagtcccagacaggttcagtggcagtgggtcaggaactgctttcacactgagaatcactagagtggaggctgaggatgtgggtatttattactgtatgcaacatctagaatatcctttcacgttcggtgctgggaccaagctggagctgaaacggattgaagttatgtatcctcctccttacctagacaatgagaagagcaatggaaccattatccatgtgaaagggaaacacctttgtccaagtcccctatttcccggaccttctaagcccttttgggtgctggtggtggttggtggagtcctggcttgctatagcttgctagtaacagtggcctttattattttctgggtgaggagtaagaggagcaggctcctgcacagtgactacatgaacatgactccccgccgccccgggcccacccgcaagcattaccagccctatgccccaccacgcgacttcgcagcctatcgctccagagtgaagttcagcaggagcgcagacgcccccgcgtaccagcagggccagaaccagctctataacgagctcaatctaggacgaagagaggagtacgatgttttggacaagagacgtggccgggaccctgagatggggggaaagccgagaaggaagaaccctcaggaaggcctgtacaatgaactgcagaaagataagatggcggaggcctacagtgagattgggatgaaaggcgagcgccggaggggcaaggggcacgatggcctttaccagggtctcagtacagccaccaaggacacctacgacgcccttcacatgcaggccctgccccctcgctga

SEQ ID NO: 65 - DNA, 1488 bp, synthetic construct
  source 1..1488: mol_type = other DNA
atgcttctcctggtgacaagccttctgctctgtgagttaccacacccagcattcctcctgatcccagaagtgaagcttgaggagtctggaggaggcttggtgcaacctggaggatccatgaaactctcctgtgttgcctctggattcactttcagtaattactggatgaactgggtccgccagtctccagagaaggggcttgagtgggttgctgaaattagattgaaatctaataattatgcaacacattatgcggagtctgtgaaagggaggttcaccatctcaagagatgattccaaaagtagtgtctacctgcaaatgaacaacttaagagctgaagacactggcatttattactgttccagactcccgtcctttgactactggggccaaggcaccactctcacagtctcctcaggaggtggcggttccggaggaggtggatcaggaggcggaggctctggtggcggtggctcagatattgtgatgactcaggctgcaccctctgtacctgtcactcctggagagtcagtatccatctcctgcaggtctactaagagtctcctgcatagtaatggcaacacttacttgtattggttcctgcagaggccaggccagtctcctcagctcctgatatatcggatgtccaaccttgcctcaggagtcccagacaggttcagtggcagtgggtcaggaactgctttcacactgagaatcactagagtggaggctgaggatgtgggtatttattactgtatgcaacatctagaatatcctttcacgttcggtgctgggaccaagctggagctgaaacggaccacgacgccagcgccgcgaccaccaacaccggcgcccaccatcgcgtcgcagcccctgtccctgcgcccagaggcgtgccggccagcggcggggggcgcagtgcacacgagggggctggacttcgcctgtgatatctacatctgggcgcccttggccgggacttgtggggtccttctcctgtcactggttatcaccctttactgcaaacggggcagaaagaaactcctgtatatattcaaacaaccatttatgagaccagtacaaactactcaagaggaagatggctgtagctgccgatttccagaagaagaagaaggaggatgtgaactgagagtgaagttcagcaggagcgcagacgcccccgcgtaccagcagggccagaaccagctctataacgagctcaatctaggacgaagagaggagtacgatgttttggacaagagacgtggccgggaccctgagatggggggaaagccgagaaggaagaaccctcaggaaggcctgtacaatgaactgcagaaagataagatggcggaggcctacagtgagattgggatgaaaggcgagcgccggaggggcaaggggcacgatggcctttaccagggtctcagtacagccaccaaggacacctacgacgcccttcacatgcaggccctgccccctcgctga

SEQ ID NO: 66 - DNA, 1620 bp, synthetic construct
  source 1..1620: mol_type = other DNA
atgcttctcctggtgacaagccttctgctctgtgagttaccacacccagcattcctcctgatcccagaagtgaagcttgaggagtctggaggaggcttggtgcaacctggaggatccatgaaactctcctgtgttgcctctggattcactttcagtaattactggatgaactgggtccgccagtctccagagaaggggcttgagtgggttgctgaaattagattgaaatctaataattatgcaacacattatgcggagtctgtgaaagggaggttcaccatctcaagagatgattccaaaagtagtgtctacctgcaaatgaacaacttaagagctgaagacactggcatttattactgttccagactcccgtcctttgactactggggccaaggcaccactctcacagtctcctcaggaggtggcggttccggaggaggtggatcaggaggcggaggctctggtggcggtggctcagatattgtgatgactcaggctgcaccctctgtacctgtcactcctggagagtcagtatccatctcctgcaggtctactaagagtctcctgcatagtaatggcaacacttacttgtattggttcctgcagaggccaggccagtctcctcagctcctgatatatcggatgtccaaccttgcctcaggagtcccagacaggttcagtggcagtgggtcaggaactgctttcacactgagaatcactagagtggaggctgaggatgtgggtatttattactgtatgcaacatctagaatatcctttcacgttcggtgctgggaccaagctggagctgaaacggaccacgacgccagcgccgcgaccaccaacaccggcgcccaccatcgcgtcgcagcccctgtccctgcgcccagaggcgtgccggccagcggcggggggcgcagtgcacacgagggggctggacttcgcctgtgatttttgggtgctggtggtggttggtggagtcctggcttgctatagcttgctagtaacagtggcctttattattttctgggtgaggagtaagaggagcaggctcctgcacagtgactacatgaacatgactccccgccgccccgggcccacccgcaagcattaccagccctatgccccaccacgcgacttcgcagcctatcgctccaaacggggcagaaagaaactcctgtatatattcaaacaaccatttatgagaccagtacaaactactcaagaggaagatggctgtagctgccgatttccagaagaagaagaaggaggatgtgaactgagagtgaagttcagcaggagcgcagacgcccccgcgtaccagcagggccagaaccagctctataacgagctcaatctaggacgaagagaggagtacgatgttttggacaagagacgtggccgggaccctgagatggggggaaagccgagaaggaagaaccctcaggaaggcctgtacaatgaactgcagaaagataagatggcggaggcctacagtgagattgggatgaaaggcgagcgccggaggggcaaggggcacgatggcctttaccagggtctcagtacagccaccaaggacacctacgacgcccttcacatgcaggccctgccccctcgctga

SEQ ID NO: 67 - DNA, 1491 bp, synthetic construct
  source 1..1491: mol_type = other DNA
atgcttctcctggtgacaagccttctgctctgtgagttaccacacccagcattcctcctgatcccagaagtgaagcttgaggagtctggaggaggcttggtgcaacctggaggatccatgaaactctcctgtgttgcctctggattcactttcagtaattactggatgaactgggtccgccagtctccagagaaggggcttgagtgggttgctgaaattagattgaaatctaataattatgcaacacattatgcggagtctgtgaaagggaggttcaccatctcaagagatgattccaaaagtagtgtctacctgcaaatgaacaacttaagagctgaagacactggcatttattactgttccagactcccgtcctttgactactggggccaaggcaccactctcacagtctcctcaggaggtggcggttccggaggaggtggatcaggaggcggaggctctggtggcggtggctcaggtggaggcggctcagatattgtgatgactcaggctgcaccctctgtacctgtcactcctggagagtcagtatccatctcctgcaggtctactaagagtctcctgcatagtaatggcaacacttacttgtattggttcctgcagaggccaggccagtctcctcagctcctgatatatcggatgtccaaccttgcctcaggagtcccagacaggttcagtggcagtgggtcaggaactgctttcacactgagaatcactagagtggaggctgaggatgtgggtatttattactgtatgcaacatctagaatatcctttcacgttcggtgctgggaccaagctggagctgaaacggattgaagttatgtatcctcctccttacctagacaatgagaagagcaatggaaccattatccatgtgaaagggaaacacctttgtccaagtcccctatttcccggaccttctaagcccttttgggtgctggtggtggttggtggagtcctggcttgctatagcttgctagtaacagtggcctttattattttctgggtgaggagtaagaggagcaggctcctgcacagtgactacatgaacatgactccccgccgccccgggcccacccgcaagcattaccagccctatgccccaccacgcgacttcgcagcctatcgctccagagtgaagttcagcaggagcgcagacgcccccgcgtaccagcagggccagaaccagctctataacgagctcaatctaggacgaagagaggagtacgatgttttggacaagagacgtggccgggaccctgagatggggggaaagccgagaaggaagaaccctcaggaaggcctgtacaatgaactgcagaaagataagatggcggaggcctacagtgagattgggatgaaaggcgagcgccggaggggcaaggggcacgatggcctttaccagggtctcagtacagccaccaaggacacctacgacgcccttcacatgcaggccctgccccctcgctga

SEQ ID NO: 68 - DNA, 1503 bp, synthetic construct
  source 1..1503: mol_type = other DNA
atgcttctcctggtgacaagccttctgctctgtgagttaccacacccagcattcctcctgatcccagaagtgaagcttgaggagtctggaggaggcttggtgcaacctggaggatccatgaaactctcctgtgttgcctctggattcactttcagtaattactggatgaactgggtccgccagtctccagagaaggggcttgagtgggttgctgaaattagattgaaatctaataattatgcaacacattatgcggagtctgtgaaagggaggttcaccatctcaagagatgattccaaaagtagtgtctacctgcaaatgaacaacttaagagctgaagacactggcatttattactgttccagactcccgtcctttgactactggggccaaggcaccactctcacagtctcctcaggaggtggcggttccggaggaggtggatcaggaggcggaggctctggtggcggtggctcaggtggaggcggctcagatattgtgatgactcaggctgcaccctctgtacctgtcactcctggagagtcagtatccatctcctgcaggtctactaagagtctcctgcatagtaatggcaacacttacttgtattggttcctgcagaggccaggccagtctcctcagctcctgatatatcggatgtccaaccttgcctcaggagtcccagacaggttcagtggcagtgggtcaggaactgctttcacactgagaatcactagagtggaggctgaggatgtgggtatttattactgtatgcaacatctagaatatcctttcacgttcggtgctgggaccaagctggagctgaaacggaccacgacgccagcgccgcgaccaccaacaccggcgcccaccatcgcgtcgcagcccctgtccctgcgcccagaggcgtgccggccagcggcggggggcgcagtgcacacgagggggctggacttcgcctgtgatatctacatctgggcgcccttggccgggacttgtggggtccttctcctgtcactggttatcaccctttactgcaaacggggcagaaagaaactcctgtatatattcaaacaaccatttatgagaccagtacaaactactcaagaggaagatggctgtagctgccgatttccagaagaagaagaaggaggatgtgaactgagagtgaagttcagcaggagcgcagacgcccccgcgtaccagcagggccagaaccagctctataacgagctcaatctaggacgaagagaggagtacgatgttttggacaagagacgtggccgggaccctgagatggggggaaagccgagaaggaagaaccctcaggaaggcctgtacaatgaactgcagaaagataagatggcggaggcctacagtgagattgggatgaaaggcgagcgccggaggggcaaggggcacgatggcctttaccagggtctcagtacagccaccaaggacacctacgacgcccttcacatgcaggccctgccccctcgctga

SEQ ID NO: 69 - DNA, 1635 bp, synthetic construct
  source 1..1635: mol_type = other DNA
atgcttctcctggtgacaagccttctgctctgtgagttaccacacccagcattcctcctgatcccagaagtgaagcttgaggagtctggaggaggcttggtgcaacctggaggatccatgaaactctcctgtgttgcctctggattcactttcagtaattactggatgaactgggtccgccagtctccagagaaggggcttgagtgggttgctgaaattagattgaaatctaataattatgcaacacattatgcggagtctgtgaaagggaggttcaccatctcaagagatgattccaaaagtagtgtctacctgcaaatgaacaacttaagagctgaagacactggcatttattactgttccagactcccgtcctttgactactggggccaaggcaccactctcacagtctcctcaggaggtggcggttccggaggaggtggatcaggaggcggaggctctggtggcggtggctcaggtggaggcggctcagatattgtgatgactcaggctgcaccctctgtacctgtcactcctggagagtcagtatccatctcctgcaggtctactaagagtctcctgcatagtaatggcaacacttacttgtattggttcctgcagaggccaggccagtctcctcagctcctgatatatcggatgtccaaccttgcctcaggagtcccagacaggttcagtggcagtgggtcaggaactgctttcacactgagaatcactagagtggaggctgaggatgtgggtatttattactgtatgcaacatctagaatatcctttcacgttcggtgctgggaccaagctggagctgaaacggaccacgacgccagcgccgcgaccaccaacaccggcgcccaccatcgcgtcgcagcccctgtccctgcgcccagaggcgtgccggccagcggcggggggcgcagtgcacacgagggggctggacttcgcctgtgatttttgggtgctggtggtggttggtggagtcctggcttgctatagcttgctagtaacagtggcctttattattttctgggtgaggagtaagaggagcaggctcctgcacagtgactacatgaacatgactccccgccgccccgggcccacccgcaagcattaccagccctatgccccaccacgcgacttcgcagcctatcgctccaaacggggcagaaagaaactcctgtatatattcaaacaaccatttatgagaccagtacaaactactcaagaggaagatggctgtagctgccgatttccagaagaagaagaaggaggatgtgaactgagagtgaagttcagcaggagcgcagacgcccccgcgtaccagcagggccagaaccagctctataacgagctcaatctaggacgaagagaggagtacgatgttttggacaagagacgtggccgggaccctgagatggggggaaagccgagaaggaagaaccctcaggaaggcctgtacaatgaactgcagaaagataagatggcggaggcctacagtgagattgggatgaaaggcgagcgccggaggggcaaggggcacgatggcctttaccagggtctcagtacagccaccaaggacacctacgacgcccttcacatgcaggccctgccccctcgctga

SEQ ID NO: 70 - DNA, 1566 bp, synthetic construct
  source 1..1566: mol_type = other DNA
atgcttctcctggtgacaagccttctgctctgtgagttaccacacccagcattcctcctgatcccagaagtgaagcttgaggagtctggaggaggcttggtgcaacctggaggatccatgaaactctcctgtgttgcctctggattcactttcagtaattactggatgaactgggtccgccagtctccagagaaggggcttgagtgggttgctgaaattagattgaaatctaataattatgcaacacattatgcggagtctgtgaaagggaggttcaccatctcaagagatgattccaaaagtagtgtctacctgcaaatgaacaacttaagagctgaagacactggcatttattactgttccagactcccgtcctttgactactggggccaaggcaccactctcacagtctcctcaggaggtggcggttccggaggaggtggatcaggaggtggcggttccggaggaggtggatcaggaggtggcggttccggaggaggtggatcaggaggaggtggatcaggaggaggtggatcaggaggaggtggatcaggaggaggtggatcagatattgtgatgactcaggctgcaccctctgtacctgtcactcctggagagtcagtatccatctcctgcaggtctactaagagtctcctgcatagtaatggcaacacttacttgtattggttcctgcagaggccaggccagtctcctcagctcctgatatatcggatgtccaaccttgcctcaggagtcccagacaggttcagtggcagtgggtcaggaactgctttcacactgagaatcactagagtggaggctgaggatgtgggtatttattactgtatgcaacatctagaatatcctttcacgttcggtgctgggaccaagctggagctgaaacggattgaagttatgtatcctcctccttacctagacaatgagaagagcaatggaaccattatccatgtgaaagggaaacacctttgtccaagtcccctatttcccggaccttctaagcccttttgggtgctggtggtggttggtggagtcctggcttgctatagcttgctagtaacagtggcctttattattttctgggtgaggagtaagaggagcaggctcctgcacagtgactacatgaacatgactccccgccgccccgggcccacccgcaagcattaccagccctatgccccaccacgcgacttcgcagcctatcgctccagagtgaagttcagcaggagcgcagacgcccccgcgtaccagcagggccagaaccagctctataacgagctcaatctaggacgaagagaggagtacgatgttttggacaagagacgtggccgggaccctgagatggggggaaagccgagaaggaagaaccctcaggaaggcctgtacaatgaactgcagaaagataagatggcggaggcctacagtgagattgggatgaaaggcgagcgccggaggggcaaggggcacgatggcctttaccagggtctcagtacagccaccaaggacacctacgacgcccttcacatgcaggccctgccccctcgctga

SEQ ID NO: 71 - DNA, 1578 bp, synthetic construct
  source 1..1578: mol_type = other DNA
atgcttctcctggtgacaagccttctgctctgtgagttaccacacccagcattcctcctgatcccagaagtgaagcttgaggagtctggaggaggcttggtgcaacctggaggatccatgaaactctcctgtgttgcctctggattcactttcagtaattactggatgaactgggtccgccagtctccagagaaggggcttgagtgggttgctgaaattagattgaaatctaataattatgcaacacattatgcggagtctgtgaaagggaggttcaccatctcaagagatgattccaaaagtagtgtctacctgcaaatgaacaacttaagagctgaagacactggcatttattactgttccagactcccgtcctttgactactggggccaaggcaccactctcacagtctcctcaggaggtggcggttccggaggaggtggatcaggaggtggcggttccggaggaggtggatcaggaggtggcggttccggaggaggtggatcaggaggaggtggatcaggaggaggtggatcaggaggaggtggatcaggaggaggtggatcagatattgtgatgactcaggctgcaccctctgtacctgtcactcctggagagtcagtatccatctcctgcaggtctactaagagtctcctgcatagtaatggcaacacttacttgtattggttcctgcagaggccaggccagtctcctcagctcctgatatatcggatgtccaaccttgcctcaggagtcccagacaggttcagtggcagtgggtcaggaactgctttcacactgagaatcactagagtggaggctgaggatgtgggtatttattactgtatgcaacatctagaatatcctttcacgttcggtgctgggaccaagctggagctgaaacggaccacgacgccagcgccgcgaccaccaacaccggcgcccaccatcgcgtcgcagcccctgtccctgcgcccagaggcgtgccggccagcggcggggggcgcagtgcacacgagggggctggacttcgcctgtgatatctacatctgggcgcccttggccgggacttgtggggtccttctcctgtcactggttatcaccctttactgcaaacggggcagaaagaaactcctgtatatattcaaacaaccatttatgagaccagtacaaactactcaagaggaagatggctgtagctgccgatttccagaagaagaagaaggaggatgtgaactgagagtgaagttcagcaggagcgcagacgcccccgcgtaccagcagggccagaaccagctctataacgagctcaatctaggacgaagagaggagtacgatgttttggacaagagacgtggccgggaccctgagatggggggaaagccgagaaggaagaaccctcaggaaggcctgtacaatgaactgcagaaagataagatggcggaggcctacagtgagattgggatgaaaggcgagcgccggaggggcaaggggcacgatggcctttaccagggtctcagtacagccaccaaggacacctacgacgcccttcacatgcaggccctgccccctcgctga

SEQ ID NO: 72 - DNA, 1710 bp, synthetic construct
  source 1..1710: mol_type = other DNA
atgcttctcctggtgacaagccttctgctctgtgagttaccacacccagcattcctcctgatcccagaagtgaagcttgaggagtctggaggaggcttggtgcaacctggaggatccatgaaactctcctgtgttgcctctggattcactttcagtaattactggatgaactgggtccgccagtctccagagaaggggcttgagtgggttgctgaaattagattgaaatctaataattatgcaacacattatgcggagtctgtgaaagggaggttcaccatctcaagagatgattccaaaagtagtgtctacctgcaaatgaacaacttaagagctgaagacactggcatttattactgttccagactcccgtcctttgactactggggccaaggcaccactctcacagtctcctcaggaggtggcggttccggaggaggtggatcaggaggtggcggttccggaggaggtggatcaggaggtggcggttccggaggaggtggatcaggaggaggtggatcaggaggaggtggatcaggaggaggtggatcaggaggaggtggatcagatattgtgatgactcaggctgcaccctctgtacctgtcactcctggagagtcagtatccatctcctgcaggtctactaagagtctcctgcatagtaatggcaacacttacttgtattggttcctgcagaggccaggccagtctcctcagctcctgatatatcggatgtccaaccttgcctcaggagtcccagacaggttcagtggcagtgggtcaggaactgctttcacactgagaatcactagagtggaggctgaggatgtgggtatttattactgtatgcaacatctagaatatcctttcacgttcggtgctgggaccaagctggagctgaaacggaccacgacgccagcgccgcgaccaccaacaccggcgcccaccatcgcgtcgcagcccctgtccctgcgcccagaggcgtgccggccagcggcggggggcgcagtgcacacgagggggctggacttcgcctgtgatttttgggtgctggtggtggttggtggagtcctggcttgctatagcttgctagtaacagtggcctttattattttctgggtgaggagtaagaggagcaggctcctgcacagtgactacatgaacatgactccccgccgccccgggcccacccgcaagcattaccagccctatgccccaccacgcgacttcgcagcctatcgctccaaacggggcagaaagaaactcctgtatatattcaaacaaccatttatgagaccagtacaaactactcaagaggaagatggctgtagctgccgatttccagaagaagaagaaggaggatgtgaactgagagtgaagttcagcaggagcgcagacgcccccgcgtaccagcagggccagaaccagctctataacgagctcaatctaggacgaagagaggagtacgatgttttggacaagagacgtggccgggaccctgagatggggggaaagccgagaaggaagaaccctcaggaaggcctgtacaatgaactgcagaaagataagatggcggaggcctacagtgagattgggatgaaaggcgagcgccggaggggcaaggggcacgatggcctttaccagggtctcagtacagccaccaaggacacctacgacgcccttcacatgcaggccctgccccctcgctga

SEQ ID NO: 73 - DNA, 1470 bp, synthetic construct
  source 1..1470: mol_type = other DNA
atgttgttgctcgtcacctctcttctgctgtgtgagctccctcatccggccttcctgcttatccccgaagttaagctcgaggagtccggaggagggctggtccagcccggaggtagtatgaagctgtcatgcgtagcctccggcttcacattcagcaattactggatgaactgggtcagacagagtcccgagaaaggtctggaatgggtggccgaaatacggctgaagagcaataactatgccacacattacgcagagtcagtcaagggccgtttcaccattagcagagatgactccaagagtagcgtgtatctgcagatgaacaacctcagggctgaggacactggtcgctactactgctctagactgccctcctttgactactggggacaaggcaccactctgactgtctcaagtgggagcacatctggaagtggcaaacctgggtctggggaaggcagcactaaaggtgatatcgtgatgacacaggcagctccctccgtccaagtgacaccaggcgaatctgtcagcatttcttgtcggtccactaagtctctccttcactctaacgggaatacctacctctactggttcctgcaacgaccaggacaatccccacagctgctcatctatcggatgagcaatctcgccagtggggtgcctgatcggtttagcggtagcggctctggtacggcatttaccctgcgcattacacgcgttgaagcagaggatgttgggagatactattgcatgcagcacctggaatatccctttaccttcggcgctggcacgaagctcgagctgaagaggattgaggtgatgtaccctcctccctacctggacaacgagaaaagcaatggaaccatcattcacgtaaaaggcaagcatctgtgtccgtcaccactgtttccggggccaagtaaacccttttgggtgttggtggttgttggtggggtactcgcgtgctattccctgcttgtgaccgtggccttcatcatcttctgggtgcgctcaaagcgatccagacttctgcatagcgactacatgaacatgactcccaggcgccctgggccaacacgtaagcactatcagccctatgctcctccacgggattttgccgcatacagatccagagtgaagttctcaaggagcgctgatgctccggcctatcagcagggccagaatcagctgtacaatgagctgaatcttggaaggagagaggaatacgacgtgttggacaaacgccgaggaagggaccctgaaatgggtggcaaaccacggaggaagaaccctcaggaaggactgtataacgagctgcagaaagataagatggcggaggcgtactcagagataggcatgaagggagaacgccgtcgaggcaaaggccacgatggcctgtatcaggggttgagcactgccacgaaagacacctatgacgcactgcacatgcaagccttgccaccccggtga

SEQ ID NO: 74 - DNA, 1482 bp, synthetic construct
  source 1..1482: mol_type = other DNA
atgttgttgctcgtcacctctcttctgctgtgtgagctccctcatccggccttcctgcttatccccgaagttaagctcgaggagtccggaggagggctggtccagcccggaggtagtatgaagctgtcatgcgtagcctccggcttcacattcagcaattactggatgaactgggtcagacagagtcccgagaaaggtctggaatgggtggccgaaatacggctgaagagcaataactatgccacacattacgcagagtcagtcaagggccgtttcaccattagcagagatgactccaagagtagcgtgtatctgcagatgaacaacctcagggctgaggacactggtcgctactactgctctagactgccctcctttgactactggggacaaggcaccactctgactgtctcaagtgggagcacatctggaagtggcaaacctgggtctggggaaggcagcactaaaggtgatatcgtgatgacacaggcagctccctccgtccaagtgacaccaggcgaatctgtcagcatttcttgtcggtccactaagtctctccttcactctaacgggaatacctacctctactggttcctgcaacgaccaggacaatccccacagctgctcatctatcggatgagcaatctcgccagtggggtgcctgatcggtttagcggtagcggctctggtacggcatttaccctgcgcattacacgcgttgaagcagaggatgttgggagatactattgcatgcagcacctggaatatccctttaccttcggcgctggcacgaagctcgagctgaagaggaccacgacgccagcgccgcgaccaccaacaccggcgcccaccatcgcgtcgcagcccctgtccctgcgcccagaggcgtgccggccagcggcggggggcgcagtgcacacgagggggctggacttcgcctgtgatatctacatctgggcgcccttggccgggacttgtggggtccttctcctgtcactggttatcaccctttactgcaaacggggcagaaagaaactcctgtatatattcaaacaaccatttatgagaccagtacaaactactcaagaggaagatggctgtagctgccgatttccagaagaagaagaaggaggatgtgaactgagagtgaagttcagcaggagcgcagacgcccccgcgtaccagcagggccagaaccagctctataacgagctcaatctaggacgaagagaggagtacgatgttttggacaagagacgtggccgggaccctgagatggggggaaagccgagaaggaagaaccctcaggaaggcctgtacaatgaactgcagaaagataagatggcggaggcctacagtgagattgggatgaaaggcgagcgccggaggggcaaggggcacgatggcctttaccagggtctcagtacagccaccaaggacacctacgacgcccttcacatgcaggccctgccccctcgctga

SEQ ID NO: 75 - DNA, 1614 bp, synthetic construct
  source 1..1614: mol_type = other DNA
atgttgttgctcgtcacctctcttctgctgtgtgagctccctcatccggccttcctgcttatccccgaagttaagctcgaggagtccggaggagggctggtccagcccggaggtagtatgaagctgtcatgcgtagcctccggcttcacattcagcaattactggatgaactgggtcagacagagtcccgagaaaggtctggaatgggtggccgaaatacggctgaagagcaataactatgccacacattacgcagagtcagtcaagggccgtttcaccattagcagagatgactccaagagtagcgtgtatctgcagatgaacaacctcagggctgaggacactggtcgctactactgctctagactgccctcctttgactactggggacaaggcaccactctgactgtctcaagtgggagcacatctggaagtggcaaacctgggtctggggaaggcagcactaaaggtgatatcgtgatgacacaggcagctccctccgtccaagtgacaccaggcgaatctgtcagcatttcttgtcggtccactaagtctctccttcactctaacgggaatacctacctctactggttcctgcaacgaccaggacaatccccacagctgctcatctatcggatgagcaatctcgccagtggggtgcctgatcggtttagcggtagcggctctggtacggcatttaccctgcgcattacacgcgttgaagcagaggatgttgggagatactattgcatgcagcacctggaatatccctttaccttcggcgctggcacgaagctcgagctgaagaggaccacgacgccagcgccgcgaccaccaacaccggcgcccaccatcgcgtcgcagcccctgtccctgcgcccagaggcgtgccggccagcggcggggggcgcagtgcacacgagggggctggacttcgcctgtgatttttgggtgctggtggtggttggtggagtcctggcttgctatagcttgctagtaacagtggcctttattattttctgggtgaggagtaagaggagcaggctcctgcacagtgactacatgaacatgactccccgccgccccgggcccacccgcaagcattaccagccctatgccccaccacgcgacttcgcagcctatcgctccaaacggggcagaaagaaactcctgtatatattcaaacaaccatttatgagaccagtacaaactactcaagaggaagatggctgtagctgccgatttccagaagaagaagaaggaggatgtgaactgagagtgaagttcagcaggagcgcagacgcccccgcgtaccagcagggccagaaccagctctataacgagctcaatctaggacgaagagaggagtacgatgttttggacaagagacgtggccgggaccctgagatggggggaaagccgagaaggaagaaccctcaggaaggcctgtacaatgaactgcagaaagataagatggcggaggcctacagtgagattgggatgaaaggcgagcgccggaggggcaaggggcacgatggcctttaccagggtctcagtacagccaccaaggacacctacgacgcccttcacatgcaggccctgccccctcgctga

SEQ ID NO: 76 - DNA, 1491 bp, synthetic construct
  source 1..1491: mol_type = other DNA
atgttgttgctcgtcacctctcttctgctgtgtgagctccctcatccggccttcctgcttatccccgaagttaagctcgaggagtccggaggagggctggtccagcccggaggtagtatgaagctgtcatgcgtagcctccggcttcacattcagcaattactggatgaactgggtcagacagagtcccgagaaaggtctggaatgggtggccgaaatacggctgaagagcaataactatgccacacattacgcagagtcagtcaagggccgtttcaccattagcagagatgactccaagagtagcgtgtatctgcagatgaacaacctcagggctgaggacactggtcgctactactgctctagactgccctcctttgactactggggacaaggcaccactctgactgtctcaagtggaggtggcggttccggaggaggtggatcaggaggcggaggctctggtggcggtggctcaggtggaggcggctcagatatcgtgatgacacaggcagctccctccgtccaagtgacaccaggcgaatctgtcagcatttcttgtcggtccactaagtctctccttcactctaacgggaatacctacctctactggttcctgcaacgaccaggacaatccccacagctgctcatctatcggatgagcaatctcgccagtggggtgcctgatcggtttagcggtagcggctctggtacggcatttaccctgcgcattacacgcgttgaagcagaggatgttgggagatactattgcatgcagcacctggaatatccctttaccttcggcgctggcacgaagctcgagctgaagaggattgaggtgatgtaccctcctccctacctggacaacgagaaaagcaatggaaccatcattcacgtaaaaggcaagcatctgtgtccgtcaccactgtttccggggccaagtaaacccttttgggtgttggtggttgttggtggggtactcgcgtgctattccctgcttgtgaccgtggccttcatcatcttctgggtgcgctcaaagcgatccagacttctgcatagcgactacatgaacatgactcccaggcgccctgggccaacacgtaagcactatcagccctatgctcctccacgggattttgccgcatacagatccagagtgaagttctcaaggagcgctgatgctccggcctatcagcagggccagaatcagctgtacaatgagctgaatcttggaaggagagaggaatacgacgtgttggacaaacgccgaggaagggaccctgaaatgggtggcaaaccacggaggaagaaccctcaggaaggactgtataacgagctgcagaaagataagatggcggaggcgtactcagagataggcatgaagggagaacgccgtcgaggcaaaggccacgatggcctgtatcaggggttgagcactgccacgaaagacacctatgacgcactgcacatgcaagccttgccaccccggtga

SEQ ID NO: 77 - DNA, 1503 bp, synthetic construct
  source 1..1503: mol_type = other DNA
atgttgttgctcgtcacctctcttctgctgtgtgagctccctcatccggccttcctgcttatccccgaagttaagctcgaggagtccggaggagggctggtccagcccggaggtagtatgaagctgtcatgcgtagcctccggcttcacattcagcaattactggatgaactgggtcagacagagtcccgagaaaggtctggaatgggtggccgaaatacggctgaagagcaataactatgccacacattacgcagagtcagtcaagggccgtttcaccattagcagagatgactccaagagtagcgtgtatctgcagatgaacaacctcagggctgaggacactggtcgctactactgctctagactgccctcctttgactactggggacaaggcaccactctgactgtctcaagtggaggtggcggttccggaggaggtggatcaggaggcggaggctctggtggcggtggctcaggtggaggcggctcagatatcgtgatgacacaggcagctccctccgtccaagtgacaccaggcgaatctgtcagcatttcttgtcggtccactaagtctctccttcactctaacgggaatacctacctctactggttcctgcaacgaccaggacaatccccacagctgctcatctatcggatgagcaatctcgccagtggggtgcctgatcggtttagcggtagcggctctggtacggcatttaccctgcgcattacacgcgttgaagcagaggatgttgggagatactattgcatgcagcacctggaatatccctttaccttcggcgctggcacgaagctcgagctgaagaggaccacgacgccagcgccgcgaccaccaacaccggcgcccaccatcgcgtcgcagcccctgtccctgcgcccagaggcgtgccggccagcggcggggggcgcagtgcacacgagggggctggacttcgcctgtgatatctacatctgggcgcccttggccgggacttgtggggtccttctcctgtcactggttatcaccctttactgcaaacggggcagaaagaaactcctgtatatattcaaacaaccatttatgagaccagtacaaactactcaagaggaagatggctgtagctgccgatttccagaagaagaagaaggaggatgtgaactgagagtgaagttcagcaggagcgcagacgcccccgcgtaccagcagggccagaaccagctctataacgagctcaatctaggacgaagagaggagtacgatgttttggacaagagacgtggccgggaccctgagatggggggaaagccgagaaggaagaaccctcaggaaggcctgtacaatgaactgcagaaagataagatggcggaggcctacagtgagattgggatgaaaggcgagcgccggaggggcaaggggcacgatggcctttaccagggtctcagtacagccaccaaggacacctacgacgcccttcacatgcaggccctgccccctcgctga

SEQ ID NO: 78 - DNA, 1635 bp, synthetic construct
  source 1..1635: mol_type = other DNA
atgttgttgctcgtcacctctcttctgctgtgtgagctccctcatccggccttcctgcttatccccgaagttaagctcgaggagtccggaggagggctggtccagcccggaggtagtatgaagctgtcatgcgtagcctccggcttcacattcagcaattactggatgaactgggtcagacagagtcccgagaaaggtctggaatgggtggccgaaatacggctgaagagcaataactatgccacacattacgcagagtcagtcaagggccgtttcaccattagcagagatgactccaagagtagcgtgtatctgcagatgaacaacctcagggctgaggacactggtcgctactactgctctagactgccctcctttgactactggggacaaggcaccactctgactgtctcaagtggaggtggcggttccggaggaggtggatcaggaggcggaggctctggtggcggtggctcaggtggaggcggctcagatatcgtgatgacacaggcagctccctccgtccaagtgacaccaggcgaatctgtcagcatttcttgtcggtccactaagtctctccttcactctaacgggaatacctacctctactggttcctgcaacgaccaggacaatccccacagctgctcatctatcggatgagcaatctcgccagtggggtgcctgatcggtttagcggtagcggctctggtacggcatttaccctgcgcattacacgcgttgaagcagaggatgttgggagatactattgcatgcagcacctggaatatccctttaccttcggcgctggcacgaagctcgagctgaagaggaccacgacgccagcgccgcgaccaccaacaccggcgcccaccatcgcgtcgcagcccctgtccctgcgcccagaggcgtgccggccagcggcggggggcgcagtgcacacgagggggctggacttcgcctgtgatttttgggtgctggtggtggttggtggagtcctggcttgctatagcttgctagtaacagtggcctttattattttctgggtgaggagtaagaggagcaggctcctgcacagtgactacatgaacatgactccccgccgccccgggcccacccgcaagcattaccagccctatgccccaccacgcgacttcgcagcctatcgctccaaacggggcagaaagaaactcctgtatatattcaaacaaccatttatgagaccagtacaaactactcaagaggaagatggctgtagctgccgatttccagaagaagaagaaggaggatgtgaactgagagtgaagttcagcaggagcgcagacgcccccgcgtaccagcagggccagaaccagctctataacgagctcaatctaggacgaagagaggagtacgatgttttggacaagagacgtggccgggaccctgagatggggggaaagccgagaaggaagaaccctcaggaaggcctgtacaatgaactgcagaaagataagatggcggaggcctacagtgagattgggatgaaaggcgagcgccggaggggcaaggggcacgatggcctttaccagggtctcagtacagccaccaaggacacctacgacgcccttcacatgcaggccctgccccctcgctga

SEQ ID NO: 79 - DNA, 1506 bp, synthetic construct
  source 1..1506: mol_type = other DNA
atgcttctcctggtgacaagccttctgctctgtgagttaccacacccagcattcctcctgatcccagaagtgaagcttgaggagtctggaggaggcttggtgcaacctggaggatccatgaaactctcctgtgttgcctctggattcactttcagtaattactggatgaactgggtccgccagtctccagagaaggggcttgagtgggttgctgaaattagattgaaatctaataattatgcaacacattatgcggagtctgtgaaagggaggttcaccatctcaagagatgattccaaaagtagtgtctacctgcaaatgaacaacttaagagctgaagacactggcatttattactgttccagactcccgtcctttgactactggggccaaggcaccactctcacagtctcctcaggaggtggcggttccggaggaggtggatcaggaggtggcggttccggaggaggtggatcaggaggtggcggttccggaggaggtggatcagatattgtgatgactcaggctgcaccctctgtacctgtcactcctggagagtcagtatccatctcctgcaggtctactaagagtctcctgcatagtaatggcaacacttacttgtattggttcctgcagaggccaggccagtctcctcagctcctgatatatcggatgtccaaccttgcctcaggagtcccagacaggttcagtggcagtgggtcaggaactgctttcacactgagaatcactagagtggaggctgaggatgtgggtatttattactgtatgcaacatctagaatatcctttcacgttcggtgctgggaccaagctggagctgaaacggattgaagttatgtatcctcctccttacctagacaatgagaagagcaatggaaccattatccatgtgaaagggaaacacctttgtccaagtcccctatttcccggaccttctaagcccttttgggtgctggtggtggttggtggagtcctggcttgctatagcttgctagtaacagtggcctttattattttctgggtgaggagtaagaggagcaggctcctgcacagtgactacatgaacatgactccccgccgccccgggcccacccgcaagcattaccagccctatgccccaccacgcgacttcgcagcctatcgctccagagtgaagttcagcaggagcgcagacgcccccgcgtaccagcagggccagaaccagctctataacgagctcaatctaggacgaagagaggagtacgatgttttggacaagagacgtggccgggaccctgagatggggggaaagccgagaaggaagaaccctcaggaaggcctgtacaatgaactgcagaaagataagatggcggaggcctacagtgagattgggatgaaaggcgagcgccggaggggcaaggggcacgatggcctttaccagggtctcagtacagccaccaaggacacctacgacgcccttcacatgcaggccctgccccctcgctga

SEQ ID NO: 80 - DNA, 1518 bp, synthetic construct
  source 1..1518: mol_type = other DNA
atgcttctcctggtgacaagccttctgctctgtgagttaccacacccagcattcctcctgatcccagaagtgaagcttgaggagtctggaggaggcttggtgcaacctggaggatccatgaaactctcctgtgttgcctctggattcactttcagtaattactggatgaactgggtccgccagtctccagagaaggggcttgagtgggttgctgaaattagattgaaatctaataattatgcaacacattatgcggagtctgtgaaagggaggttcaccatctcaagagatgattccaaaagtagtgtctacctgcaaatgaacaacttaagagctgaagacactggcatttattactgttccagactcccgtcctttgactactggggccaaggcaccactctcacagtctcctcaggaggtggcggttccggaggaggtggatcaggaggtggcggttccggaggaggtggatcaggaggtggcggttccggaggaggtggatcagatattgtgatgactcaggctgcaccctctgtacctgtcactcctggagagtcagtatccatctcctgcaggtctactaagagtctcctgcatagtaatggcaacacttacttgtattggttcctgcagaggccaggccagtctcctcagctcctgatatatcggatgtccaaccttgcctcaggagtcccagacaggttcagtggcagtgggtcaggaactgctttcacactgagaatcactagagtggaggctgaggatgtgggtatttattactgtatgcaacatctagaatatcctttcacgttcggtgctgggaccaagctggagctgaaacggaccacgacgccagcgccgcgaccaccaacaccggcgcccaccatcgcgtcgcagcccctgtccctgcgcccagaggcgtgccggccagcggcggggggcgcagtgcacacgagggggctggacttcgcctgtgatatctacatctgggcgcccttggccgggacttgtggggtccttctcctgtcactggttatcaccctttactgcaaacggggcagaaagaaactcctgtatatattcaaacaaccatttatgagaccagtacaaactactcaagaggaagatggctgtagctgccgatttccagaagaagaagaaggaggatgtgaactgagagtgaagttcagcaggagcgcagacgcccccgcgtaccagcagggccagaaccagctctataacgagctcaatctaggacgaagagaggagtacgatgttttggacaagagacgtggccgggaccctgagatggggggaaagccgagaaggaagaaccctcaggaaggcctgtacaatgaactgcagaaagataagatggcggaggcctacagtgagattgggatgaaaggcgagcgccggaggggcaaggggcacgatggcctttaccagggtctcagtacagccaccaaggacacctacgacgcccttcacatgcaggccctgccccctcgctga

SEQ ID NO: 81 - DNA, 1650 bp, synthetic construct
  source 1..1650: mol_type = other DNA
atgcttctcctggtgacaagccttctgctctgtgagttaccacacccagcattcctcctgatcccagaagtgaagcttgaggagtctggaggaggcttggtgcaacctggaggatccatgaaactctcctgtgttgcctctggattcactttcagtaattactggatgaactgggtccgccagtctccagagaaggggcttgagtgggttgctgaaattagattgaaatctaataattatgcaacacattatgcggagtctgtgaaagggaggttcaccatctcaagagatgattccaaaagtagtgtctacctgcaaatgaacaacttaagagctgaagacactggcatttattactgttccagactcccgtcctttgactactggggccaaggcaccactctcacagtctcctcaggaggtggcggttccggaggaggtggatcaggaggtggcggttccggaggaggtggatcaggaggtggcggttccggaggaggtggatcagatattgtgatgactcaggctgcaccctctgtacctgtcactcctggagagtcagtatccatctcctgcaggtctactaagagtctcctgcatagtaatggcaacacttacttgtattggttcctgcagaggccaggccagtctcctcagctcctgatatatcggatgtccaaccttgcctcaggagtcccagacaggttcagtggcagtgggtcaggaactgctttcacactgagaatcactagagtggaggctgaggatgtgggtatttattactgtatgcaacatctagaatatcctttcacgttcggtgctgggaccaagctggagctgaaacggaccacgacgccagcgccgcgaccaccaacaccggcgcccaccatcgcgtcgcagcccctgtccctgcgcccagaggcgtgccggccagcggcggggggcgcagtgcacacgagggggctggacttcgcctgtgatttttgggtgctggtggtggttggtggagtcctggcttgctatagcttgctagtaacagtggcctttattattttctgggtgaggagtaagaggagcaggctcctgcacagtgactacatgaacatgactccccgccgccccgggcccacccgcaagcattaccagccctatgccccaccacgcgacttcgcagcctatcgctccaaacggggcagaaagaaactcctgtatatattcaaacaaccatttatgagaccagtacaaactactcaagaggaagatggctgtagctgccgatttccagaagaagaagaaggaggatgtgaactgagagtgaagttcagcaggagcgcagacgcccccgcgtaccagcagggccagaaccagctctataacgagctcaatctaggacgaagagaggagtacgatgttttggacaagagacgtggccgggaccctgagatggggggaaagccgagaaggaagaaccctcaggaaggcctgtacaatgaactgcagaaagataagatggcggaggcctacagtgagattgggatgaaaggcgagcgccggaggggcaaggggcacgatggcctttaccagggtctcagtacagccaccaaggacacctacgacgcccttcacatgcaggccctgccccctcgctga

SEQ ID NO: 82 - DNA, 1518 bp, synthetic construct
  source 1..1518: mol_type = other DNA
atgttgttgctcgtcacctctcttctgctgtgtgagctccctcatccggccttcctgcttatccccgaagttaagctcgaggagtccggaggagggctggtccagcccggaggtagtatgaagctgtcatgcgtagcctccggcttcacattcagcaattactggatgaactgggtcagacagagtcccgagaaaggtctggaatgggtggccgaaatacggctgaagagcaataactatgccacacattacgcagagtcagtcaagggccgtttcaccattagcagagatgactccaagagtagcgtgtatctgcagatgaacaacctcagggctgaggacactggtcgctactactgctctagactgccctcctttgactactggggacaaggcaccactctgactgtctcaagtggaggtggcggttccggaggaggtggatcaggaggtggcggttccggaggaggtggatcaggaggtggcggttccggaggaggtggatcagatatcgtgatgacacaggcagctccctccgtccaagtgacaccaggcgaatctgtcagcatttcttgtcggtccactaagtctctccttcactctaacgggaatacctacctctactggttcctgcaacgaccaggacaatccccacagctgctcatctatcggatgagcaatctcgccagtggggtgcctgatcggtttagcggtagcggctctggtacggcatttaccctgcgcattacacgcgttgaagcagaggatgttgggagatactattgcatgcagcacctggaatatccctttaccttcggcgctggcacgaagctcgagctgaagaggaccacgacgccagcgccgcgaccaccaacaccggcgcccaccatcgcgtcgcagcccctgtccctgcgcccagaggcgtgccggccagcggcggggggcgcagtgcacacgagggggctggacttcgcctgtgatatctacatctgggcgcccttggccgggacttgtggggtccttctcctgtcactggttatcaccctttactgcaaacggggcagaaagaaactcctgtatatattcaaacaaccatttatgagaccagtacaaactactcaagaggaagatggctgtagctgccgatttccagaagaagaagaaggaggatgtgaactgagagtgaagttcagcaggagcgcagacgcccccgcgtaccagcagggccagaaccagctctataacgagctcaatctaggacgaagagaggagtacgatgttttggacaagagacgtggccgggaccctgagatggggggaaagccgagaaggaagaaccctcaggaaggcctgtacaatgaactgcagaaagataagatggcggaggcctacagtgagattgggatgaaaggcgagcgccggaggggcaaggggcacgatggcctttaccagggtctcagtacagccaccaaggacacctacgacgcccttcacatgcaggccctgccccctcgctga

SEQ ID NO: 83 - DNA, 1650 bp, synthetic construct
  source 1..1650: mol_type = other DNA
atgttgttgctcgtcacctctcttctgctgtgtgagctccctcatccggccttcctgcttatccccgaagttaagctcgaggagtccggaggagggctggtccagcccggaggtagtatgaagctgtcatgcgtagcctccggcttcacattcagcaattactggatgaactgggtcagacagagtcccgagaaaggtctggaatgggtggccgaaatacggctgaagagcaataactatgccacacattacgcagagtcagtcaagggccgtttcaccattagcagagatgactccaagagtagcgtgtatctgcagatgaacaacctcagggctgaggacactggtcgctactactgctctagactgccctcctttgactactggggacaaggcaccactctgactgtctcaagtggaggtggcggttccggaggaggtggatcaggaggtggcggttccggaggaggtggatcaggaggtggcggttccggaggaggtggatcagatatcgtgatgacacaggcagctccctccgtccaagtgacaccaggcgaatctgtcagcatttcttgtcggtccactaagtctctccttcactctaacgggaatacctacctctactggttcctgcaacgaccaggacaatccccacagctgctcatctatcggatgagcaatctcgccagtggggtgcctgatcggtttagcggtagcggctctggtacggcatttaccctgcgcattacacgcgttgaagcagaggatgttgggagatactattgcatgcagcacctggaatatccctttaccttcggcgctggcacgaagctcgagctgaagaggaccacgacgccagcgccgcgaccaccaacaccggcgcccaccatcgcgtcgcagcccctgtccctgcgcccagaggcgtgccggccagcggcggggggcgcagtgcacacgagggggctggacttcgcctgtgatttttgggtgctggtggtggttggtggagtcctggcttgctatagcttgctagtaacagtggcctttattattttctgggtgaggagtaagaggagcaggctcctgcacagtgactacatgaacatgactccccgccgccccgggcccacccgcaagcattaccagccctatgccccaccacgcgacttcgcagcctatcgctccaaacggggcagaaagaaactcctgtatatattcaaacaaccatttatgagaccagtacaaactactcaagaggaagatggctgtagctgccgatttccagaagaagaagaaggaggatgtgaactgagagtgaagttcagcaggagcgcagacgcccccgcgtaccagcagggccagaaccagctctataacgagctcaatctaggacgaagagaggagtacgatgttttggacaagagacgtggccgggaccctgagatggggggaaagccgagaaggaagaaccctcaggaaggcctgtacaatgaactgcagaaagataagatggcggaggcctacagtgagattgggatgaaaggcgagcgccggaggggcaaggggcacgatggcctttaccagggtctcagtacagccaccaaggacacctacgacgcccttcacatgcaggccctgccccctcgctga

SEQ ID NO: 84 - DNA, 1566 bp, synthetic construct
  source 1..1566: mol_type = other DNA
atgttgttgctcgtcacctctcttctgctgtgtgagctccctcatccggccttcctgcttatccccgaagttaagctcgaggagtccggaggagggctggtccagcccggaggtagtatgaagctgtcatgcgtagcctccggcttcacattcagcaattactggatgaactgggtcagacagagtcccgagaaaggtctggaatgggtggccgaaatacggctgaagagcaataactatgccacacattacgcagagtcagtcaagggccgtttcaccattagcagagatgactccaagagtagcgtgtatctgcagatgaacaacctcagggctgaggacactggtcgctactactgctctagactgccctcctttgactactggggacaaggcaccactctgactgtctcaagtggaggtggcggttccggaggaggtggatcaggaggtggcggttccggaggaggtggatcaggaggtggcggttccggaggaggtggatcaggaggaggtggatcaggaggaggtggatcaggaggaggtggatcaggaggaggtggatcagatatcgtgatgacacaggcagctccctccgtccaagtgacaccaggcgaatctgtcagcatttcttgtcggtccactaagtctctccttcactctaacgggaatacctacctctactggttcctgcaacgaccaggacaatccccacagctgctcatctatcggatgagcaatctcgccagtggggtgcctgatcggtttagcggtagcggctctggtacggcatttaccctgcgcattacacgcgttgaagcagaggatgttgggagatactattgcatgcagcacctggaatatccctttaccttcggcgctggcacgaagctcgagctgaagaggattgaggtgatgtaccctcctccctacctggacaacgagaaaagcaatggaaccatcattcacgtaaaaggcaagcatctgtgtccgtcaccactgtttccggggccaagtaaacccttttgggtgttggtggttgttggtggggtactcgcgtgctattccctgcttgtgaccgtggccttcatcatcttctgggtgcgctcaaagcgatccagacttctgcatagcgactacatgaacatgactcccaggcgccctgggccaacacgtaagcactatcagccctatgctcctccacgggattttgccgcatacagatccagagtgaagttctcaaggagcgctgatgctccggcctatcagcagggccagaatcagctgtacaatgagctgaatcttggaaggagagaggaatacgacgtgttggacaaacgccgaggaagggaccctgaaatgggtggcaaaccacggaggaagaaccctcaggaaggactgtataacgagctgcagaaagataagatggcggaggcgtactcagagataggcatgaagggagaacgccgtcgaggcaaaggccacgatggcctgtatcaggggttgagcactgccacgaaagacacctatgacgcactgcacatgcaagccttgccaccccggtga

SEQ ID NO: 85 - DNA, 1578 bp, synthetic construct
  source 1..1578: mol_type = other DNA
atgttgttgctcgtcacctctcttctgctgtgtgagctccctcatccggccttcctgcttatccccgaagttaagctcgaggagtccggaggagggctggtccagcccggaggtagtatgaagctgtcatgcgtagcctccggcttcacattcagcaattactggatgaactgggtcagacagagtcccgagaaaggtctggaatgggtggccgaaatacggctgaagagcaataactatgccacacattacgcagagtcagtcaagggccgtttcaccattagcagagatgactccaagagtagcgtgtatctgcagatgaacaacctcagggctgaggacactggtcgctactactgctctagactgccctcctttgactactggggacaaggcaccactctgactgtctcaagtggaggtggcggttccggaggaggtggatcaggaggtggcggttccggaggaggtggatcaggaggtggcggttccggaggaggtggatcaggaggaggtggatcaggaggaggtggatcaggaggaggtggatcaggaggaggtggatcagatatcgtgatgacacaggcagctccctccgtccaagtgacaccaggcgaatctgtcagcatttcttgtcggtccactaagtctctccttcactctaacgggaatacctacctctactggttcctgcaacgaccaggacaatccccacagctgctcatctatcggatgagcaatctcgccagtggggtgcctgatcggtttagcggtagcggctctggtacggcatttaccctgcgcattacacgcgttgaagcagaggatgttgggagatactattgcatgcagcacctggaatatccctttaccttcggcgctggcacgaagctcgagctgaagaggaccacgacgccagcgccgcgaccaccaacaccggcgcccaccatcgcgtcgcagcccctgtccctgcgcccagaggcgtgccggccagcggcggggggcgcagtgcacacgagggggctggacttcgcctgtgatatctacatctgggcgcccttggccgggacttgtggggtccttctcctgtcactggttatcaccctttactgcaaacggggcagaaagaaactcctgtatatattcaaacaaccatttatgagaccagtacaaactactcaagaggaagatggctgtagctgccgatttccagaagaagaagaaggaggatgtgaactgagagtgaagttcagcaggagcgcagacgcccccgcgtaccagcagggccagaaccagctctataacgagctcaatctaggacgaagagaggagtacgatgttttggacaagagacgtggccgggaccctgagatggggggaaagccgagaaggaagaaccctcaggaaggcctgtacaatgaactgcagaaagataagatggcggaggcctacagtgagattgggatgaaaggcgagcgccggaggggcaaggggcacgatggcctttaccagggtctcagtacagccaccaaggacacctacgacgcccttcacatgcaggccctgccccctcgctga

SEQ ID NO: 86 - DNA, 1710 bp, synthetic construct
  source 1..1710: mol_type = other DNA
atgttgttgctcgtcacctctcttctgctgtgtgagctccctcatccggccttcctgcttatccccgaagttaagctcgaggagtccggaggagggctggtccagcccggaggtagtatgaagctgtcatgcgtagcctccggcttcacattcagcaattactggatgaactgggtcagacagagtcccgagaaaggtctggaatgggtggccgaaatacggctgaagagcaataactatgccacacattacgcagagtcagtcaagggccgtttcaccattagcagagatgactccaagagtagcgtgtatctgcagatgaacaacctcagggctgaggacactggtcgctactactgctctagactgccctcctttgactactggggacaaggcaccactctgactgtctcaagtggaggtggcggttccggaggaggtggatcaggaggtggcggttccggaggaggtggatcaggaggtggcggttccggaggaggtggatcaggaggaggtggatcaggaggaggtggatcaggaggaggtggatcaggaggaggtggatcagatatcgtgatgacacaggcagctccctccgtccaagtgacaccaggcgaatctgtcagcatttcttgtcggtccactaagtctctccttcactctaacgggaatacctacctctactggttcctgcaacgaccaggacaatccccacagctgctcatctatcggatgagcaatctcgccagtggggtgcctgatcggtttagcggtagcggctctggtacggcatttaccctgcgcattacacgcgttgaagcagaggatgttgggagatactattgcatgcagcacctggaatatccctttaccttcggcgctggcacgaagctcgagctgaagaggaccacgacgccagcgccgcgaccaccaacaccggcgcccaccatcgcgtcgcagcccctgtccctgcgcccagaggcgtgccggccagcggcggggggcgcagtgcacacgagggggctggacttcgcctgtgatttttgggtgctggtggtggttggtggagtcctggcttgctatagcttgctagtaacagtggcctttattattttctgggtgaggagtaagaggagcaggctcctgcacagtgactacatgaacatgactccccgccgccccgggcccacccgcaagcattaccagccctatgccccaccacgcgacttcgcagcctatcgctccaaacggggcagaaagaaactcctgtatatattcaaacaaccatttatgagaccagtacaaactactcaagaggaagatggctgtagctgccgatttccagaagaagaagaaggaggatgtgaactgagagtgaagttcagcaggagcgcagacgcccccgcgtaccagcagggccagaaccagctctataacgagctcaatctaggacgaagagaggagtacgatgttttggacaagagacgtggccgggaccctgagatggggggaaagccgagaaggaagaaccctcaggaaggcctgtacaatgaactgcagaaagataagatggcggaggcctacagtgagattgggatgaaaggcgagcgccggaggggcaaggggcacgatggcctttaccagggtctcagtacagccaccaaggacacctacgacgcccttcacatgcaggccctgccccctcgctga

SEQ ID NO: 87 - DNA, 1506 bp, synthetic construct
  source 1..1506: mol_type = other DNA
atgttgttgctcgtcacctctcttctgctgtgtgagctccctcatccggccttcctgcttatccccgaagttaagctcgaggagtccggaggagggctggtccagcccggaggtagtatgaagctgtcatgcgtagcctccggcttcacattcagcaattactggatgaactgggtcagacagagtcccgagaaaggtctggaatgggtggccgaaatacggctgaagagcaataactatgccacacattacgcagagtcagtcaagggccgtttcaccattagcagagatgactccaagagtagcgtgtatctgcagatgaacaacctcagggctgaggacactggtcgctactactgctctagactgccctcctttgactactggggacaaggcaccactctgactgtctcaagtggaggtggcggttccggaggaggtggatcaggaggtggcggttccggaggaggtggatcaggaggtggcggttccggaggaggtggatcagatatcgtgatgacacaggcagctccctccgtccaagtgacaccaggcgaatctgtcagcatttcttgtcggtccactaagtctctccttcactctaacgggaatacctacctctactggttcctgcaacgaccaggacaatccccacagctgctcatctatcggatgagcaatctcgccagtggggtgcctgatcggtttagcggtagcggctctggtacggcatttaccctgcgcattacacgcgttgaagcagaggatgttgggagatactattgcatgcagcacctggaatatccctttaccttcggcgctggcacgaagctcgagctgaagaggattgaggtgatgtaccctcctccctacctggacaacgagaaaagcaatggaaccatcattcacgtaaaaggcaagcatctgtgtccgtcaccactgtttccggggccaagtaaacccttttgggtgttggtggttgttggtggggtactcgcgtgctattccctgcttgtgaccgtggccttcatcatcttctgggtgcgctcaaagcgatccagacttctgcatagcgactacatgaacatgactcccaggcgccctgggccaacacgtaagcactatcagccctatgctcctccacgggattttgccgcatacagatccagagtgaagttctcaaggagcgctgatgctccggcctatcagcagggccagaatcagctgtacaatgagctgaatcttggaaggagagaggaatacgacgtgttggacaaacgccgaggaagggaccctgaaatgggtggcaaaccacggaggaagaaccctcaggaaggactgtataacgagctgcagaaagataagatggcggaggcgtactcagagataggcatgaagggagaacgccgtcgaggcaaaggccacgatggcctgtatcaggggttgagcactgccacgaaagacacctatgacgcactgcacatgcaagccttgccaccccggtga

SEQ ID NO: 88 - DNA, 1470 bp, synthetic construct
  source 1..1470: mol_type = other DNA
atgctgttgctggtcaccagcctcctcttgtgtgagcttcctcatccagcctttcttctgattcccgaagtcaaactcgaggagtctggcggtgggttggtgcagccaggtggctccatgaagctgtcatgtgtcgcaagcggcttcacgttctcaaactactggatgaattgggtgagacaatcacccgagaaggggctggaatgggtggcagaaatccgtctgaaaagcaacaactatgctacccattacgcggagtctgtgaagggtcggttcacaattagccgcgacgacagcaagtccagtgtctatctccagatgaacaacctccgagccgaggatactggaaggtactattgcagcagactgcctagcttcgattactggggccaaggcactactttgacagtgtcctcagggagtaccagcgggtccggtaaaccaggctcaggagaaggttccacgaaaggggacattgtgatgacacaggctgctcctagcgttcgggtgacacctggagagagcgtaagtatcagctgcagaagcaccaagtctctcctgcactctaatggcaatacctacctgtactggttccttcagcggccagggcagtctcctcagcttctgatataccgcatgtctaatctggcgtcaggggtacctgacagattctcagggtctggaagcggaaccgcctttactctgcggattacacgggtggaagctgaggatgttgggcgctattactgcatgcagcacttggagtatccgttcacttttggcgcgggtacaaagctggaactcaaaagaatcgaggtgatgtatccacctccctatctggacaacgagaaatccaacggcaccataatccacgtgaaaggcaagcatctgtgtccctctcccctgtttcccgggccgagtaaaccgttttgggttctggtggtagtgggcggtgtcctggcttgctattccctgcttgtcacggtggcctttatcatcttctgggttcgatccaaaaggagcagactgctgcattccgactacatgaatatgactccaagacgccctggaccaacacggaagcactaccaaccgtatgcaccaccccgcgactttgcagcctacaggtctagggtcaagttctcccgcagtgccgatgctcccgcctatcagcaagggcagaatcagctgtacaacgagctcaatctgggacgtcgtgaggaatacgacgttctcgacaagaggcgaggacgggatcccgaaatgggaggcaaacccaggcgcaagaatcctcaagaaggcctgtacaacgaactgcagaaggacaagatggccgaagcttacagtgagattggcatgaagggagagagaaggcgaggcaaaggccacgatggtctttatcagggactgagtaccgccactaaggatacctatgatgccctccacatgcaggcattgccacccaggtga

SEQ ID NO: 89 - DNA, 1482 bp, synthetic construct
  source 1..1482: mol_type = other DNA
atgctgttgctggtcaccagcctcctcttgtgtgagcttcctcatccagcctttcttctgattcccgaagtcaaactcgaggagtctggcggtgggttggtgcagccaggtggctccatgaagctgtcatgtgtcgcaagcggcttcacgttctcaaactactggatgaattgggtgagacaatcacccgagaaggggctggaatgggtggcagaaatccgtctgaaaagcaacaactatgctacccattacgcggagtctgtgaagggtcggttcacaattagccgcgacgacagcaagtccagtgtctatctccagatgaacaacctccgagccgaggatactggaaggtactattgcagcagactgcctagcttcgattactggggccaaggcactactttgacagtgtcctcagggagtaccagcgggtccggtaaaccaggctcaggagaaggttccacgaaaggggacattgtgatgacacaggctgctcctagcgttcgggtgacacctggagagagcgtaagtatcagctgcagaagcaccaagtctctcctgcactctaatggcaatacctacctgtactggttccttcagcggccagggcagtctcctcagcttctgatataccgcatgtctaatctggcgtcaggggtacctgacagattctcagggtctggaagcggaaccgcctttactctgcggattacacgggtggaagctgaggatgttgggcgctattactgcatgcagcacttggagtatccgttcacttttggcgcgggtacaaagctggaactcaaaagaaccacgacgccagcgccgcgaccaccaacaccggcgcccaccatcgcgtcgcagcccctgtccctgcgcccagaggcgtgccggccagcggcggggggcgcagtgcacacgagggggctggacttcgcctgtgatatctacatctgggcgcccttggccgggacttgtggggtccttctcctgtcactggttatcaccctttactgcaaacggggcagaaagaaactcctgtatatattcaaacaaccatttatgagaccagtacaaactactcaagaggaagatggctgtagctgccgatttccagaagaagaagaaggaggatgtgaactgagagtgaagttcagcaggagcgcagacgcccccgcgtaccagcagggccagaaccagctctataacgagctcaatctaggacgaagagaggagtacgatgttttggacaagagacgtggccgggaccctgagatggggggaaagccgagaaggaagaaccctcaggaaggcctgtacaatgaactgcagaaagataagatggcggaggcctacagtgagattgggatgaaaggcgagcgccggaggggcaaggggcacgatggcctttaccagggtctcagtacagccaccaaggacacctacgacgcccttcacatgcaggccctgccccctcgctga

SEQ ID NO: 90 - DNA, 1614 bp, synthetic construct
  source 1..1614: mol_type = other DNA
atgctgttgctggtcaccagcctcctcttgtgtgagcttcctcatccagcctttcttctgattcccgaagtcaaactcgaggagtctggcggtgggttggtgcagccaggtggctccatgaagctgtcatgtgtcgcaagcggcttcacgttctcaaactactggatgaattgggtgagacaatcacccgagaaggggctggaatgggtggcagaaatccgtctgaaaagcaacaactatgctacccattacgcggagtctgtgaagggtcggttcacaattagccgcgacgacagcaagtccagtgtctatctccagatgaacaacctccgagccgaggatactggaaggtactattgcagcagactgcctagcttcgattactggggccaaggcactactttgacagtgtcctcagggagtaccagcgggtccggtaaaccaggctcaggagaaggttccacgaaaggggacattgtgatgacacaggctgctcctagcgttcgggtgacacctggagagagcgtaagtatcagctgcagaagcaccaagtctctcctgcactctaatggcaatacctacctgtactggttccttcagcggccagggcagtctcctcagcttctgatataccgcatgtctaatctggcgtcaggggtacctgacagattctcagggtctggaagcggaaccgcctttactctgcggattacacgggtggaagctgaggatgttgggcgctattactgcatgcagcacttggagtatccgttcacttttggcgcgggtacaaagctggaactcaaaagaaccacgacgccagcgccgcgaccaccaacaccggcgcccaccatcgcgtcgcagcccctgtccctgcgcccagaggcgtgccggccagcggcggggggcgcagtgcacacgagggggctggacttcgcctgtgatttttgggtgctggtggtggttggtggagtcctggcttgctatagcttgctagtaacagtggcctttattattttctgggtgaggagtaagaggagcaggctcctgcacagtgactacatgaacatgactccccgccgccccgggcccacccgcaagcattaccagccctatgccccaccacgcgacttcgcagcctatcgctccaaacggggcagaaagaaactcctgtatatattcaaacaaccatttatgagaccagtacaaactactcaagaggaagatggctgtagctgccgatttccagaagaagaagaaggaggatgtgaactgagagtgaagttcagcaggagcgcagacgcccccgcgtaccagcagggccagaaccagctctataacgagctcaatctaggacgaagagaggagtacgatgttttggacaagagacgtggccgggaccctgagatggggggaaagccgagaaggaagaaccctcaggaaggcctgtacaatgaactgcagaaagataagatggcggaggcctacagtgagattgggatgaaaggcgagcgccggaggggcaaggggcacgatggcctttaccagggtctcagtacagccaccaaggacacctacgacgcccttcacatgcaggccctgccccctcgctga

SEQ ID NO: 91 - DNA, 1491 bp, synthetic construct
  source 1..1491: mol_type = other DNA
atgctgttgctggtcaccagcctcctcttgtgtgagcttcctcatccagcctttcttctgattcccgaagtcaaactcgaggagtctggcggtgggttggtgcagccaggtggctccatgaagctgtcatgtgtcgcaagcggcttcacgttctcaaactactggatgaattgggtgagacaatcacccgagaaggggctggaatgggtggcagaaatccgtctgaaaagcaacaactatgctacccattacgcggagtctgtgaagggtcggttcacaattagccgcgacgacagcaagtccagtgtctatctccagatgaacaacctccgagccgaggatactggaaggtactattgcagcagactgcctagcttcgattactggggccaaggcactactttgacagtgtcctcaggaggtggcggttccggaggaggtggatcaggaggcggaggctctggtggcggtggctcaggtggaggcggctcagacattgtgatgacacaggctgctcctagcgttcgggtgacacctggagagagcgtaagtatcagctgcagaagcaccaagtctctcctgcactctaatggcaatacctacctgtactggttccttcagcggccagggcagtctcctcagcttctgatataccgcatgtctaatctggcgtcaggggtacctgacagattctcagggtctggaagcggaaccgcctttactctgcggattacacgggtggaagctgaggatgttgggcgctattactgcatgcagcacttggagtatccgttcacttttggcgcgggtacaaagctggaactcaaaagaatcgaggtgatgtatccacctccctatctggacaacgagaaatccaacggcaccataatccacgtgaaaggcaagcatctgtgtccctctcccctgtttcccgggccgagtaaaccgttttgggttctggtggtagtgggcggtgtcctggcttgctattccctgcttgtcacggtggcctttatcatcttctgggttcgatccaaaaggagcagactgctgcattccgactacatgaatatgactccaagacgccctggaccaacacggaagcactaccaaccgtatgcaccaccccgcgactttgcagcctacaggtctagggtcaagttctcccgcagtgccgatgctcccgcctatcagcaagggcagaatcagctgtacaacgagctcaatctgggacgtcgtgaggaatacgacgttctcgacaagaggcgaggacgggatcccgaaatgggaggcaaacccaggcgcaagaatcctcaagaaggcctgtacaacgaactgcagaaggacaagatggccgaagcttacagtgagattggcatgaagggagagagaaggcgaggcaaaggccacgatggtctttatcagggactgagtaccgccactaaggatacctatgatgccctccacatgcaggcattgccacccaggtga

SEQ ID NO: 92 - DNA, 1503 bp, synthetic construct
  source 1..1503: mol_type = other DNA
atgctgttgctggtcaccagcctcctcttgtgtgagcttcctcatccagcctttcttctgattcccgaagtcaaactcgaggagtctggcggtgggttggtgcagccaggtggctccatgaagctgtcatgtgtcgcaagcggcttcacgttctcaaactactggatgaattgggtgagacaatcacccgagaaggggctggaatgggtggcagaaatccgtctgaaaagcaacaactatgctacccattacgcggagtctgtgaagggtcggttcacaattagccgcgacgacagcaagtccagtgtctatctccagatgaacaacctccgagccgaggatactggaaggtactattgcagcagactgcctagcttcgattactggggccaaggcactactttgacagtgtcctcaggaggtggcggttccggaggaggtggatcaggaggcggaggctctggtggcggtggctcaggtggaggcggctcagacattgtgatgacacaggctgctcctagcgttcgggtgacacctggagagagcgtaagtatcagctgcagaagcaccaagtctctcctgcactctaatggcaatacctacctgtactggttccttcagcggccagggcagtctcctcagcttctgatataccgcatgtctaatctggcgtcaggggtacctgacagattctcagggtctggaagcggaaccgcctttactctgcggattacacgggtggaagctgaggatgttgggcgctattactgcatgcagcacttggagtatccgttcacttttggcgcgggtacaaagctggaactcaaaagaaccacgacgccagcgccgcgaccaccaacaccggcgcccaccatcgcgtcgcagcccctgtccctgcgcccagaggcgtgccggccagcggcggggggcgcagtgcacacgagggggctggacttcgcctgtgatatctacatctgggcgcccttggccgggacttgtggggtccttctcctgtcactggttatcaccctttactgcaaacggggcagaaagaaactcctgtatatattcaaacaaccatttatgagaccagtacaaactactcaagaggaagatggctgtagctgccgatttccagaagaagaagaaggaggatgtgaactgagagtgaagttcagcaggagcgcagacgcccccgcgtaccagcagggccagaaccagctctataacgagctcaatctaggacgaagagaggagtacgatgttttggacaagagacgtggccgggaccctgagatggggggaaagccgagaaggaagaaccctcaggaaggcctgtacaatgaactgcagaaagataagatggcggaggcctacagtgagattgggatgaaaggcgagcgccggaggggcaaggggcacgatggcctttaccagggtctcagtacagccaccaaggacacctacgacgcccttcacatgcaggccctgccccctcgctga

SEQ ID NO: 93 - DNA, 1635 bp, synthetic construct
  source 1..1635: mol_type = other DNA
atgctgttgctggtcaccagcctcctcttgtgtgagcttcctcatccagcctttcttctgattcccgaagtcaaactcgaggagtctggcggtgggttggtgcagccaggtggctccatgaagctgtcatgtgtcgcaagcggcttcacgttctcaaactactggatgaattgggtgagacaatcacccgagaaggggctggaatgggtggcagaaatccgtctgaaaagcaacaactatgctacccattacgcggagtctgtgaagggtcggttcacaattagccgcgacgacagcaagtccagtgtctatctccagatgaacaacctccgagccgaggatactggaaggtactattgcagcagactgcctagcttcgattactggggccaaggcactactttgacagtgtcctcaggaggtggcggttccggaggaggtggatcaggaggcggaggctctggtggcggtggctcaggtggaggcggctcagacattgtgatgacacaggctgctcctagcgttcgggtgacacctggagagagcgtaagtatcagctgcagaagcaccaagtctctcctgcactctaatggcaatacctacctgtactggttccttcagcggccagggcagtctcctcagcttctgatataccgcatgtctaatctggcgtcaggggtacctgacagattctcagggtctggaagcggaaccgcctttactctgcggattacacgggtggaagctgaggatgttgggcgctattactgcatgcagcacttggagtatccgttcacttttggcgcgggtacaaagctggaactcaaaagaaccacgacgccagcgccgcgaccaccaacaccggcgcccaccatcgcgtcgcagcccctgtccctgcgcccagaggcgtgccggccagcggcggggggcgcagtgcacacgagggggctggacttcgcctgtgatttttgggtgctggtggtggttggtggagtcctggcttgctatagcttgctagtaacagtggcctttattattttctgggtgaggagtaagaggagcaggctcctgcacagtgactacatgaacatgactccccgccgccccgggcccacccgcaagcattaccagccctatgccccaccacgcgacttcgcagcctatcgctccaaacggggcagaaagaaactcctgtatatattcaaacaaccatttatgagaccagtacaaactactcaagaggaagatggctgtagctgccgatttccagaagaagaagaaggaggatgtgaactgagagtgaagttcagcaggagcgcagacgcccccgcgtaccagcagggccagaaccagctctataacgagctcaatctaggacgaagagaggagtacgatgttttggacaagagacgtggccgggaccctgagatggggggaaagccgagaaggaagaaccctcaggaaggcctgtacaatgaactgcagaaagataagatggcggaggcctacagtgagattgggatgaaaggcgagcgccggaggggcaaggggcacgatggcctttaccagggtctcagtacagccaccaaggacacctacgacgcccttcacatgcaggccctgccccctcgctga

SEQ ID NO: 94 - DNA, 1506 bp, synthetic construct
  source 1..1506: mol_type = other DNA
atgctgttgctggtcaccagcctcctcttgtgtgagcttcctcatccagcctttcttctgattcccgaagtcaaactcgaggagtctggcggtgggttggtgcagccaggtggctccatgaagctgtcatgtgtcgcaagcggcttcacgttctcaaactactggatgaattgggtgagacaatcacccgagaaggggctggaatgggtggcagaaatccgtctgaaaagcaacaactatgctacccattacgcggagtctgtgaagggtcggttcacaattagccgcgacgacagcaagtccagtgtctatctccagatgaacaacctccgagccgaggatactggaaggtactattgcagcagactgcctagcttcgattactggggccaaggcactactttgacagtgtcctcaggaggtggcggttccggaggaggtggatcaggaggtggcggttccggaggaggtggatcaggaggtggcggttccggaggaggtggatcagacattgtgatgacacaggctgctcctagcgttcgggtgacacctggagagagcgtaagtatcagctgcagaagcaccaagtctctcctgcactctaatggcaatacctacctgtactggttccttcagcggccagggcagtctcctcagcttctgatataccgcatgtctaatctggcgtcaggggtacctgacagattctcagggtctggaagcggaaccgcctttactctgcggattacacgggtggaagctgaggatgttgggcgctattactgcatgcagcacttggagtatccgttcacttttggcgcgggtacaaagctggaactcaaaagaatcgaggtgatgtatccacctccctatctggacaacgagaaatccaacggcaccataatccacgtgaaaggcaagcatctgtgtccctctcccctgtttcccgggccgagtaaaccgttttgggttctggtggtagtgggcggtgtcctggcttgctattccctgcttgtcacggtggcctttatcatcttctgggttcgatccaaaaggagcagactgctgcattccgactacatgaatatgactccaagacgccctggaccaacacggaagcactaccaaccgtatgcaccaccccgcgactttgcagcctacaggtctagggtcaagttctcccgcagtgccgatgctcccgcctatcagcaagggcagaatcagctgtacaacgagctcaatctgggacgtcgtgaggaatacgacgttctcgacaagaggcgaggacgggatcccgaaatgggaggcaaacccaggcgcaagaatcctcaagaaggcctgtacaacgaactgcagaaggacaagatggccgaagcttacagtgagattggcatgaagggagagagaaggcgaggcaaaggccacgatggtctttatcagggactgagtaccgccactaaggatacctatgatgccctccacatgcaggcattgccacccaggtga

SEQ ID NO: 95 - DNA, 1518 bp, synthetic construct
  source 1..1518: mol_type = other DNA
atgctgttgctggtcaccagcctcctcttgtgtgagcttcctcatccagcctttcttctgattcccgaagtcaaactcgaggagtctggcggtgggttggtgcagccaggtggctccatgaagctgtcatgtgtcgcaagcggcttcacgttctcaaactactggatgaattgggtgagacaatcacccgagaaggggctggaatgggtggcagaaatccgtctgaaaagcaacaactatgctacccattacgcggagtctgtgaagggtcggttcacaattagccgcgacgacagcaagtccagtgtctatctccagatgaacaacctccgagccgaggatactggaaggtactattgcagcagactgcctagcttcgattactggggccaaggcactactttgacagtgtcctcaggaggtggcggttccggaggaggtggatcaggaggtggcggttccggaggaggtggatcaggaggtggcggttccggaggaggtggatcagacattgtgatgacacaggctgctcctagcgttcgggtgacacctggagagagcgtaagtatcagctgcagaagcaccaagtctctcctgcactctaatggcaatacctacctgtactggttccttcagcggccagggcagtctcctcagcttctgatataccgcatgtctaatctggcgtcaggggtacctgacagattctcagggtctggaagcggaaccgcctttactctgcggattacacgggtggaagctgaggatgttgggcgctattactgcatgcagcacttggagtatccgttcacttttggcgcgggtacaaagctggaactcaaaagaaccacgacgccagcgccgcgaccaccaacaccggcgcccaccatcgcgtcgcagcccctgtccctgcgcccagaggcgtgccggccagcggcggggggcgcagtgcacacgagggggctggacttcgcctgtgatatctacatctgggcgcccttggccgggacttgtggggtccttctcctgtcactggttatcaccctttactgcaaacggggcagaaagaaactcctgtatatattcaaacaaccatttatgagaccagtacaaactactcaagaggaagatggctgtagctgccgatttccagaagaagaagaaggaggatgtgaactgagagtgaagttcagcaggagcgcagacgcccccgcgtaccagcagggccagaaccagctctataacgagctcaatctaggacgaagagaggagtacgatgttttggacaagagacgtggccgggaccctgagatggggggaaagccgagaaggaagaaccctcaggaaggcctgtacaatgaactgcagaaagataagatggcggaggcctacagtgagattgggatgaaaggcgagcgccggaggggcaaggggcacgatggcctttaccagggtctcagtacagccaccaaggacacctacgacgcccttcacatgcaggccctgccccctcgctga

SEQ ID NO: 96 - DNA, 1650 bp, synthetic construct
  source 1..1650: mol_type = other DNA
atgctgttgctggtcaccagcctcctcttgtgtgagcttcctcatccagcctttcttctgattcccgaagtcaaactcgaggagtctggcggtgggttggtgcagccaggtggctccatgaagctgtcatgtgtcgcaagcggcttcacgttctcaaactactggatgaattgggtgagacaatcacccgagaaggggctggaatgggtggcagaaatccgtctgaaaagcaacaactatgctacccattacgcggagtctgtgaagggtcggttcacaattagccgcgacgacagcaagtccagtgtctatctccagatgaacaacctccgagccgaggatactggaaggtactattgcagcagactgcctagcttcgattactggggccaaggcactactttgacagtgtcctcaggaggtggcggttccggaggaggtggatcaggaggtggcggttccggaggaggtggatcaggaggtggcggttccggaggaggtggatcagacattgtgatgacacaggctgctcctagcgttcgggtgacacctggagagagcgtaagtatcagctgcagaagcaccaagtctctcctgcactctaatggcaatacctacctgtactggttccttcagcggccagggcagtctcctcagcttctgatataccgcatgtctaatctggcgtcaggggtacctgacagattctcagggtctggaagcggaaccgcctttactctgcggattacacgggtggaagctgaggatgttgggcgctattactgcatgcagcacttggagtatccgttcacttttggcgcgggtacaaagctggaactcaaaagaaccacgacgccagcgccgcgaccaccaacaccggcgcccaccatcgcgtcgcagcccctgtccctgcgcccagaggcgtgccggccagcggcggggggcgcagtgcacacgagggggctggacttcgcctgtgatttttgggtgctggtggtggttggtggagtcctggcttgctatagcttgctagtaacagtggcctttattattttctgggtgaggagtaagaggagcaggctcctgcacagtgactacatgaacatgactccccgccgccccgggcccacccgcaagcattaccagccctatgccccaccacgcgacttcgcagcctatcgctccaaacggggcagaaagaaactcctgtatatattcaaacaaccatttatgagaccagtacaaactactcaagaggaagatggctgtagctgccgatttccagaagaagaagaaggaggatgtgaactgagagtgaagttcagcaggagcgcagacgcccccgcgtaccagcagggccagaaccagctctataacgagctcaatctaggacgaagagaggagtacgatgttttggacaagagacgtggccgggaccctgagatggggggaaagccgagaaggaagaaccctcaggaaggcctgtacaatgaactgcagaaagataagatggcggaggcctacagtgagattgggatgaaaggcgagcgccggaggggcaaggggcacgatggcctttaccagggtctcagtacagccaccaaggacacctacgacgcccttcacatgcaggccctgccccctcgctga

SEQ ID NO: 97 - DNA, 1566 bp, synthetic construct
  source 1..1566: mol_type = other DNA
atgctgttgctggtcaccagcctcctcttgtgtgagcttcctcatccagcctttcttctgattcccgaagtcaaactcgaggagtctggcggtgggttggtgcagccaggtggctccatgaagctgtcatgtgtcgcaagcggcttcacgttctcaaactactggatgaattgggtgagacaatcacccgagaaggggctggaatgggtggcagaaatccgtctgaaaagcaacaactatgctacccattacgcggagtctgtgaagggtcggttcacaattagccgcgacgacagcaagtccagtgtctatctccagatgaacaacctccgagccgaggatactggaaggtactattgcagcagactgcctagcttcgattactggggccaaggcactactttgacagtgtcctcaggaggtggcggttccggaggaggtggatcaggaggtggcggttccggaggaggtggatcaggaggtggcggttccggaggaggtggatcaggaggaggtggatcaggaggaggtggatcaggaggaggtggatcaggaggaggtggatcagacattgtgatgacacaggctgctcctagcgttcgggtgacacctggagagagcgtaagtatcagctgcagaagcaccaagtctctcctgcactctaatggcaatacctacctgtactggttccttcagcggccagggcagtctcctcagcttctgatataccgcatgtctaatctggcgtcaggggtacctgacagattctcagggtctggaagcggaaccgcctttactctgcggattacacgggtggaagctgaggatgttgggcgctattactgcatgcagcacttggagtatccgttcacttttggcgcgggtacaaagctggaactcaaaagaatcgaggtgatgtatccacctccctatctggacaacgagaaatccaacggcaccataatccacgtgaaaggcaagcatctgtgtccctctcccctgtttcccgggccgagtaaaccgttttgggttctggtggtagtgggcggtgtcctggcttgctattccctgcttgtcacggtggcctttatcatcttctgggttcgatccaaaaggagcagactgctgcattccgactacatgaatatgactccaagacgccctggaccaacacggaagcactaccaaccgtatgcaccaccccgcgactttgcagcctacaggtctagggtcaagttctcccgcagtgccgatgctcccgcctatcagcaagggcagaatcagctgtacaacgagctcaatctgggacgtcgtgaggaatacgacgttctcgacaagaggcgaggacgggatcccgaaatgggaggcaaacccaggcgcaagaatcctcaagaaggcctgtacaacgaactgcagaaggacaagatggccgaagcttacagtgagattggcatgaagggagagagaaggcgaggcaaaggccacgatggtctttatcagggactgagtaccgccactaaggatacctatgatgccctccacatgcaggcattgccacccaggtga

SEQ ID NO: 98 - DNA, 1578 bp, synthetic construct
  source 1..1578: mol_type = other DNA
atgctgttgctggtcaccagcctcctcttgtgtgagcttcctcatccagcctttcttctgattcccgaagtcaaactcgaggagtctggcggtgggttggtgcagccaggtggctccatgaagctgtcatgtgtcgcaagcggcttcacgttctcaaactactggatgaattgggtgagacaatcacccgagaaggggctggaatgggtggcagaaatccgtctgaaaagcaacaactatgctacccattacgcggagtctgtgaagggtcggttcacaattagccgcgacgacagcaagtccagtgtctatctccagatgaacaacctccgagccgaggatactggaaggtactattgcagcagactgcctagcttcgattactggggccaaggcactactttgacagtgtcctcaggaggtggcggttccggaggaggtggatcaggaggtggcggttccggaggaggtggatcaggaggtggcggttccggaggaggtggatcaggaggaggtggatcaggaggaggtggatcaggaggaggtggatcaggaggaggtggatcagacattgtgatgacacaggctgctcctagcgttcgggtgacacctggagagagcgtaagtatcagctgcagaagcaccaagtctctcctgcactctaatggcaatacctacctgtactggttccttcagcggccagggcagtctcctcagcttctgatataccgcatgtctaatctggcgtcaggggtacctgacagattctcagggtctggaagcggaaccgcctttactctgcggattacacgggtggaagctgaggatgttgggcgctattactgcatgcagcacttggagtatccgttcacttttggcgcgggtacaaagctggaactcaaaagaaccacgacgccagcgccgcgaccaccaacaccggcgcccaccatcgcgtcgcagcccctgtccctgcgcccagaggcgtgccggccagcggcggggggcgcagtgcacacgagggggctggacttcgcctgtgatatctacatctgggcgcccttggccgggacttgtggggtccttctcctgtcactggttatcaccctttactgcaaacggggcagaaagaaactcctgtatatattcaaacaaccatttatgagaccagtacaaactactcaagaggaagatggctgtagctgccgatttccagaagaagaagaaggaggatgtgaactgagagtgaagttcagcaggagcgcagacgcccccgcgtaccagcagggccagaaccagctctataacgagctcaatctaggacgaagagaggagtacgatgttttggacaagagacgtggccgggaccctgagatggggggaaagccgagaaggaagaaccctcaggaaggcctgtacaatgaactgcagaaagataagatggcggaggcctacagtgagattgggatgaaaggcgagcgccggaggggcaaggggcacgatggcctttaccagggtctcagtacagccaccaaggacacctacgacgcccttcacatgcaggccctgccccctcgctga

SEQ ID NO: 99 - DNA, 1710 bp, synthetic construct
  source 1..1710: mol_type = other DNA
atgctgttgctggtcaccagcctcctcttgtgtgagcttcctcatccagcctttcttctgattcccgaagtcaaactcgaggagtctggcggtgggttggtgcagccaggtggctccatgaagctgtcatgtgtcgcaagcggcttcacgttctcaaactactggatgaattgggtgagacaatcacccgagaaggggctggaatgggtggcagaaatccgtctgaaaagcaacaactatgctacccattacgcggagtctgtgaagggtcggttcacaattagccgcgacgacagcaagtccagtgtctatctccagatgaacaacctccgagccgaggatactggaaggtactattgcagcagactgcctagcttcgattactggggccaaggcactactttgacagtgtcctcaggaggtggcggttccggaggaggtggatcaggaggtggcggttccggaggaggtggatcaggaggtggcggttccggaggaggtggatcaggaggaggtggatcaggaggaggtggatcaggaggaggtggatcaggaggaggtggatcagacattgtgatgacacaggctgctcctagcgttcgggtgacacctggagagagcgtaagtatcagctgcagaagcaccaagtctctcctgcactctaatggcaatacctacctgtactggttccttcagcggccagggcagtctcctcagcttctgatataccgcatgtctaatctggcgtcaggggtacctgacagattctcagggtctggaagcggaaccgcctttactctgcggattacacgggtggaagctgaggatgttgggcgctattactgcatgcagcacttggagtatccgttcacttttggcgcgggtacaaagctggaactcaaaagaaccacgacgccagcgccgcgaccaccaacaccggcgcccaccatcgcgtcgcagcccctgtccctgcgcccagaggcgtgccggccagcggcggggggcgcagtgcacacgagggggctggacttcgcctgtgatttttgggtgctggtggtggttggtggagtcctggcttgctatagcttgctagtaacagtggcctttattattttctgggtgaggagtaagaggagcaggctcctgcacagtgactacatgaacatgactccccgccgccccgggcccacccgcaagcattaccagccctatgccccaccacgcgacttcgcagcctatcgctccaaacggggcagaaagaaactcctgtatatattcaaacaaccatttatgagaccagtacaaactactcaagaggaagatggctgtagctgccgatttccagaagaagaagaaggaggatgtgaactgagagtgaagttcagcaggagcgcagacgcccccgcgtaccagcagggccagaaccagctctataacgagctcaatctaggacgaagagaggagtacgatgttttggacaagagacgtggccgggaccctgagatggggggaaagccgagaaggaagaaccctcaggaaggcctgtacaatgaactgcagaaagataagatggcggaggcctacagtgagattgggatgaaaggcgagcgccggaggggcaaggggcacgatggcctttaccagggtctcagtacagccaccaaggacacctacgacgcccttcacatgcaggccctgccccctcgctga

SEQ ID NO: 100 - DNA, 1479 bp, synthetic construct; identical to SEQ ID NO: 59
  source 1..1479: mol_type = other DNA

SEQ ID NO: 101 - DNA, 1491 bp, synthetic construct
  source 1..1491: mol_type = other DNA
atgttgttgctcgtcacctctcttctgctgtgtgagctccctcatccggccttcctgcttatccccgaagttaagctcgaggagtccggaggagggctggtccagcccggaggtagtatgaagctgtcatgcgtagcctccggcttcacattcagcaattactggatgaactgggtcagacagagtcccgagaaaggtctggaatgggtggccgaaatacggctgaagagcaataactatgccacacattacgcagagtcagtcaagggccgtttcaccattagcagagatgactccaagagtagcgtgtatctgcagatgaacaacctcagggctgaggacactggtcgctactactgctctagactgccctcctttgactactggggacaaggcaccactctgactgtctcaagtgggagcacatctggaagtggcaaacctgggtctggggaaggcagcactaaaggtgatatcgtgatgacacaggcagctccctccgtccaagtgacaccaggcgaatctgtcagcatttcttgtcggtccactaagtctctccttcactctaacgggaatacctacctctactggttcctgcaacgaccaggacaatccccacagctgctcatctatcggatgagcaatctcgccagtggggtgcctgatcggtttagcggtagcggctctggtacggcatttaccctgcgcattacacgcgttgaagcagaggatgttgggagatactattgcatgcagcacctggaatatccctttaccttcggcgctggcacgaagctcgagctgaagagggctgccgctaccacgacgccagcgccgcgaccaccaacaccggcgcccaccatcgcgtcgcagcccctgtccctgcgcccagaggcgtgccggccagcggcggggggcgcagtgcacacgagggggctggacttcgcctgtgatatctacatctgggcgcccttggccgggacttgtggggtccttctcctgtcactggttatcaccctttactgcaaacggggcagaaagaaactcctgtatatattcaaacaaccatttatgagaccagtacaaactactcaagaggaagatggctgtagctgccgatttccagaagaagaagaaggaggatgtgaactgagagtgaagttcagcaggagcgcagacgcccccgcgtaccagcagggccagaaccagctctataacgagctcaatctaggacgaagagaggagtacgatgttttggacaagagacgtggccgggaccctgagatggggggaaagccgagaaggaagaaccctcaggaaggcctgtacaatgaactgcagaaagataagatggcggaggcctacagtgagattgggatgaaaggcgagcgccggaggggcaaggggcacgatggcctttaccagggtctcagtacagccaccaaggacacctacgacgcccttcacatgcaggccctgccccctcgctga

SEQ ID NO: 102 - DNA, 1512 bp, synthetic construct
  source 1..1512: mol_type = other DNA
atgttgttgctcgtcacctctcttctgctgtgtgagctccctcatccggccttcctgcttatccccgaagttaagctcgaggagtccggaggagggctggtccagcccggaggtagtatgaagctgtcatgcgtagcctccggcttcacattcagcaattactggatgaactgggtcagacagagtcccgagaaaggtctggaatgggtggccgaaatacggctgaagagcaataactatgccacacattacgcagagtcagtcaagggccgtttcaccattagcagagatgactccaagagtagcgtgtatctgcagatgaacaacctcagggctgaggacactggtcgctactactgctctagactgccctcctttgactactggggacaaggcaccactctgactgtctcaagtggaggtggcggttccggaggaggtggatcaggaggcggaggctctggtggcggtggctcaggtggaggcggctcagatatcgtgatgacacaggcagctccctccgtccaagtgacaccaggcgaatctgtcagcatttcttgtcggtccactaagtctctccttcactctaacgggaatacctacctctactggttcctgcaacgaccaggacaatccccacagctgctcatctatcggatgagcaatctcgccagtggggtgcctgatcggtttagcggtagcggctctggtacggcatttaccctgcgcattacacgcgttgaagcagaggatgttgggagatactattgcatgcagcacctggaatatccctttaccttcggcgctggcacgaagctcgagctgaagagggctgccgctaccacgacgccagcgccgcgaccaccaacaccggcgcccaccatcgcgtcgcagcccctgtccctgcgcccagaggcgtgccggccagcggcggggggcgcagtgcacacgagggggctggacttcgcctgtgatatctacatctgggcgcccttggccgggacttgtggggtccttctcctgtcactggttatcaccctttactgcaaacggggcagaaagaaactcctgtatatattcaaacaaccatttatgagaccagtacaaactactcaagaggaagatggctgtagctgccgatttccagaagaagaagaaggaggatgtgaactgagagtgaagttcagcaggagcgcagacgcccccgcgtaccagcagggccagaaccagctctataacgagctcaatctaggacgaagagaggagtacgatgttttggacaagagacgtggccgggaccctgagatggggggaaagccgagaaggaagaaccctcaggaaggcctgtacaatgaactgcagaaagataagatggcggaggcctacagtgagattgggatgaaaggcgagcgccggaggggcaaggggcacgatggcctttaccagggtctcagtacagccaccaaggacacctacgacgcccttcacatgcaggccctgccccctcgctga

SEQ ID NO: 103 - DNA, 1587 bp, synthetic construct
  source 1..1587: mol_type = other DNA
atgttgttgctcgtcacctctcttctgctgtgtgagctccctcatccggccttcctgcttatccccgaagttaagctcgaggagtccggaggagggctggtccagcccggaggtagtatgaagctgtcatgcgtagcctccggcttcacattcagcaattactggatgaactgggtcagacagagtcccgagaaaggtctggaatgggtggccgaaatacggctgaagagcaataactatgccacacattacgcagagtcagtcaagggccgtttcaccattagcagagatgactccaagagtagcgtgtatctgcagatgaacaacctcagggctgaggacactggtcgctactactgctctagactgccctcctttgactactggggacaaggcaccactctgactgtctcaagtggaggtggcggttccggaggaggtggatcaggaggtggcggttccggaggaggtggatcaggaggtggcggttccggaggaggtggatcaggaggaggtggatcaggaggaggtggatcaggaggaggtggatcaggaggaggtggatcagatatcgtgatgacacaggcagctccctccgtccaagtgacaccaggcgaatctgtcagcatttcttgtcggtccactaagtctctccttcactctaacgggaatacctacctctactggttcctgcaacgaccaggacaatccccacagctgctcatctatcggatgagcaatctcgccagtggggtgcctgatcggtttagcggtagcggctctggtacggcatttaccctgcgcattacacgcgttgaagcagaggatgttgggagatactattgcatgcagcacctggaatatccctttaccttcggcgctggcacgaagctcgagctgaagagggctgccgctaccacgacgccagcgccgcgaccaccaacaccggcgcccaccatcgcgtcgcagcccctgtccctgcgcccagaggcgtgccggccagcggcggggggcgcagtgcacacgagggggctggacttcgcctgtgatatctacatctgggcgcccttggccgggacttgtggggtccttctcctgtcactggttatcaccctttactgcaaacggggcagaaagaaactcctgtatatattcaaacaaccatttatgagaccagtacaaactactcaagaggaagatggctgtagctgccgatttccagaagaagaagaaggaggatgtgaactgagagtgaagttcagcaggagcgcagacgcccccgcgtaccagcagggccagaaccagctctataacgagctcaatctaggacgaagagaggagtacgatgttttggacaagagacgtggccgggaccctgagatggggggaaagccgagaaggaagaaccctcaggaaggcctgtacaatgaactgcagaaagataagatggcggaggcctacagtgagattgggatgaaaggcgagcgccggaggggcaaggggcacgatggcctttaccagggtctcagtacagccaccaaggacacctacgacgcccttcacatgcaggccctgccccctcgctga

SEQ ID NO: 104 - protein, 492 aa, synthetic construct
MLLLVTSLLLCELPHPAFLLIPEVKLEESGGGLVQPGGSMKLSCVASGFTFSNYWMNWVRQSPEKGLEWVAEIRLKSNNYATHYAESVKGRFTISRDDSKSSVYLQMNNLRAEDTGIYYCSRLPSFDYWGQGTTLTVSSGSTSGSGKPGSGEGSTKGDIVMTQAAPSVPVTPGESVSISCRSTKSLLHSNGNTYLYWFLQRPGQSPQLLIYRMSNLASGVPDRFSGSGSGTAFTLRITRVEAEDVGIYYCMQHLEYPFTFGAGTKLELKRAAAIEVMYPPPYLDNEKSNGTIIHVKGKHLCPSPLFPGPSKPFWVLVVVGGVLACYSLLVTVAFIIFWVRSKRSRLLHSDYMNMTPRRPGPTRKHYQPYAPPRDFAAYRSRVKFSRSADAPAYQQGQNQLYNELNLGRREEYDVLDKRRGRDPEMGGKPRRKNPQEGLYNELQKDKMAEAYSEIGMKGERRRGKGHDGLYQGLSTATKDTYDALHMQALPPR

SEQ ID NO: 105 - protein, 492 aa, synthetic construct
MLLLVTSLLLCELPHPAFLLIPDIVMTQAAPSVPVTPGESVSISCRSTKSLLHSNGNTYLYWFLQRPGQSPQLLIYRMSNLASGVPDRFSGSGSGTAFTLRITRVEAEDVGIYYCMQHLEYPFTFGAGTKLELKRGSTSGSGKPGSGEGSTKGEVKLEESGGGLVQPGGSMKLSCVASGFTFSNYWMNWVRQSPEKGLEWVAEIRLKSNNYATHYAESVKGRFTISRDDSKSSVYLQMNNLRAEDTGIYYCSRLPSFDYWGQGTTLTVSSAAAIEVMYPPPYLDNEKSNGTIIHVKGKHLCPSPLFPGPSKPFWVLVVVGGVLACYSLLVTVAFIIFWVRSKRSRLLHSDYMNMTPRRPGPTRKHYQPYAPPRDFAAYRSRVKFSRSADAPAYQQGQNQLYNELNLGRREEYDVLDKRRGRDPEMGGKPRRKNPQEGLYNELQKDKMAEAYSEIGMKGERRRGKGHDGLYQGLSTATKDTYDALHMQALPPR

SEQ ID NO: 106 - protein, 492 aa, synthetic construct; identical to SEQ ID NO: 104

SEQ ID NO: 107 - protein, 484 aa, synthetic construct
MLLLVTSLLLCELPHPAFLLIPEVKLEESGGGLVQPGGSMKLSCVASGFTFSNYWMNWVRQSPEKGLEWVAEIRLKSNNYATHYAESVKGRFTISRDDSKSSVYLQMNNLRAEDTGIYYCSRLPSFDYWGQGTTLTVSSGGGGSGGGGSDIVMTQAAPSVPVTPGESVSISCRSTKSLLHSNGNTYLYWFLQRPGQSPQLLIYRMSNLASGVPDRFSGSGSGTAFTLRITRVEAEDVGIYYCMQHLEYPFTFGAGTKLELKRAAAIEVMYPPPYLDNEKSNGTIIHVKGKHLCPSPLFPGPSKPFWVLVVVGGVLACYSLLVTVAFIIFWVRSKRSRLLHSDYMNMTPRRPGPTRKHYQPYAPPRDFAAYRSRVKFSRSADAPAYQQGQNQLYNELNLGRREEYDVLDKRRGRDPEMGGKPRRKNPQEGLYNELQKDKMAEAYSEIGMKGERRRGKGHDGLYQGLSTATKDTYDALHMQALPPR

SEQ ID NO: 108 - protein, 489 aa, synthetic construct
MLLLVTSLLLCELPHPAFLLIPEVKLEESGGGLVQPGGSMKLSCVASGFTFSNYWMNWVRQSPEKGLEWVAEIRLKSNNYATHYAESVKGRFTISRDDSKSSVYLQMNNLRAEDTGIYYCSRLPSFDYWGQGTTLTVSSGGGGSGGGGSGGGGSDIVMTQAAPSVPVTPGESVSISCRSTKSLLHSNGNTYLYWFLQRPGQSPQLLIYRMSNLASGVPDRFSGSGSGTAFTLRITRVEAEDVGIYYCMQHLEYPFTFGAGTKLELKRAAAIEVMYPPPYLDNEKSNGTIIHVKGKHLCPSPLFPGPSKPFWVLVVVGGVLACYSLLVTVAFIIFWVRSKRSRLLHSDYMNMTPRRPGPTRKHYQPYAPPRDFAAYRSRVKFSRSADAPAYQQGQNQLYNELNLGRREEYDVLDKRRGRDPEMGGKPRRKNPQEGLYNELQKDKMAEAYSEIGMKGERRRGKGHDGLYQGLSTATKDTYDALHMQALPPR

SEQ ID NO: 109 - protein, 494 aa, synthetic construct
MLLLVTSLLLCELPHPAFLLIPEVKLEESGGGLVQPGGSMKLSCVASGFTFSNYWMNWVRQSPEKGLEWVAEIRLKSNNYATHYAESVKGRFTISRDDSKSSVYLQMNNLRAEDTGIYYCSRLPSFDYWGQGTTLTVSSGGGGSGGGGSGGGGSGGGGSDIVMTQAAPSVPVTPGESVSISCRSTKSLLHSNGNTYLYWFLQRPGQSPQLLIYRMSNLASGVPDRFSGSGSGTAFTLRITRVEAEDVGIYYCMQHLEYPFTFGAGTKLELKRAAAIEVMYPPPYLDNEKSNGTIIHVKGKHLCPSPLFPGPSKPFWVLVVVGGVLACYSLLVTVAFIIFWVRSKRSRLLHSDYMNMTPRRPGPTRKHYQPYAPPRDFAAYRSRVKFSRSADAPAYQQGQNQLYNELNLGRREEYDVLDKRRGRDPEMGGKPRRKNPQEGLYNELQKDKMAEAYSEIGMKGERRRGKGHDGLYQGLSTATKDTYDALHMQALPPR

SEQ ID NO: 110 - protein, 499 aa, synthetic construct
MLLLVTSLLLCELPHPAFLLIPEVKLEESGGGLVQPGGSMKLSCVASGFTFSNYWMNWVRQSPEKGLEWVAEIRLKSNNYATHYAESVKGRFTISRDDSKSSVYLQMNNLRAEDTGIYYCSRLPSFDYWGQGTTLTVSSGGGGSGGGGSGGGGSGGGGSGGGGSDIVMTQAAPSVPVTPGESVSISCRSTKSLLHSNGNTYLYWFLQRPGQSPQLLIYRMSNLASGVPDRFSGSGSGTAFTLRITRVEAEDVGIYYCMQHLEYPFTFGAGTKLELKRAAAIEVMYPPPYLDNEKSNGTIIHVKGKHLCPSPLFPGPSKPFWVLVVVGGVLACYSLLVTVAFIIFWVRSKRSRLLHSDYMNMTPRRPGPTRKHYQPYAPPRDFAAYRSRVKFSRSADAPAYQQGQNQLYNELNLGRREEYDVLDKRRGRDPEMGGKPRRKNPQEGLYNELQKDKMAEAYSEIGMKGERRRGKGHDGLYQGLSTATKDTYDALHMQALPPR

SEQ ID NO: 111 - protein, 494 aa, synthetic construct; identical to SEQ ID NO: 109

SEQ ID NO: 112 - protein, 499 aa, synthetic construct; identical to SEQ ID NO: 110

SEQ ID NO: 113 - protein, 504 aa, synthetic construct
MLLLVTSLLLCELPHPAFLLIPEVKLEESGGGLVQPGGSMKLSCVASGFTFSNYWMNWVRQSPEKGLEWVAEIRLKSNNYATHYAESVKGRFTISRDDSKSSVYLQMNNLRAEDTGIYYCSRLPSFDYWGQGTTLTVSSGGGGSGGGGSGGGGSGGGGSGGGGSGGGGSDIVMTQAAPSVPVTPGESVSISCRSTKSLLHSNGNTYLYWFLQRPGQSPQLLIYRMSNLASGVPDRFSGSGSGTAFTLRITRVEAEDVGIYYCMQHLEYPFTFGAGTKLELKRAAAIEVMYPPPYLDNEKSNGTIIHVKGKHLCPSPLFPGPSKPFWVLVVVGGVLACYSLLVTVAFIIFWVRSKRSRLLHSDYMNMTPRRPGPTRKHYQPYAPPRDFAAYRSRVKFSRSADAPAYQQGQNQLYNELNLGRREEYDVLDKRRGRDPEMGGKPRRKNPQEGLYNELQKDKMAEAYSEIGMKGERRRGKGHDGLYQGLSTATKDTYDALHMQALPPR

SEQ ID NO: 114 - protein, 509 aa, synthetic construct
MLLLVTSLLLCELPHPAFLLIPEVKLEESGGGLVQPGGSMKLSCVASGFTFSNYWMNWVRQSPEKGLEWVAEIRLKSNNYATHYAESVKGRFTISRDDSKSSVYLQMNNLRAEDTGIYYCSRLPSFDYWGQGTTLTVSSGGGGSGGGGSGGGGSGGGGSGGGGSGGGGSGGGGSDIVMTQAAPSVPVTPGESVSISCRSTKSLLHSNGNTYLYWFLQRPGQSPQLLIYRMSNLASGVPDRFSGSGSGTAFTLRITRVEAEDVGIYYCMQHLEYPFTFGAGTKLELKRAAAIEVMYPPPYLDNEKSNGTIIHVKGKHLCPSPLFPGPSKPFWVLVVVGGVLACYSLLVTVAFIIFWVRSKRSRLLHSDYMNMTPRRPGPTRKHYQPYAPPRDFAAYRSRVKFSRSADAPAYQQGQNQLYNELNLGRREEYDVLDKRRGRDPEMGGKPRRKNPQEGLYNELQKDKMAEAYSEIGMKGERRRGKGHDGLYQGLSTATKDTYDALHMQALPPR

SEQ ID NO: 115 - protein, 514 aa, synthetic construct
MLLLVTSLLLCELPHPAFLLIPEVKLEESGGGLVQPGGSMKLSCVASGFTFSNYWMNWVRQSPEKGLEWVAEIRLKSNNYATHYAESVKGRFTISRDDSKSSVYLQMNNLRAEDTGIYYCSRLPSFDYWGQGTTLTVSSGGGGSGGGGSGGGGSGGGGSGGGGSGGGGSGGGGSGGGGSDIVMTQAAPSVPVTPGESVSISCRSTKSLLHSNGNTYLYWFLQRPGQSPQLLIYRMSNLASGVPDRFSGSGSGTAFTLRITRVEAEDVGIYYCMQHLEYPFTFGAGTKLELKRAAAIEVMYPPPYLDNEKSNGTIIHVKGKHLCPSPLFPGPSKPFWVLVVVGGVLACYSLLVTVAFIIFWVRSKRSRLLHSDYMNMTPRRPGPTRKHYQPYAPPRDFAAYRSRVKFSRSADAPAYQQGQNQLYNELNLGRREEYDVLDKRRGRDPEMGGKPRRKNPQEGLYNELQKDKMAEAYSEIGMKGERRRGKGHDGLYQGLSTATKDTYDALHMQALPPR

SEQ ID NO: 116 - protein, 524 aa, synthetic construct
MLLLVTSLLLCELPHPAFLLIPEVKLEESGGGLVQPGGSMKLSCVASGFTFSNYWMNWVRQSPEKGLEWVAEIRLKSNNYATHYAESVKGRFTISRDDSKSSVYLQMNNLRAEDTGIYYCSRLPSFDYWGQGTTLTVSSGGGGSGGGGSGGGGSGGGGSGGGGSGGGGSGGGGSGGGGSGGGGSGGGGSDIVMTQAAPSVPVTPGESVSISCRSTKSLLHSNGNTYLYWFLQRPGQSPQLLIYRMSNLASGVPDRFSGSGSGTAFTLRITRVEAEDVGIYYCMQHLEYPFTFGAGTKLELKRAAAIEVMYPPPYLDNEKSNGTIIHVKGKHLCPSPLFPGPSKPFWVLVVVGGVLACYSLLVTVAFIIFWVRSKRSRLLHSDYMNMTPRRPGPTRKHYQPYAPPRDFAAYRSRVKFSRSADAPAYQQGQNQLYNELNLGRREEYDVLDKRRGRDPEMGGKPRRKNPQEGLYNELQKDKMAEAYSEIGMKGERRRGKGHDGLYQGLSTATKDTYDALHMQALPPR

SEQ ID NO: 117 - protein, 492 aa, synthetic construct
MLLLVTSLLLCELPHPAFLLIPEVKLEESGGGLVQPGGSMKLSCVASGFTFSNYWMNWVRQSPEKGLEWVAEIRLKSNNYATHYAESVKGRFTISRDDSKSSVYLQMNNLRAEDTGRYYCSRLPSFDYWGQGTTLTVSSGSTSGSGKPGSGEGSTKGDIVMTQAAPSVRVTPGESVSISCRSTKSLLHSNGNTYLYWFLQRPGQSPQLLIYRMSNLASGVPDRFSGSGSGTAFTLRITRVEAEDVGRYYCMQHLEYPFTFGAGTKLELKRAAAIEVMYPPPYLDNEKSNGTIIHVKGKHLCPSPLFPGPSKPFWVLVVVGGVLACYSLLVTVAFIIFWVRSKRSRLLHSDYMNMTPRRPGPTRKHYQPYAPPRDFAAYRSRVKFSRSADAPAYQQGQNQLYNELNLGRREEYDVLDKRRGRDPEMGGKPRRKNPQEGLYNELQKDKMAEAYSEIGMKGERRRGKGHDGLYQGLSTATKDTYDALHMQALPPR

SEQ ID NO: 118 - protein, 492 aa, synthetic construct
MLLLVTSLLLCELPHPAFLLIPEVKLEESGGGLVQPGGSMKLSCVASGFTFSNYWMNWVRQSPEKGLEWVAEIRLKSNNYATHYAESVKGRFTISRDDSKSSVYLQMNNLRAEDTGRYYCSRLPSFDYWGQGTTLTVSSGSTSGSGKPGSGEGSTKGDIVMTQAAPSVQVTPGESVSISCRSTKSLLHSNGNTYLYWFLQRPGQSPQLLIYRMSNLASGVPDRFSGSGSGTAFTLRITRVEAEDVGRYYCMQHLEYPFTFGAGTKLELKRAAAIEVMYPPPYLDNEKSNGTIIHVKGKHLCPSPLFPGPSKPFWVLVVVGGVLACYSLLVTVAFIIFWVRSKRSRLLHSDYMNMTPRRPGPTRKHYQPYAPPRDFAAYRSRVKFSRSADAPAYQQGQNQLYNELNLGRREEYDVLDKRRGRDPEMGGKPRRKNPQEGLYNELQKDKMAEAYSEIGMKGERRRGKGHDGLYQGLSTATKDTYDALHMQALPPR

SEQ ID NO: 119 - protein, 486 aa, synthetic construct
MALPVTALLLPLALLLHAARPDIQMTQTTSSLSASLGDRVTISCRASQDISKYLNWYQQKPDGTVKLLIYHTSRLHSGVPSRFSGSGSGTDYSLTISNLEQEDIATYFCQQGNTLPYTFGGGTKLEITGGGGSGGGGSGGGGSEVKLQESGPGLVAPSQSLSVTCTVSGVSLPDYGVSWIRQPPRKGLEWLGVIWGSETTYYNSALKSRLTIIKDNSKSQVFLKMNSLQTDDTAIYYCAKHYYYGGSYAMDYWGQGTSVTVSSTTTPAPRPPTPAPTIASQPLSLRPEACRPAAGGAVHTRGLDFACDIYIWAPLAGTCGVLLLSLVITLYCKRGRKKLLYIFKQPFMRPVQTTQEEDGCSCRFPEEEEGGCELRVKFSRSADAPAYKQGQNQLYNELNLGRREEYDVLDKRRGRDPEMGGKPRRKNPQEGLYNELQKDKMAEAYSEIGMKGERRRGKGHDGLYQGLSTATKDTYDALHMQALPPR

SEQ ID NO: 120 - protein, 489 aa, synthetic construct
MLLLVTSLLLCELPHPAFLLIPEVKLEESGGGLVQPGGSMKLSCVASGFTFSNYWMNWVRQSPEKGLEWVAEIRLKSNNYATHYAESVKGRFTISRDDSKSSVYLQMNNLRAEDTGIYYCSRLPSFDYWGQGTTLTVSSGSTSGSGKPGSGEGSTKGDIVMTQAAPSVPVTPGESVSISCRSTKSLLHSNGNTYLYWFLQRPGQSPQLLIYRMSNLASGVPDRFSGSGSGTAFTLRITRVEAEDVGIYYCMQHLEYPFTFGAGTKLELKRIEVMYPPPYLDNEKSNGTIIHVKGKHLCPSPLFPGPSKPFWVLVVVGGVLACYSLLVTVAFIIFWVRSKRSRLLHSDYMNMTPRRPGPTRKHYQPYAPPRDFAAYRSRVKFSRSADAPAYQQGQNQLYNELNLGRREEYDVLDKRRGRDPEMGGKPRRKNPQEGLYNELQKDKMAEAYSEIGMKGERRRGKGHDGLYQGLSTATKDTYDALHMQALPPR

SEQ ID NO: 121 - protein, 493 aa, synthetic construct
MLLLVTSLLLCELPHPAFLLIPEVKLEESGGGLVQPGGSMKLSCVASGFTFSNYWMNWVRQSPEKGLEWVAEIRLKSNNYATHYAESVKGRFTISRDDSKSSVYLQMNNLRAEDTGIYYCSRLPSFDYWGQGTTLTVSSGSTSGSGKPGSGEGSTKGDIVMTQAAPSVPVTPGESVSISCRSTKSLLHSNGNTYLYWFLQRPGQSPQLLIYRMSNLASGVPDRFSGSGSGTAFTLRITRVEAEDVGIYYCMQHLEYPFTFGAGTKLELKRTTTPAPRPPTPAPTIASQPLSLRPEACRPAAGGAVHTRGLDFACDIYIWAPLAGTCGVLLLSLVITLYCKRGRKKLLYIFKQPFMRPVQTTQEEDGCSCRFPEEEEGGCELRVKFSRSADAPAYQQGQNQLYNELNLGRREEYDVLDKRRGRDPEMGGKPRRKNPQEGLYNELQKDKMAEAYSEIGMKGERRRGKGHDGLYQGLSTATKDTYDALHMQALPPR

SEQ ID NO: 122 - protein, 537 aa, synthetic construct
MLLLVTSLLLCELPHPAFLLIPEVKLEESGGGLVQPGGSMKLSCVASGFTFSNYWMNWVRQSPEKGLEWVAEIRLKSNNYATHYAESVKGRFTISRDDSKSSVYLQMNNLRAEDTGIYYCSRLPSFDYWGQGTTLTVSSGSTSGSGKPGSGEGSTKGDIVMTQAAPSVPVTPGESVSISCRSTKSLLHSNGNTYLYWFLQRPGQSPQLLIYRMSNLASGVPDRFSGSGSGTAFTLRITRVEAEDVGIYYCMQHLEYPFTFGAGTKLELKRTTTPAPRPPTPAPTIASQPLSLRPEACRPAAGGAVHTRGLDFACDFWVLVVVGGVLACYSLLVTVAFIIFWVRSKRSRLLHSDYMNMTPRRPGPTRKHYQPYAPPRDFAAYRSKRGRKKLLYIFKQPFMRPVQTTQEEDGCSCRFPEEEEGGCELRVKFSRSADAPAYQQGQNQLYNELNLGRREEYDVLDKRRGRDPEMGGKPRRKNPQEGLYNELQKDKMAEAYSEIGMKGERRRGKGHDGLYQGLSTATKDTYDALHMQALPPR

SEQ ID NO: 123 - protein, 491 aa, synthetic construct
MLLLVTSLLLCELPHPAFLLIPEVKLEESGGGLVQPGGSMKLSCVASGFTFSNYWMNWVRQSPEKGLEWVAEIRLKSNNYATHYAESVKGRFTISRDDSKSSVYLQMNNLRAEDTGIYYCSRLPSFDYWGQGTTLTVSSGGGGSGGGGSGGGGSGGGGSDIVMTQAAPSVPVTPGESVSISCRSTKSLLHSNGNTYLYWFLQRPGQSPQLLIYRMSNLASGVPDRFSGSGSGTAFTLRITRVEAEDVGIYYCMQHLEYPFTFGAGTKLELKRIEVMYPPPYLDNEKSNGTIIHVKGKHLCPSPLFPGPSKPFWVLVVVGGVLACYSLLVTVAFIIFWVRSKRSRLLHSDYMNMTPRRPGPTRKHYQPYAPPRDFAAYRSRVKFSRSADAPAYQQGQNQLYNELNLGRREEYDVLDKRRGRDPEMGGKPRRKNPQEGLYNELQKDKMAEAYSEIGMKGERRRGKGHDGLYQGLSTATKDTYDALHMQALPPR

SEQ ID NO: 124 - protein, 495 aa, synthetic construct
MLLLVTSLLLCELPHPAFLLIPEVKLEESGGGLVQPGGSMKLSCVASGFTFSNYWMNWVRQSPEKGLEWVAEIRLKSNNYATHYAESVKGRFTISRDDSKSSVYLQMNNLRAEDTGIYYCSRLPSFDYWGQGTTLTVSSGGGGSGGGGSGGGGSGGGGSDIVMTQAAPSVPVTPGESVSISCRSTKSLLHSNGNTYLYWFLQRPGQSPQLLIYRMSNLASGVPDRFSGSGSGTAFTLRITRVEAEDVGIYYCMQHLEYPFTFGAGTKLELKRTTTPAPRPPTPAPTIASQPLSLRPEACRPAAGGAVHTRGLDFACDIYIWAPLAGTCGVLLLSLVITLYCKRGRKKLLYIFKQPFMRPVQTTQEEDGCSCRFPEEEEGGCELRVKFSRSADAPAYQQGQNQLYNELNLGRREEYDVLDKRRGRDPEMGGKPRRKNPQEGLYNELQKDKMAEAYSEIGMKGERRRGKGHDGLYQGLSTATKDTYDALHMQALPPR

SEQ ID NO: 125 - protein, 539 aa, synthetic construct
MLLLVTSLLLCELPHPAFLLIPEVKLEESGGGLVQPGGSMKLSCVASGFTFSNYWMNWVRQSPEKGLEWVAEIRLKSNNYATHYAESVKGRFTISRDDSKSSVYLQMNNLRAEDTGIYYCSRLPSFDYWGQGTTLTVSSGGGGSGGGGSGGGGSGGGGSDIVMTQAAPSVPVTPGESVSISCRSTKSLLHSNGNTYLYWFLQRPGQSPQLLIYRMSNLASGVPDRFSGSGSGTAFTLRITRVEAEDVGIYYCMQHLEYPFTFGAGTKLELKRTTTPAPRPPTPAPTIASQPLSLRPEACRPAAGGAVHTRGLDFACDFWVLVVVGGVLACYSLLVTVAFIIFWVRSKRSRLLHSDYMNMTPRRPGPTRKHYQPYAPPRDFAAYRSKRGRKKLLYIFKQPFMRPVQTTQEEDGCSCRFPEEEEGGCELRVKFSRSADAPAYQQGQNQLYNELNLGRREEYDVLDKRRGRDPEMGGKPRRKNPQEGLYNELQKDKMAEAYSEIGMKGERRRGKGHDGLYQGLSTATKDTYDALHMQALPPR

SEQ ID NO: 126 - protein, 496 aa, synthetic construct
MLLLVTSLLLCELPHPAFLLIPEVKLEESGGGLVQPGGSMKLSCVASGFTFSNYWMNWVRQSPEKGLEWVAEIRLKSNNYATHYAESVKGRFTISRDDSKSSVYLQMNNLRAEDTGIYYCSRLPSFDYWGQGTTLTVSSGGGGSGGGGSGGGGSGGGGSGGGGSDIVMTQAAPSVPVTPGESVSISCRSTKSLLHSNGNTYLYWFLQRPGQSPQLLIYRMSNLASGVPDRFSGSGSGTAFTLRITRVEAEDVGIYYCMQHLEYPFTFGAGTKLELKRIEVMYPPPYLDNEKSNGTIIHVKGKHLCPSPLFPGPSKPFWVLVVVGGVLACYSLLVTVAFIIFWVRSKRSRLLHSDYMNMTPRRPGPTRKHYQPYAPPRDFAAYRSRVKFSRSADAPAYQQGQNQLYNELNLGRREEYDVLDKRRGRDPEMGGKPRRKNPQEGLYNELQKDKMAEAYSEIGMKGERRRGKGHDGLYQGLSTATKDTYDALHMQALPPR

SEQ ID NO: 127 - protein, 500 aa, synthetic construct
MLLLVTSLLLCELPHPAFLLIPEVKLEESGGGLVQPGGSMKLSCVASGFTFSNYWMNWVRQSPEKGLEWVAEIRLKSNNYATHYAESVKGRFTISRDDSKSSVYLQMNNLRAEDTGIYYCSRLPSFDYWGQGTTLTVSSGGGGSGGGGSGGGGSGGGGSGGGGSDIVMTQAAPSVPVTPGESVSISCRSTKSLLHSNGNTYLYWFLQRPGQSPQLLIYRMSNLASGVPDRFSGSGSGTAFTLRITRVEAEDVGIYYCMQHLEYPFTFGAGTKLELKRTTTPAPRPPTPAPTIASQPLSLRPEACRPAAGGAVHTRGLDFACDIYIWAPLAGTCGVLLLSLVITLYCKRGRKKLLYIFKQPFMRPVQTTQEEDGCSCRFPEEEEGGCELRVKFSRSADAPAYQQGQNQLYNELNLGRREEYDVLDKRRGRDPEMGGKPRRKNPQEGLYNELQKDKMAEAYSEIGMKGERRRGKGHDGLYQGLSTATKDTYDALHMQALPPR

SEQ ID NO: 128 - protein, 544 aa, synthetic construct
MLLLVTSLLLCELPHPAFLLIPEVKLEESGGGLVQPGGSMKLSCVASGFTFSNYWMNWVRQSPEKGLEWVAEIRLKSNNYATHYAESVKGRFTISRDDSKSSVYLQMNNLRAEDTGIYYCSRLPSFDYWGQGTTLTVSSGGGGSGGGGSGGGGSGGGGSGGGGSDIVMTQAAPSVPVTPGESVSISCRSTKSLLHSNGNTYLYWFLQRPGQSPQLLIYRMSNLASGVPDRFSGSGSGTAFTLRITRVEAEDVGIYYCMQHLEYPFTFGAGTKLELKRTTTPAPRPPTPAPTIASQPLSLRPEACRPAAGGAVHTRGLDFACDFWVLVVVGGVLACYSLLVTVAFIIFWVRSKRSRLLHSDYMNMTPRRPGPTRKHYQPYAPPRDFAAYRSKRGRKKLLYIFKQPFMRPVQTTQEEDGCSCRFPEEEEGGCELRVKFSRSADAPAYQQGQNQLYNELNLGRREEYDVLDKRRGRDPEMGGKPRRKNPQEGLYNELQKDKMAEAYSEIGMKGERRRGKGHDGLYQGLSTATKDTYDALHMQALPPR

SEQ ID NO: 129 - protein, 521 aa, synthetic construct
MLLLVTSLLLCELPHPAFLLIPEVKLEESGGGLVQPGGSMKLSCVASGFTFSNYWMNWVRQSPEKGLEWVAEIRLKSNNYATHYAESVKGRFTISRDDSKSSVYLQMNNLRAEDTGIYYCSRLPSFDYWGQGTTLTVSSGGGGSGGGGSGGGGSGGGGSGGGGSGGGGSGGGGSGGGGSGGGGSGGGGSDIVMTQAAPSVPVTPGESVSISCRSTKSLLHSNGNTYLYWFLQRPGQSPQLLIYRMSNLASGVPDRFSGSGSGTAFTLRITRVEAEDVGIYYCMQHLEYPFTFGAGTKLELKRIEVMYPPPYLDNEKSNGTIIHVKGKHLCPSPLFPGPSKPFWVLVVVGGVLACYSLLVTVAFIIFWVRSKRSRLLHSDYMNMTPRRPGPTRKHYQPYAPPRDFAAYRSRVKFSRSADAPAYQQGQNQLYNELNLGRREEYDVLDKRRGRDPEMGGKPRRKNPQEGLYNELQKDKMAEAYSEIGMKGERRRGKGHDGLYQGLSTATKDTYDALHMQALPPR

SEQ ID NO: 130 - protein, 525 aa, synthetic construct
MLLLVTSLLLCELPHPAFLLIPEVKLEESGGGLVQPGGSMKLSCVASGFTFSNYWMNWVRQSPEKGLEWVAEIRLKSNNYATHYAESVKGRFTISRDDSKSSVYLQMNNLRAEDTGIYYCSRLPSFDYWGQGTTLTVSSGGGGSGGGGSGGGGSGGGGSGGGGSGGGGSGGGGSGGGGSGGGGSGGGGSDIVMTQAAPSVPVTPGESVSISCRSTKSLLHSNGNTYLYWFLQRPGQSPQLLIYRMSNLASGVPDRFSGSGSGTAFTLRITRVEAEDVGIYYCMQHLEYPFTFGAGTKLELKRTTTPAPRPPTPAPTIASQPLSLRPEACRPAAGGAVHTRGLDFACDIYIWAPLAGTCGVLLLSLVITLYCKRGRKKLLYIFKQPFMRPVQTTQEEDGCSCRFPEEEEGGCELRVKFSRSADAPAYQQGQNQLYNELNLGRREEYDVLDKRRGRDPEMGGKPRRKNPQEGLYNELQKDKMAEAYSEIGMKGERRRGKGHDGLYQGLSTATKDTYDALHMQALPPR

SEQ ID NO: 131 - protein, 569 aa, synthetic construct
MLLLVTSLLLCELPHPAFLLIPEVKLEESGGGLVQPGGSMKLSCVASGFTFSNYWMNWVRQSPEKGLEWVAEIRLKSNNYATHYAESVKGRFTISRDDSKSSVYLQMNNLRAEDTGIYYCSRLPSFDYWGQGTTLTVSSGGGGSGGGGSGGGGSGGGGSGGGGSGGGGSGGGGSGGGGSGGGGSGGGGSDIVMTQAAPSVPVTPGESVSISCRSTKSLLHSNGNTYLYWFLQRPGQSPQLLIYRMSNLASGVPDRFSGSGSGTAFTLRITRVEAEDVGIYYCMQHLEYPFTFGAGTKLELKRTTTPAPRPPTPAPTIASQPLSLRPEACRPAAGGAVHTRGLDFACDFWVLVVVGGVLACYSLLVTVAFIIFWVRSKRSRLLHSDYMNMTPRRPGPTRKHYQPYAPPRDFAAYRSKRGRKKLLYIFKQPFMRPVQTTQEEDGCSCRFPEEEEGGCELRVKFSRSADAPAYQQGQNQLYNELNLGRREEYDVLDKRRGRDPEMGGKPRRKNPQEGLYNELQKDKMAEAYSEIGMKGERRRGKGHDGLYQGLSTATKDTYDALHMQALPPR

SEQ ID NO: 132 - protein, 489 aa, synthetic construct
MLLLVTSLLLCELPHPAFLLIPEVKLEESGGGLVQPGGSMKLSCVASGFTFSNYWMNWVRQSPEKGLEWVAEIRLKSNNYATHYAESVKGRFTISRDDSKSSVYLQMNNLRAEDTGRYYCSRLPSFDYWGQGTTLTVSSGSTSGSGKPGSGEGSTKGDIVMTQAAPSVQVTPGESVSISCRSTKSLLHSNGNTYLYWFLQRPGQSPQLLIYRMSNLASGVPDRFSGSGSGTAFTLRITRVEAEDVGRYYCMQHLEYPFTFGAGTKLELKRIEVMYPPPYLDNEKSNGTIIHVKGKHLCPSPLFPGPSKPFWVLVVVGGVLACYSLLVTVAFIIFWVRSKRSRLLHSDYMNMTPRRPGPTRKHYQPYAPPRDFAAYRSRVKFSRSADAPAYQQGQNQLYNELNLGRREEYDVLDKRRGRDPEMGGKPRRKNPQEGLYNELQKDKMAEAYSEIGMKGERRRGKGHDGLYQGLSTATKDTYDALHMQALPPR

SEQ ID NO: 133 - protein, 493 aa, synthetic construct
MLLLVTSLLLCELPHPAFLLIPEVKLEESGGGLVQPGGSMKLSCVASGFTFSNYWMNWVRQSPEKGLEWVAEIRLKSNNYATHYAESVKGRFTISRDDSKSSVYLQMNNLRAEDTGRYYCSRLPSFDYWGQGTTLTVSSGSTSGSGKPGSGEGSTKGDIVMTQAAPSVQVTPGESVSISCRSTKSLLHSNGNTYLYWFLQRPGQSPQLLIYRMSNLASGVPDRFSGSGSGTAFTLRITRVEAEDVGRYYCMQHLEYPFTFGAGTKLELKRTTTPAPRPPTPAPTIASQPLSLRPEACRPAAGGAVHTRGLDFACDIYIWAPLAGTCGVLLLSLVITLYCKRGRKKLLYIFKQPFMRPVQTTQEEDGCSCRFPEEEEGGCELRVKFSRSADAPAYQQGQNQLYNELNLGRREEYDVLDKRRGRDPEMGGKPRRKNPQEGLYNELQKDKMAEAYSEIGMKGERRRGKGHDGLYQGLSTATKDTYDALHMQALPPR

SEQ ID NO: 134 - protein, 537 aa, synthetic construct
MLLLVTSLLLCELPHPAFLLIPEVKLEESGGGLVQPGGSMKLSCVASGFTFSNYWMNWVRQSPEKGLEWVAEIRLKSNNYATHYAESVKGRFTISRDDSKSSVYLQMNNLRAEDTGRYYCSRLPSFDYWGQGTTLTVSSGSTSGSGKPGSGEGSTKGDIVMTQAAPSVQVTPGESVSISCRSTKSLLHSNGNTYLYWFLQRPGQSPQLLIYRMSNLASGVPDRFSGSGSGTAFTLRITRVEAEDVGRYYCMQHLEYPFTFGAGTKLELKRTTTPAPRPPTPAPTIASQPLSLRPEACRPAAGGAVHTRGLDFACDFWVLVVVGGVLACYSLLVTVAFIIFWVRSKRSRLLHSDYMNMTPRRPGPTRKHYQPYAPPRDFAAYRSKRGRKKLLYIFKQPFMRPVQTTQEEDGCSCRFPEEEEGGCELRVKFSRSADAPAYQQGQNQLYNELNLGRREEYDVLDKRRGRDPEMGGKPRRKNPQEGLYNELQKDKMAEAYSEIGMKGERRRGKGHDGLYQGLSTATKDTYDALHMQALPPR

SEQ ID NO: 135 - protein, 496 aa, synthetic construct
MLLLVTSLLLCELPHPAFLLIPEVKLEESGGGLVQPGGSMKLSCVASGFTFSNYWMNWVRQSPEKGLEWVAEIRLKSNNYATHYAESVKGRFTISRDDSKSSVYLQMNNLRAEDTGRYYCSRLPSFDYWGQGTTLTVSSGGGGSGGGGSGGGGSGGGGSGGGGSDIVMTQAAPSVQVTPGESVSISCRSTKSLLHSNGNTYLYWFLQRPGQSPQLLIYRMSNLASGVPDRFSGSGSGTAFTLRITRVEAEDVGRYYCMQHLEYPFTFGAGTKLELKRIEVMYPPPYLDNEKSNGTIIHVKGKHLCPSPLFPGPSKPFWVLVVVGGVLACYSLLVTVAFIIFWVRSKRSRLLHSDYMNMTPRRPGPTRKHYQPYAPPRDFAAYRSRVKFSRSADAPAYQQGQNQLYNELNLGRREEYDVLDKRRGRDPEMGGKPRRKNPQEGLYNELQKDKMAEAYSEIGMKGERRRGKGHDGLYQGLSTATKDTYDALHMQALPPR

SEQ ID NO: 136 - protein, 500 aa, synthetic construct
MLLLVTSLLLCELPHPAFLLIPEVKLEESGGGLVQPGGSMKLSCVASGFTFSNYWMNWVRQSPEKGLEWVAEIRLKSNNYATHYAESVKGRFTISRDDSKSSVYLQMNNLRAEDTGRYYCSRLPSFDYWGQGTTLTVSSGGGGSGGGGSGGGGSGGGGSGGGGSDIVMTQAAPSVQVTPGESVSISCRSTKSLLHSNGNTYLYWFLQRPGQSPQLLIYRMSNLASGVPDRFSGSGSGTAFTLRITRVEAEDVGRYYCMQHLEYPFTFGAGTKLELKRTTTPAPRPPTPAPTIASQPLSLRPEACRPAAGGAVHTRGLDFACDIYIWAPLAGTCGVLLLSLVITLYCKRGRKKLLYIFKQPFMRPVQTTQEEDGCSCRFPEEEEGGCELRVKFSRSADAPAYQQGQNQLYNELNLGRREEYDVLDKRRGRDPEMGGKPRRKNPQEGLYNELQKDKMAEAYSEIGMKGERRRGKGHDGLYQGLSTATKDTYDALHMQALPPR

SEQ ID NO: 137 - protein, 544 aa, synthetic construct
MLLLVTSLLLCELPHPAFLLIPEVKLEESGGGLVQPGGSMKLSCVASGFTFSNYWMNWVRQSPEKGLEWVAEIRLKSNNYATHYAESVKGRFTISRDDSKSSVYLQMNNLRAEDTGRYYCSRLPSFDYWGQGTTLTVSSGGGGSGGGGSGGGGSGGGGSGGGGSDIVMTQAAPSVQVTPGESVSISCRSTKSLLHSNGNTYLYWFLQRPGQSPQLLIYRMSNLASGVPDRFSGSGSGTAFTLRITRVEAEDVGRYYCMQHLEYPFTFGAGTKLELKRTTTPAPRPPTPAPTIASQPLSLRPEACRPAAGGAVHTRGLDFACDFWVLVVVGGVLACYSLLVTVAFIIFWVRSKRSRLLHSDYMNMTPRRPGPTRKHYQPYAPPRDFAAYRSKRGRKKLLYIFKQPFMRPVQTTQEEDGCSCRFPEEEEGGCELRVKFSRSADAPAYQQGQNQLYNELNLGRREEYDVLDKRRGRDPEMGGKPRRKNPQEGLYNELQKDKMAEAYSEIGMKGERRRGKGHDGLYQGLSTATKDTYDALHMQALPPR

SEQ ID NO: 138 - protein, 501 aa, synthetic construct
MLLLVTSLLLCELPHPAFLLIPEVKLEESGGGLVQPGGSMKLSCVASGFTFSNYWMNWVRQSPEKGLEWVAEIRLKSNNYATHYAESVKGRFTISRDDSKSSVYLQMNNLRAEDTGIYYCSRLPSFDYWGQGTTLTVSSGGGGSGGGGSGGGGSGGGGSGGGGSGGGGSDIVMTQAAPSVPVTPGESVSISCRSTKSLLHSNGNTYLYWFLQRPGQSPQLLIYRMSNLASGVPDRFSGSGSGTAFTLRITRVEAEDVGIYYCMQHLEYPFTFGAGTKLELKRIEVMYPPPYLDNEKSNGTIIHVKGKHLCPSPLFPGPSKPFWVLVVVGGVLACYSLLVTVAFIIFWVRSKRSRLLHSDYMNMTPRRPGPTRKHYQPYAPPRDFAAYRSRVKFSRSADAPAYQQGQNQLYNELNLGRREEYDVLDKRRGRDPEMGGKPRRKNPQEGLYNELQKDKMAEAYSEIGMKGERRRGKGHDGLYQGLSTATKDTYDALHMQALPPR

SEQ ID NO: 139 - protein, 505 aa, synthetic construct
MLLLVTSLLLCELPHPAFLLIPEVKLEESGGGLVQPGGSMKLSCVASGFTFSNYWMNWVRQSPEKGLEWVAEIRLKSNNYATHYAESVKGRFTISRDDSKSSVYLQMNNLRAEDTGIYYCSRLPSFDYWGQGTTLTVSSGGGGSGGGGSGGGGSGGGGSGGGGSGGGGSDIVMTQAAPSVPVTPGESVSISCRSTKSLLHSNGNTYLYWFLQRPGQSPQLLIYRMSNLASGVPDRFSGSGSGTAFTLRITRVEAEDVGIYYCMQHLEYPFTFGAGTKLELKRTTTPAPRPPTPAPTIASQPLSLRPEACRPAAGGAVHTRGLDFACDIYIWAPLAGTCGVLLLSLVITLYCKRGRKKLLYIFKQPFMRPVQTTQEEDGCSCRFPEEEEGGCELRVKFSRSADAPAYQQGQNQLYNELNLGRREEYDVLDKRRGRDPEMGGKPRRKNPQEGLYNELQKDKMAEAYSEIGMKGERRRGKGHDGLYQGLSTATKDTYDALHMQALPPR

SEQ ID NO: 140 - protein, 549 aa, synthetic construct
MLLLVTSLLLCELPHPAFLLIPEVKLEESGGGLVQPGGSMKLSCVASGFTFSNYWMNWVRQSPEKGLEWVAEIRLKSNNYATHYAESVKGRFTISRDDSKSSVYLQMNNLRAEDTGIYYCSRLPSFDYWGQGTTLTVSSGGGGSGGGGSGGGGSGGGGSGGGGSGGGGSDIVMTQAAPSVPVTPGESVSISCRSTKSLLHSNGNTYLYWFLQRPGQSPQLLIYRMSNLASGVPDRFSGSGSGTAFTLRITRVEAEDVGIYYCMQHLEYPFTFGAGTKLELKRTTTPAPRPPTPAPTIASQPLSLRPEACRPAAGGAVHTRGLDFACDFWVLVVVGGVLACYSLLVTVAFIIFWVRSKRSRLLHSDYMNMTPRRPGPTRKHYQPYAPPRDFAAYRSKRGRKKLLYIFKQPFMRPVQTTQEEDGCSCRFPEEEEGGCELRVKFSRSADAPAYQQGQNQLYNELNLGRREEYDVLDKRRGRDPEMGGKPRRKNPQEGLYNELQKDKMAEAYSEIGMKGERRRGKGHDGLYQGLSTATKDTYDALHMQALPPR

SEQ ID NO: 141 - protein, 505 aa, synthetic construct
MLLLVTSLLLCELPHPAFLLIPEVKLEESGGGLVQPGGSMKLSCVASGFTFSNYWMNWVRQSPEKGLEWVAEIRLKSNNYATHYAESVKGRFTISRDDSKSSVYLQMNNLRAEDTGRYYCSRLPSFDYWGQGTTLTVSSGGGGSGGGGSGGGGSGGGGSGGGGSGGGGSDIVMTQAAPSVQVTPGESVSISCRSTKSLLHSNGNTYLYWFLQRPGQSPQLLIYRMSNLASGVPDRFSGSGSGTAFTLRITRVEAEDVGRYYCMQHLEYPFTFGAGTKLELKRTTTPAPRPPTPAPTIASQPLSLRPEACRPAAGGAVHTRGLDFACDIYIWAPLAGTCGVLLLSLVITLYCKRGRKKLLYIFKQPFMRPVQTTQEEDGCSCRFPEEEEGGCELRVKFSRSADAPAYQQGQNQLYNELNLGRREEYDVLDKRRGRDPEMGGKPRRKNPQEGLYNELQKDKMAEAYSEIGMKGERRRGKGHDGLYQGLSTATKDTYDALHMQALPPR

SEQ ID NO: 142 - protein, 549 aa, synthetic construct
MLLLVTSLLLCELPHPAFLLIPEVKLEESGGGLVQPGGSMKLSCVASGFTFSNYWMNWVRQSPEKGLEWVAEIRLKSNNYATHYAESVKGRFTISRDDSKSSVYLQMNNLRAEDTGRYYCSRLPSFDYWGQGTTLTVSSGGGGSGGGGSGGGGSGGGGSGGGGSGGGGSDIVMTQAAPSVQVTPGESVSISCRSTKSLLHSNGNTYLYWFLQRPGQSPQLLIYRMSNLASGVPDRFSGSGSGTAFTLRITRVEAEDVGRYYCMQHLEYPFTFGAGTKLELKRTTTPAPRPPTPAPTIASQPLSLRPEACRPAAGGAVHTRGLDFACDFWVLVVVGGVLACYSLLVTVAFIIFWVRSKRSRLLHSDYMNMTPRRPGPTRKHYQPYAPPRDFAAYRSKRGRKKLLYIFKQPFMRPVQTTQEEDGCSCRFPEEEEGGCELRVKFSRSADAPAYQQGQNQLYNELNLGRREEYDVLDKRRGRDPEMGGKPRRKNPQEGLYNELQKDKMAEAYSEIGMKGERRRGKGHDGLYQGLSTATKDTYDALHMQALPPR

SEQ ID NO: 143 - protein, 521 aa, synthetic construct
MLLLVTSLLLCELPHPAFLLIPEVKLEESGGGLVQPGGSMKLSCVASGFTFSNYWMNWVRQSPEKGLEWVAEIRLKSNNYATHYAESVKGRFTISRDDSKSSVYLQMNNLRAEDTGRYYCSRLPSFDYWGQGTTLTVSSGGGGSGGGGSGGGGSGGGGSGGGGSGGGGSGGGGSGGGGSGGGGSGGGGSDIVMTQAAPSVQVTPGESVSISCRSTKSLLHSNGNTYLYWFLQRPGQSPQLLIYRMSNLASGVPDRFSGSGSGTAFTLRITRVEAEDVGRYYCMQHLEYPFTFGAGTKLELKRIEVMYPPPYLDNEKSNGTIIHVKGKHLCPSPLFPGPSKPFWVLVVVGGVLACYSLLVTVAFIIFWVRSKRSRLLHSDYMNMTPRRPGPTRKHYQPYAPPRDFAAYRSRVKFSRSADAPAYQQGQNQLYNELNLGRREEYDVLDKRRGRDPEMGGKPRRKNPQEGLYNELQKDKMAEAYSEIGMKGERRRGKGHDGLYQGLSTATKDTYDALHMQALPPR

SEQ ID NO: 144 - protein, 525 aa, synthetic construct
MLLLVTSLLLCELPHPAFLLIPEVKLEESGGGLVQPGGSMKLSCVASGFTFSNYWMNWVRQSPEKGLEWVAEIRLKSNNYATHYAESVKGRFTISRDDSKSSVYLQMNNLRAEDTGRYYCSRLPSFDYWGQGTTLTVSSGGGGSGGGGSGGGGSGGGGSGGGGSGGGGSGGGGSGGGGSGGGGSGGGGSDIVMTQAAPSVQVTPGESVSISCRSTKSLLHSNGNTYLYWFLQRPGQSPQLLIYRMSNLASGVPDRFSGSGSGTAFTLRITRVEAEDVGRYYCMQHLEYPFTFGAGTKLELKRTTTPAPRPPTPAPTIASQPLSLRPEACRPAAGGAVHTRGLDFACDIYIWAPLAGTCGVLLLSLVITLYCKRGRKKLLYIFKQPFMRPVQTTQEEDGCSCRFPEEEEGGCELRVKFSRSADAPAYQQGQNQLYNELNLGRREEYDVLDKRRGRDPEMGGKPRRKNPQEGLYNELQKDKMAEAYSEIGMKGERRRGKGHDGLYQGLSTATKDTYDALHMQALPPR

SEQ ID NO: 145 - protein, 569 aa, synthetic construct
MLLLVTSLLLCELPHPAFLLIPEVKLEESGGGLVQPGGSMKLSCVASGFTFSNYWMNWVRQSPEKGLEWVAEIRLKSNNYATHYAESVKGRFTISRDDSKSSVYLQMNNLRAEDTGRYYCSRLPSFDYWGQGTTLTVSSGGGGSGGGGSGGGGSGGGGSGGGGSGGGGSGGGGSGGGGSGGGGSGGGGSDIVMTQAAPSVQVTPGESVSISCRSTKSLLHSNGNTYLYWFLQRPGQSPQLLIYRMSNLASGVPDRFSGSGSGTAFTLRITRVEAEDVGRYYCMQHLEYPFTFGAGTKLELKRTTTPAPRPPTPAPTIASQPLSLRPEACRPAAGGAVHTRGLDFACDFWVLVVVGGVLACYSLLVTVAFIIFWVRSKRSRLLHSDYMNMTPRRPGPTRKHYQPYAPPRDFAAYRSKRGRKKLLYIFKQPFMRPVQTTQEEDGCSCRFPEEEEGGCELRVKFSRSADAPAYQQGQNQLYNELNLGRREEYDVLDKRRGRDPEMGGKPRRKNPQEGLYNELQKDKMAEAYSEIGMKGERRRGKGHDGLYQGLSTATKDTYDALHMQALPPR

SEQ ID NO: 146 - protein, 501 aa, synthetic construct
MLLLVTSLLLCELPHPAFLLIPEVKLEESGGGLVQPGGSMKLSCVASGFTFSNYWMNWVRQSPEKGLEWVAEIRLKSNNYATHYAESVKGRFTISRDDSKSSVYLQMNNLRAEDTGRYYCSRLPSFDYWGQGTTLTVSSGGGGSGGGGSGGGGSGGGGSGGGGSGGGGSDIVMTQAAPSVQVTPGESVSISCRSTKSLLHSNGNTYLYWFLQRPGQSPQLLIYRMSNLASGVPDRFSGSGSGTAFTLRITRVEAEDVGRYYCMQHLEYPFTFGAGTKLELKRIEVMYPPPYLDNEKSNGTIIHVKGKHLCPSPLFPGPSKPFWVLVVVGGVLACYSLLVTVAFIIFWVRSKRSRLLHSDYMNMTPRRPGPTRKHYQPYAPPRDFAAYRSRVKFSRSADAPAYQQGQNQLYNELNLGRREEYDVLDKRRGRDPEMGGKPRRKNPQEGLYNELQKDKMAEAYSEIGMKGERRRGKGHDGLYQGLSTATKDTYDALHMQALPPR

SEQ ID NO: 147 - protein, 489 aa, synthetic construct
MLLLVTSLLLCELPHPAFLLIPEVKLEESGGGLVQPGGSMKLSCVASGFTFSNYWMNWVRQSPEKGLEWVAEIRLKSNNYATHYAESVKGRFTISRDDSKSSVYLQMNNLRAEDTGRYYCSRLPSFDYWGQGTTLTVSSGSTSGSGKPGSGEGSTKGDIVMTQAAPSVRVTPGESVSISCRSTKSLLHSNGNTYLYWFLQRPGQSPQLLIYRMSNLASGVPDRFSGSGSGTAFTLRITRVEAEDVGRYYCMQHLEYPFTFGAGTKLELKRIEVMYPPPYLDNEKSNGTIIHVKGKHLCPSPLFPGPSKPFWVLVVVGGVLACYSLLVTVAFIIFWVRSKRSRLLHSDYMNMTPRRPGPTRKHYQPYAPPRDFAAYRSRVKFSRSADAPAYQQGQNQLYNELNLGRREEYDVLDKRRGRDPEMGGKPRRKNPQEGLYNELQKDKMAEAYSEIGMKGERRRGKGHDGLYQGLSTATKDTYDALHMQALPPR

SEQ ID NO: 148 - protein, 493 aa, synthetic construct
MLLLVTSLLLCELPHPAFLLIPEVKLEESGGGLVQPGGSMKLSCVASGFTFSNYWMNWVRQSPEKGLEWVAEIRLKSNNYATHYAESVKGRFTISRDDSKSSVYLQMNNLRAEDTGRYYCSRLPSFDYWGQGTTLTVSSGSTSGSGKPGSGEGSTKGDIVMTQAAPSVRVTPGESVSISCRSTKSLLHSNGNTYLYWFLQRPGQSPQLLIYRMSNLASGVPDRFSGSGSGTAFTLRITRVEAEDVGRYYCMQHLEYPFTFGAGTKLELKRTTTPAPRPPTPAPTIASQPLSLRPEACRPAAGGAVHTRGLDFACDIYIWAPLAGTCGVLLLSLVITLYCKRGRKKLLYIFKQPFMRPVQTTQEEDGCSCRFPEEEEGGCELRVKFSRSADAPAYQQGQNQLYNELNLGRREEYDVLDKRRGRDPEMGGKPRRKNPQEGLYNELQKDKMAEAYSEIGMKGERRRGKGHDGLYQGLSTATKDTYDALHMQALPPR

SEQ ID NO: 149 - protein, 537 aa, synthetic construct
MLLLVTSLLLCELPHPAFLLIPEVKLEESGGGLVQPGGSMKLSCVASGFTFSNYWMNWVRQSPEKGLEWVAEIRLKSNNYATHYAESVKGRFTISRDDSKSSVYLQMNNLRAEDTGRYYCSRLPSFDYWGQGTTLTVSSGSTSGSGKPGSGEGSTKGDIVMTQAAPSVRVTPGESVSISCRSTKSLLHSNGNTYLYWFLQRPGQSPQLLIYRMSNLASGVPDRFSGSGSGTAFTLRITRVEAEDVGRYYCMQHLEYPFTFGAGTKLELKRTTTPAPRPPTPAPTIASQPLSLRPEACRPAAGGAVHTRGLDFACDFWVLVVVGGVLACYSLLVTVAFIIFWVRSKRSRLLHSDYMNMTPRRPGPTRKHYQPYAPPRDFAAYRSKRGRKKLLYIFKQPFMRPVQTTQEEDGCSCRFPEEEEGGCELRVKFSRSADAPAYQQGQNQLYNELNLGRREEYDVLDKRRGRDPEMGGKPRRKNPQEGLYNELQKDKMAEAYSEIGMKGERRRGKGHDGLYQGLSTATKDTYDALHMQALPPR

SEQ ID NO: 150 - protein, 496 aa, synthetic construct
MLLLVTSLLLCELPHPAFLLIPEVKLEESGGGLVQPGGSMKLSCVASGFTFSNYWMNWVRQSPEKGLEWVAEIRLKSNNYATHYAESVKGRFTISRDDSKSSVYLQMNNLRAEDTGRYYCSRLPSFDYWGQGTTLTVSSGGGGSGGGGSGGGGSGGGGSGGGGSDIVMTQAAPSVRVTPGESVSISCRSTKSLLHSNGNTYLYWFLQRPGQSPQLLIYRMSNLASGVPDRFSGSGSGTAFTLRITRVEAEDVGRYYCMQHLEYPFTFGAGTKLELKRIEVMYPPPYLDNEKSNGTIIHVKGKHLCPSPLFPGPSKPFWVLVVVGGVLACYSLLVTVAFIIFWVRSKRSRLLHSDYMNMTPRRPGPTRKHYQPYAPPRDFAAYRSRVKFSRSADAPAYQQGQNQLYNELNLGRREEYDVLDKRRGRDPEMGGKPRRKNPQEGLYNELQKDKMAEAYSEIGMKGERRRGKGHDGLYQGLSTATKDTYDALHMQALPPR

SEQ ID NO: 151 - protein, 500 aa, synthetic construct
MLLLVTSLLLCELPHPAFLLIPEVKLEESGGGLVQPGGSMKLSCVASGFTFSNYWMNWVRQSPEKGLEWVAEIRLKSNNYATHYAESVKGRFTISRDDSKSSVYLQMNNLRAEDTGRYYCSRLPSFDYWGQGTTLTVSSGGGGSGGGGSGGGGSGGGGSGGGGSDIVMTQAAPSVRVTPGESVSISCRSTKSLLHSNGNTYLYWFLQRPGQSPQLLIYRMSNLASGVPDRFSGSGSGTAFTLRITRVEAEDVGRYYCMQHLEYPFTFGAGTKLELKRTTTPAPRPPTPAPTIASQPLSLRPEACRPAAGGAVHTRGLDFACDIYIWAPLAGTCGVLLLSLVITLYCKRGRKKLLYIFKQPFMRPVQTTQEEDGCSCRFPEEEEGGCELRVKFSRSADAPAYQQGQNQLYNELNLGRREEYDVLDKRRGRDPEMGGKPRRKNPQEGLYNELQKDKMAEAYSEIGMKGERRRGKGHDGLYQGLSTATKDTYDALHMQALPPR

SEQ ID NO: 152 - protein, 544 aa, synthetic construct
MLLLVTSLLLCELPHPAFLLIPEVKLEESGGGLVQPGGSMKLSCVASGFTFSNYWMNWVRQSPEKGLEWVAEIRLKSNNYATHYAESVKGRFTISRDDSKSSVYLQMNNLRAEDTGRYYCSRLPSFDYWGQGTTLTVSSGGGGSGGGGSGGGGSGGGGSGGGGSDIVMTQAAPSVRVTPGESVSISCRSTKSLLHSNGNTYLYWFLQRPGQSPQLLIYRMSNLASGVPDRFSGSGSGTAFTLRITRVEAEDVGRYYCMQHLEYPFTFGAGTKLELKRTTTPAPRPPTPAPTIASQPLSLRPEACRPAAGGAVHTRGLDFACDFWVLVVVGGVLACYSLLVTVAFIIFWVRSKRSRLLHSDYMNMTPRRPGPTRKHYQPYAPPRDFAAYRSKRGRKKLLYIFKQPFMRPVQTTQEEDGCSCRFPEEEEGGCELRVKFSRSADAPAYQQGQNQLYNELNLGRREEYDVLDKRRGRDPEMGGKPRRKNPQEGLYNELQKDKMAEAYSEIGMKGERRRGKGHDGLYQGLSTATKDTYDALHMQALPPR

SEQ ID NO: 153 - protein, 501 aa, synthetic construct
MLLLVTSLLLCELPHPAFLLIPEVKLEESGGGLVQPGGSMKLSCVASGFTFSNYWMNWVRQSPEKGLEWVAEIRLKSNNYATHYAESVKGRFTISRDDSKSSVYLQMNNLRAEDTGRYYCSRLPSFDYWGQGTTLTVSSGGGGSGGGGSGGGGSGGGGSGGGGSGGGGSDIVMTQAAPSVRVTPGESVSISCRSTKSLLHSNGNTYLYWFLQRPGQSPQLLIYRMSNLASGVPDRFSGSGSGTAFTLRITRVEAEDVGRYYCMQHLEYPFTFGAGTKLELKRIEVMYPPPYLDNEKSNGTIIHVKGKHLCPSPLFPGPSKPFWVLVVVGGVLACYSLLVTVAFIIFWVRSKRSRLLHSDYMNMTPRRPGPTRKHYQPYAPPRDFAAYRSRVKFSRSADAPAYQQGQNQLYNELNLGRREEYDVLDKRRGRDPEMGGKPRRKNPQEGLYNELQKDKMAEAYSEIGMKGERRRGKGHDGLYQGLSTATKDTYDALHMQALPPR

SEQ ID NO: 154 - protein, 505 aa, synthetic construct
MLLLVTSLLLCELPHPAFLLIPEVKLEESGGGLVQPGGSMKLSCVASGFTFSNYWMNWVRQSPEKGLEWVAEIRLKSNNYATHYAESVKGRFTISRDDSKSSVYLQMNNLRAEDTGRYYCSRLPSFDYWGQGTTLTVSSGGGGSGGGGSGGGGSGGGGSGGGGSGGGGSDIVMTQAAPSVRVTPGESVSISCRSTKSLLHSNGNTYLYWFLQRPGQSPQLLIYRMSNLASGVPDRFSGSGSGTAFTLRITRVEAEDVGRYYCMQHLEYPFTFGAGTKLELKRTTTPAPRPPTPAPTIASQPLSLRPEACRPAAGGAVHTRGLDFACDIYIWAPLAGTCGVLLLSLVITLYCKRGRKKLLYIFKQPFMRPVQTTQEEDGCSCRFPEEEEGGCELRVKFSRSADAPAYQQGQNQLYNELNLGRREEYDVLDKRRGRDPEMGGKPRRKNPQEGLYNELQKDKMAEAYSEIGMKGERRRGKGHDGLYQGLSTATKDTYDALHMQALPPR

SEQ ID NO: 155 - protein, 549 aa, synthetic construct
MLLLVTSLLLCELPHPAFLLIPEVKLEESGGGLVQPGGSMKLSCVASGFTFSNYWMNWVRQSPEKGLEWVAEIRLKSNNYATHYAESVKGRFTISRDDSKSSVYLQMNNLRAEDTGRYYCSRLPSFDYWGQGTTLTVSSGGGGSGGGGSGGGGSGGGGSGGGGSGGGGSDIVMTQAAPSVRVTPGESVSISCRSTKSLLHSNGNTYLYWFLQRPGQSPQLLIYRMSNLASGVPDRFSGSGSGTAFTLRITRVEAEDVGRYYCMQHLEYPFTFGAGTKLELKRTTTPAPRPPTPAPTIASQPLSLRPEACRPAAGGAVHTRGLDFACDFWVLVVVGGVLACYSLLVTVAFIIFWVRSKRSRLLHSDYMNMTPRRPGPTRKHYQPYAPPRDFAAYRSKRGRKKLLYIFKQPFMRPVQTTQEEDGCSCRFPEEEEGGCELRVKFSRSADAPAYQQGQNQLYNELNLGRREEYDVLDKRRGRDPEMGGKPRRKNPQEGLYNELQKDKMAEAYSEIGMKGERRRGKGHDGLYQGLSTATKDTYDALHMQALPPR

SEQ ID NO: 156 - protein, 521 aa, synthetic construct
MLLLVTSLLLCELPHPAFLLIPEVKLEESGGGLVQPGGSMKLSCVASGFTFSNYWMNWVRQSPEKGLEWVAEIRLKSNNYATHYAESVKGRFTISRDDSKSSVYLQMNNLRAEDTGRYYCSRLPSFDYWGQGTTLTVSSGGGGSGGGGSGGGGSGGGGSGGGGSGGGGSGGGGSGGGGSGGGGSGGGGSDIVMTQAAPSVRVTPGESVSISCRSTKSLLHSNGNTYLYWFLQRPGQSPQLLIYRMSNLASGVPDRFSGSGSGTAFTLRITRVEAEDVGRYYCMQHLEYPFTFGAGTKLELKRIEVMYPPPYLDNEKSNGTIIHVKGKHLCPSPLFPGPSKPFWVLVVVGGVLACYSLLVTVAFIIFWVRSKRSRLLHSDYMNMTPRRPGPTRKHYQPYAPPRDFAAYRSRVKFSRSADAPAYQQGQNQLYNELNLGRREEYDVLDKRRGRDPEMGGKPRRKNPQEGLYNELQKDKMAEAYSEIGMKGERRRGKGHDGLYQGLSTATKDTYDALHMQALPPR

SEQ ID NO: 157 - protein, 525 aa, synthetic construct
MLLLVTSLLLCELPHPAFLLIPEVKLEESGGGLVQPGGSMKLSCVASGFTFSNYWMNWVRQSPEKGLEWVAEIRLKSNNYATHYAESVKGRFTISRDDSKSSVYLQMNNLRAEDTGRYYCSRLPSFDYWGQGTTLTVSSGGGGSGGGGSGGGGSGGGGSGGGGSGGGGSGGGGSGGGGSGGGGSGGGGSDIVMTQAAPSVRVTPGESVSISCRSTKSLLHSNGNTYLYWFLQRPGQSPQLLIYRMSNLASGVPDRFSGSGSGTAFTLRITRVEAEDVGRYYCMQHLEYPFTFGAGTKLELKRTTTPAPRPPTPAPTIASQPLSLRPEACRPAAGGAVHTRGLDFACDIYIWAPLAGTCGVLLLSLVITLYCKRGRKKLLYIFKQPFMRPVQTTQEEDGCSCRFPEEEEGGCELRVKFSRSADAPAYQQGQNQLYNELNLGRREEYDVLDKRRGRDPEMGGKPRRKNPQEGLYNELQKDKMAEAYSEIGMKGERRRGKGHDGLYQGLSTATKDTYDALHMQALPPR

SEQ ID NO: 158 - protein, 569 aa, synthetic construct
MLLLVTSLLLCELPHPAFLLIPEVKLEESGGGLVQPGGSMKLSCVASGFTFSNYWMNWVRQSPEKGLEWVAEIRLKSNNYATHYAESVKGRFTISRDDSKSSVYLQMNNLRAEDTGRYYCSRLPSFDYWGQGTTLTVSSGGGGSGGGGSGGGGSGGGGSGGGGSGGGGSGGGGSGGGGSGGGGSGGGGSDIVMTQAAPSVRVTPGESVSISCRSTKSLLHSNGNTYLYWFLQRPGQSPQLLIYRMSNLASGVPDRFSGSGSGTAFTLRITRVEAEDVGRYYCMQHLEYPFTFGAGTKLELKRTTTPAPRPPTPAPTIASQPLSLRPEACRPAAGGAVHTRGLDFACDFWVLVVVGGVLACYSLLVTVAFIIFWVRSKRSRLLHSDYMNMTPRRPGPTRKHYQPYAPPRDFAAYRSKRGRKKLLYIFKQPFMRPVQTTQEEDGCSCRFPEEEEGGCELRVKFSRSADAPAYQQGQNQLYNELNLGRREEYDVLDKRRGRDPEMGGKPRRKNPQEGLYNELQKDKMAEAYSEIGMKGERRRGKGHDGLYQGLSTATKDTYDALHMQALPPR

SEQ ID NO: 159 - protein, 492 aa, synthetic construct; identical to SEQ ID NO: 118

SEQ ID NO: 160 - protein, 496 aa, synthetic construct
MLLLVTSLLLCELPHPAFLLIPEVKLEESGGGLVQPGGSMKLSCVASGFTFSNYWMNWVRQSPEKGLEWVAEIRLKSNNYATHYAESVKGRFTISRDDSKSSVYLQMNNLRAEDTGRYYCSRLPSFDYWGQGTTLTVSSGSTSGSGKPGSGEGSTKGDIVMTQAAPSVQVTPGESVSISCRSTKSLLHSNGNTYLYWFLQRPGQSPQLLIYRMSNLASGVPDRFSGSGSGTAFTLRITRVEAEDVGRYYCMQHLEYPFTFGAGTKLELKRAAATTTPAPRPPTPAPTIASQPLSLRPEACRPAAGGAVHTRGLDFACDIYIWAPLAGTCGVLLLSLVITLYCKRGRKKLLYIFKQPFMRPVQTTQEEDGCSCRFPEEEEGGCELRVKFSRSADAPAYQQGQNQLYNELNLGRREEYDVLDKRRGRDPEMGGKPRRKNPQEGLYNELQKDKMAEAYSEIGMKGERRRGKGHDGLYQGLSTATKDTYDALHMQALPPR

SEQ ID NO: 161 - protein, 503 aa, synthetic construct
MLLLVTSLLLCELPHPAFLLIPEVKLEESGGGLVQPGGSMKLSCVASGFTFSNYWMNWVRQSPEKGLEWVAEIRLKSNNYATHYAESVKGRFTISRDDSKSSVYLQMNNLRAEDTGRYYCSRLPSFDYWGQGTTLTVSSGGGGSGGGGSGGGGSGGGGSGGGGSDIVMTQAAPSVQVTPGESVSISCRSTKSLLHSNGNTYLYWFLQRPGQSPQLLIYRMSNLASGVPDRFSGSGSGTAFTLRITRVEAEDVGRYYCMQHLEYPFTFGAGTKLELKRAAATTTPAPRPPTPAPTIASQPLSLRPEACRPAAGGAVHTRGLDFACDIYIWAPLAGTCGVLLLSLVITLYCKRGRKKLLYIFKQPFMRPVQTTQEEDGCSCRFPEEEEGGCELRVKFSRSADAPAYQQGQNQLYNELNLGRREEYDVLDKRRGRDPEMGGKPRRKNPQEGLYNELQKDKMAEAYSEIGMKGERRRGKGHDGLYQGLSTATKDTYDALHMQALPPR

SEQ ID NO: 162 - protein, 528 aa, synthetic construct
MLLLVTSLLLCELPHPAFLLIPEVKLEESGGGLVQPGGSMKLSCVASGFTFSNYWMNWVRQSPEKGLEWVAEIRLKSNNYATHYAESVKGRFTISRDDSKSSVYLQMNNLRAEDTGRYYCSRLPSFDYWGQGTTLTVSSGGGGSGGGGSGGGGSGGGGSGGGGSGGGGSGGGGSGGGGSGGGGSGGGGSDIVMTQAAPSVQVTPGESVSISCRSTKSLLHSNGNTYLYWFLQRPGQSPQLLIYRMSNLASGVPDRFSGSGSGTAFTLRITRVEAEDVGRYYCMQHLEYPFTFGAGTKLELKRAAATTTPAPRPPTPAPTIASQPLSLRPEACRPAAGGAVHTRGLDFACDIYIWAPLAGTCGVLLLSLVITLYCKRGRKKLLYIFKQPFMRPVQTTQEEDGCSCRFPEEEEGGCELRVKFSRSADAPAYQQGQNQLYNELNLGRREEYDVLDKRRGRDPEMGGKPRRKNPQEGLYNELQKDKMAEAYSEIGMKGERRRGKGHDGLYQGLSTATKDTYDALHMQALPPR